European Patent Specification EP 3 393 523 B9, published October 4, 2023. Title: ENDOTHELIUM-SPECIFIC NUCLEIC ACID REGULATORY ELEMENTS AND METHODS AND USE THEREOF. Applicant: VRIJE UNIVERSITEIT BRUSSEL. The sequence listing filed with the application follows.

SEQUENCE LISTING (56 sequences)

SEQ ID NO: 1 - DNA, 76 bp, Homo sapiens
gccctcacaaaggaacaataacaggaaaccatcccagggggaagtgggccagggccagctggaaaacctgaagggg

SEQ ID NO: 2 - DNA, 277 bp, Homo sapiens
ggccgaggcagccgcccaccgcagggcctgcctatctgcagccagcccagccctcacaaaggaacaataacaggaaaccatcccagggggaagtgggccagggccagctggaaaacctgaaggggaggcagccaggcctccctcgccagcggggtgtggctcccctccaaagacggtcggctgacaggctccacagagctccactcacgctcagccctggacggacaggcagtccaacggaacagaaacatccctcagcccacaggcacggtgagtg

SEQ ID NO: 3 - DNA, 408 bp, Homo sapiens
gcttcctcctctgctactaatctggtctcacagaccatcccatttcctgctagcccaccagccgccttccttgctcccaatgacacttcctggccttgtgccctcctgttacctcctttgcctccagagaggttggagcagaggctgggcagtgccagaaatcaggcatgaaatcctcagggggaccaaggaggcaccagcctccctcccacagtctcagctacctctgctacggtgacccccagccccacccctggggcccacagctcatgcctggctcaccattcctttgtttatggaccacaggaacagtcgttttcagggcagagtcaacttcctcatggactgggagtacaaagggaattggcagatggtgccaggacaggccctgtccccatctgccacagc

SEQ ID NO: 4 - DNA, 173 bp, Homo sapiens
gcttcctcctctgctactaatctggtctcacagaccatcccatttcctgctagcccaccagccgccttccttgctcccaatgacacttcctggccttgtgccctcctgttacctcctttgcctccagagaggttggagcagaggctgggcagtgccagaaatcaggcatgaaa

SEQ ID NO: 5 - DNA, 307 bp, Homo sapiens
cccagctgagggctggtgccagagccgtgtctgcttgccccatcaagaggtgggagggattgatccaccttcctgccccacagatggtgcagcctccaacctattgttttccaggacgcttcggtggagagcacaaggaatgtagggtctagaaacaggaagccctggcttccgctggacaaggtttcctccagactcaggcctgccctccagacaacaaggcagggcccttggtcccaccctgccctgcctggctcactgggccaccccaaggaaggccttgccctctctgggcttctgcatgtga

SEQ ID NO: 6 - DNA, 450 bp, Homo sapiens
aggtatccaccaaggggcccaagagctgctgagcccctgagcagccctaccaatttcagcttatggtggtgaggggtaggggaggtgtatactggcctggaaggggttaagctgcccgcctgcagcctcagcctgagctattgtgttgccaaacaagggccggacatgagggcaggaagccagcaggggccacacattttctgcaaagttggatgattcactgctgacttggggacacccaggggacagaggggacaccatcccaggaagaatcttaggctcattttgcccacatggacccatgactgttccctgtatcctctctctgcaccccctcagtcacactgaagcaactatgagaattcccatttgacagatgggaccatcgaggctgagggaagctgtgcagccagtccaaggtcacacaaccaacacaaggtagaagcaggg

SEQ ID NO: 7 - DNA, 123 bp, Homo sapiens
agggcccctggagctggtcccaatgtgtttccttctattcttttgacaggaagctcctggagagccagtccccacccccatcccgccccagcactccctctctcttctccactatggacagag

SEQ ID NO: 8 - DNA, 499 bp, Homo sapiens
tagggcctctctgaaagatgtggggagtcctatctgcattgggatccctgaggagggagaggaatgtggagaattcagggtccagggagcatgggtgactggtgggctgggcttccaggctgaatcatgggaaaggagaacctggtctgaaacagtactgggcgggattggtgttagattccaggaaaacccccaggcggtctgtggtggaacctgatggaccctcagaagggaagagaatggggatggggccaggttgccatggttggtcattgtgcataggcactagaggccatgctgggtgggcacagtcgctgctgcagcctcacatcctcatctggacatggctgagcagggcccctggagctggtcccaatgtgtttccttctattcttttgacaggaagctcctggagagccagtccccacccccatcccgccccagcactccctctctcttctccactatggacagagcctccactgagctgctgcctgcc

SEQ ID NO: 9 - DNA, 455 bp, Homo sapiens
gagacataaaaggaaaatgaagcgagcaacaattaaaaaaaattccccgcacacaacaatacaatctatttaaactgtggctcatacttttcataccaatggtatgactttttttctggagtcccctcttctgattcttgaactccggggctggcagcttgcaaaggggaagcggactccagcactgcacgggcaggtttagcaaaggtctctaatgggtattttctttttcttagccctgcccccgaattgtcagacggcgggcgtctgcctctgaagttagcagtgatttcctttcgggcctggccttatctccggctgcacgttgcctgttggtgactaataacacaataacattgtctggggctggaataaagtcggagctgtttacccccactctaataggggttcaatataaaaagccggcagagagctgtccaagtcagacgcgcctc

SEQ ID NO: 10 - DNA, 153 bp, Homo sapiens
tgtccacttctcctgacccctcggccgccaccccagaaggctggagcagggacgccgtcgctccggccgcctgctcccctcgggtccccgtgcgagcccacgccggccccggtgcccgcccgcagccctgccactggacacaggataaggccc

SEQ ID NO: 11 - DNA, 125 bp, Homo sapiens
gggccccccacccagtgacaaagcccgtggcacttcctctacccggttggcaggcggcctggcccagccccttctctaaggaagcgcatttcctgcctccctgggccggccgggctggatgagcc

SEQ ID NO: 12 - DNA, 498 bp, Homo sapiens
gggatgggagggtggggtgcttggggagacaagcctagagcctgggccctcccaccccactgcctccccccatcccagggccccccacccagtgacaaagcccgtggcacttcctctacccggttggcaggcggcctggcccagccccttctctaaggaagcgcatttcctgcctccctgggccggccgggctggatgagccaggagctccctgctgccggtcataccacagccttcatctgcgccctggggccaggactgctgctgtcactgccatccattggagcccagcaccccctccccgcccatccttcggacagcaactccagcccagccccgcgtccctgtgtccacttctcctgacccctcggccgccaccccagaaggctggagcagggacgccgtcgctccggccgcctgctcccctcgggtccccgtgcgagcccacgccggccccggtgcccgcccgcagccctgccactggacacaggataaggc

SEQ ID NO: 13 - DNA, 136 bp, Homo sapiens
agcggtgacgtcaaggggcgcgctgtggcagcacctccccgcgcgctagttaaaaagaagaagaaaagagggaacgaaacatgagaggctgtgtgagaagctgcagccgccggcagaggagacctcagcatcatct

SEQ ID NO: 14 - DNA, 574 bp, Homo sapiens
ctgggcgggggcgcgcgagaagcggtgacgtcaaggggcgcgctgtggcagcacctccccgcgcgctagttaaaaagaagaagaaaagagggaacgaaacatgagaggctgtgtgagaagctgcagccgccggcagaggagacctcagcatcatctagagcccagcgctggccctgcctccgcctgccccgccgccgccgtcgccgtttctgttcctgctactgtcccacctaaacaactcccgttacacggacaagtgaacatctgtggctgtcctctccttttcttcctcctcttccaactccttctcctcctcccacttcccagccgcagcagaaagcccccaacccaactgacactggcacaactgcaaacggtgtcatccgcacaactttatctcgctcctcgggctcccctaaggcattggacccatcgccgcgtcttttattttttgcaaagttgcatcgctgtacatatttttgtccccgccacctccctctgtctctggagtgccctacagccccgcaaactcctcctggagctgcgccctagtgcccctgctgggcagtggcgt

SEQ ID NO: 15 - DNA, 170 bp, Homo sapiens
agggaactccctgtgctgggcctacccagctgaccccatcgctggaaacaatgggggtcaggcaacacttccccactctctcccgccgggctgtgctcacttccttcctgctggctgcctgaggaagtgtccctgccctgggacagtctggcctagcctttgtttccccg

SEQ ID NO: 16 - DNA, 470 bp, Homo sapiens
gacaggcttctgagtgtagggagctggtctgccagtctttcggaggtttgaacttgtcaaggctagggcaggatcaccatatccagcctggacttgcagttctgtggggtgcctccccatacccccataagatgccaaacatgaggccctgtcatcctccatggtccccctctactggctgttcaaggcccagggctctcccatgccagatagcatcctgtctcctaccaccactgtcccagcctgagggaactccctgtgctgggcctacccagctgaccccatcgctggaaacaatgggggtcaggcaacacttccccactctctcccgccgggctgtgctcacttccttcctgctggctgcctgaggaagtgtccctgccctgggacagtctggcctagcctttgtttccccgggggtccccacccatggagctttcaaggcttctggcccctgtgaagccagcaca

SEQ ID NO: 17 - DNA, 602 bp, Homo sapiens
cagtggaaaaaaacggactcagctactggaagtccccccgaccctccccccaaggctagttcccttcttgggcacctgctctgggggaccatcagctgaacgacccccaagtattttgactcccaaaagcaccaccacctgaccccatcctctcacaccctactggatttgaggatgggccccaatcctagggaaggagtgaagaggttccctagtgttggaagctgtgggtgtgggggagattggcacctgatcctgagcccatagccttcctgtcacctggcgcagctggcggggccagatcctactcgggaagggtggggagggcagccagccagcagggcattctggagggaaacagggtcaaggcgatctcctcccccacgcctgttcctggccctttcctctcagggggcagcaggaagtgaggagaaagggctgggatgggaggcgggagcggatgggagggaatggggtttatcaagtcctcggcgagctgcccaacgggcagcagctggcgcaagtagcctagctggagaggctcaccccaggaaggagggaggccaccgacctactgggccgacggactcccacacaggtga

SEQ ID NO: 18 - DNA, 265 bp, Homo sapiens
cttgcatagatggccagcgttcatactttctgcttgtttgtacaaagtcattcttctagagtaattgttgtaaaattgctaggcaaggtggcaggtctgataagatttgatgacgtaatggctcttagtcgctaataagaggcttttgtggagtggcgtgtcacagccagcgaaggctcagctctgtgatcttcgcctgcctcacttgggggaccagaaggcagcttgtcttggaactgcctcattcacagaagaccccattgag

SEQ ID NO: 19 - DNA, 545 bp, Homo sapiens
tttacctagcatgatcttggcagttcaaagaggaatgtgccagaaaccaagcaaagaagaaaaagaaataaatggaaatggaaagtgatctgctcagaggccacaaagttgagggaggaggtttccagagtgggatttggcccaaatgttgcctgaggaagtacgtaaaggggtctcaactctggctacacaacagaacagcaggactgtgtgtgcagctcacgaagtgggtacacagggtaatctgcaagttctgggtggatctagcacctggattgttaaaacttgcatagatggccagcgttcatactttctgcttgtttgtacaaagtcattcttctagagtaattgttgtaaaattgctaggcaaggtggcaggtctgataagatttgatgacgtaatggctcttagtcgctaataagaggcttttgtggagtggcgtgtcacagccagcgaaggctcagctctgtgatcttcgcctgcctcacttgggggaccagaaggcagcttgtcttggaactgcctcattcacagaagaccccat

SEQ ID NO: 20 - DNA, 554 bp, Homo sapiens
atggcagctggcaggtgccttcacgtccagggtttccagagagaaagcatctctcctccgcagagaccctcccacgctctccctccctcaaattagtgcatctacatagaccgccctccttataaacagtctctcaggggatcctagcccattccaaatctacctgtgattgcagaatcgcaaggaatgtgatttaccgcagatcgcggggcgtcgtgtcttttaggggacctgctcactttggccactaggtggcgggcagtgcagcccctgctcctgtcgaccctgagcgttcagcgtttccgccgcctccgccccactccgtagggggagctgatgagatgaggttgaggtccaggaagacgtcaagggcttggttttgtaaacaactccattcctcgctcgctgataagttttctaagtgatgcatattcacaaccttgtcccatccaaggacccaagaattaacacattacataatatggacagccccctcctgtccaacgggcatgattttggggtctgatattctgtggatctgtgcaatagtcaac

SEQ ID NO: 21 - DNA, 450 bp, Homo sapiens
agactttttttgaaaaacggaacatctgcctatcgcaaggactactattattctgaaaatcaccttcttcattagaaagtaatatttatcattttattatagaactttgatcttacttcttgtgacttcattctgcgtagagcacactcccatccttgaattaaatgacaaagcattttatattaactgacaatgactgatgccatgggcaaatcctatttctgtaaataactgaattttcttctggactgcgcatgaggggagaaagatgtctgcagtttcggtttcctggaaaatgaaacctatctcatttgttgcctgtgtcaaggggcagtgcttcagtcggggtggagctgcttaaaaggcctgggatcacaccctttgggaacacatccaagcttaagacggtgaggtcagcttcacattctcaggaactctccttctttgggt

SEQ ID NO: 22 - DNA, 570 bp, Homo sapiens
gagactttttttgaaaaacggaacatctgcctatcgcaaggactactattattctgaaaatcaccttcttcattagaaagtaatatttatcattttattatagaactttgatcttacttcttgtgacttcattctgcgtagagcacactcccatccttgaattaaatgacaaagcattttatattaactgacaatgactgatgccatgggcaaatcctatttctgtaaataactgaattttcttctggactgcgcatgaggggagaaagatgtctgcagtttcggtttcctggaaaatgaaacctatctcatttgttgcctgtgtcaaggggcagtgcttcagtcggggtggagctgcttaaaaggcctgggatcacaccctttgggaacacatccaagcttaagacggtgaggtcagcttcacattctcaggaactctccttctttgggtaagactgggagggtgggcaggagctacccttcccgtggccccggaccttgggtgggctgtgggctcagggagcggaggggaggccttaagcatccactctctgcccggtgtttttgttc

SEQ ID NO: 23 - DNA, 513 bp, Homo sapiens
aggtggggatgaggggctaagtatgaaccaaggagctagaaatacagcactggaagctggaagcagggggcttggagactgggagctggagtgcgtgtgggcagggtgtggcagcagccggcagaggccatttccccttggcagaacattcaccatgtgaccctgagcatgtctttgaactcctctgagctcctgtttcctctccagagaaaaggctggtaatgcccattcagggttatggtcaggattgcatagggtgaaacaatagagattgaacacagtagacatgaaagagatgccagggctcagctccctttggtttagttgcttccagtgtgctctgtggcaacaccacggagccctagagctgtctctttgagccgctctgaatgtgcctcttacataatctcctgggcaacatctgctcccctaatgagatttgctccccagcaaagataagaaacttgccaaccactcccctggtccagcatttggccaaggcagacactgagg

SEQ ID NO: 24 - DNA, 217 bp, Homo sapiens
acctcactcaatgcatggaagttgacacaatggctcaacattagcgttgggctgattcatcatttggctgttgacaccagcctctggcccagccaggacagaaaaagggcccctgaggaacttctggctctgttccctctatgggggaggggcagtggacttgtgataagacagggtgttagggtgaggtggacttggggaaacaggatatttctaa

SEQ ID NO: 25 - DNA, 97 bp, Homo sapiens
ggggggaggggagaccccagaacaatgtcccccaccccacccccctcctcaataggcggaagccactggcttcctccctttcctgcctcctgcctcc

SEQ ID NO: 26 - DNA, 427 bp, Homo sapiens
gtgtgtttgtgccggggggaggggagaccccagaacaatgtcccccaccccacccccctcctcaataggcggaagccactggcttcctccctttcctgcctcctgcctcctttgtgccagcaagactgagtactggagagagacaggggatgggaaaaatcagtccagctgtccccaggtctgcccttaccataaccttccccccacctcaagtgactcctcccaggccacacccatccccagccttgtgggggccagattggggggcctagaggctcaaaggcagaatgagtcctcccaccccctaccctgccacccctcccacccaagccacctcatttcctcttcctccccagcaccgacccacactgaccaacacaggctgagcagtcaggcccacagcatctgaccccaggcccagctcgtc

SEQ ID NO: 27 - DNA, 119 bp, Homo sapiens
ctacaaagctttatcagcttggaggtacttctaataccatttcctttcattgtttccttttggtaattaaaaggaggccaatcccctgttgtggcagctcacagctattgtggtgggaa

SEQ ID NO: 28 - DNA, 385 bp, Homo sapiens
ctgccaggaggtctccctccaaactctacaaagctttatcagcttggaggtacttctaataccatttcctttcattgtttccttttggtaattaaaaggaggccaatcccctgttgtggcagctcacagctattgtggtgggaaagggagggtggttggtggatgtcacagcttgggctttatctcccccagcagtggggactccacagcccctgggctacataacagcaagacagtccggagctgtagcagacctgattgagcctttgcagcagctgagagcatggcctagggtgggcggcaccattgtccagcagctgagtttcccagggaccttggagatagccgcagccctcatttgcaggggaaggtatggcctttggaa

SEQ ID NO: 29 - DNA, 517 bp, Homo sapiens
gccattggctggtccttcactgacagcagaaacttggccaatggcaatcaatcagggggcccgcgctgccttaaataccagcagagcaaacagcctcagacaaagctgcgccgtgtatcaattaccgagaggctgcgtgctcctctgggcggagggagccggagcgagcggccagggctgctgccccagctgataagggcccgcattgttcggggacagctggcagcccgataagggcctgctcgcccgagataatggcagtgggcaggcgcctcgcggcagtttagaatttcttgggtctccaagaaaggttctattaagcccactgaccccaattgaatattaattagctaattaacggatttattgttccacgccatttctggagaggccattttttttcgagtgccattatttttgtaaatgatttttcgcattgttcataattgaatctttgcagctgccagcatcttctgcatgatttggcaaaaaaaaggaagcagaagcacttagggtt

SEQ ID NO: 30 - DNA, 511 bp, Homo sapiens
cccctaataaacaggaaggcatccgcgccattagtatccatccttttcagagcatctgagacctgtctggaccatcaaagccatccccagcccccaggagcctactggaggagacaccagcctcgccaaaacaattctccattgtgttcttccccttagaaatcatgggtttgtaaacaggcccttacatttcagcaggtcctgccctggctttgtgctggtgtgttgttttttcttccctgaacaatgtcctttccagtagggccagccgttcacaccattgtctgagacccttggactacaggaaacatcaccagattcttatcagttgggggcaggagtgggggggtgaacagatgagatcatgtccacagagcaagtggctggtgtgccacgtcattccccatgccttcatctgtgagagcagagcccgctcgccctccatcaatctgggcttcatgtgtccagagtccagtcccctctatttggtggtagacacctggactctgtt

SEQ ID NO: 31 - DNA, 390 bp, Homo sapiens
tcctacagttatgggtctgtctttcctgctagatcagaagctccagggacctgtctgtcttattaacctttcttcccctcatgatgcctggcccaggactccacgttcagaggcagtttaatgtctacagaactgatggatgctccataccctgtattcataagcctgtgttttgctgccaaacaccagagggcactgttagcatgtcgatgaagattataaaccctcagacctggaaggctgggaaaggcttatgaaaatcttgcttctgttttgggattacataagacttattgcgcctcaattgttctaaacacatctgttcgagtttattcatgaggcacgttcctgttggggttagagatgagtttgaaagctccccgtcacagg

SEQ ID NO: 32 - DNA, 573 bp, Homo sapiens
agggactgttgggcagccccagactggcacaggtggatcgggtgcctaggcagggggtggtgagttatggcgcagctgtcttggtggctggggggagcagggataagggtggacttcttagtgaccgctctctgccccaggaggtagagtcctgggggctgggctggcctgagagacgccccctcatcctttccagggtgaggtacgagggctccgccccctcctgatatcaccaggcctagggcagcatcctgatgggggaggggcaagtgacccgggccctggactgcaggaacagcccctcctccactggtggagttcccacttcctgcggaaggaactatgttagaagttgtgtatatggggtgggggttgggtgtgggtggcggggggcctgggtggggtccactgagtcgcctcccctgtctccctgcacttcctcctggaggaaatggggacaacaggatgaagtgagggcctgctgagcccagggctgccacctgggagtgaagccggggcaggctgcagggtccgggcccttctgtgtgggcaggtggaagtggtggggatgca

SEQ ID NO: 33 - DNA, 441 bp, Homo sapiens
ggggagagggtgtggggtggggtggggagagggtgtggggtggggtggggagaggggatgggatggcatggggggatgtggcagtgaggaggctgggcccttggagctgccgagtgcaggggcctggaggactccgggaaggcgtcctagtgcatcaagcgtgggcttggcctgcttgggtctcccctcctggcccccctagcaatgggcggacttgggcccgctctgggaggattccaggaacggctcctgcctggttataaatagacttctccgaaaggcctggggctgtgccagctgcagcaggtgcctcccaggcccggccagagggccccaggcaagggggtggagcccgggtgggggtgatgaggatgctggggtccacttttgtagcgccagaggcgacgggctctgtctggttgtagcatcacagagcttgat

SEQ ID NO: 34 - DNA, 1303 bp, Homo sapiens
gcttgcccagctatataataaaacaagtttgggacttcccaaccattcacccatggaaaaacagaagcaactcttcaaaggacagattcccaggatctgccctgggagattccaaatcagttgatctggggtgagcccagtcctctgtagtttttagaagctcctcctatgtctctcctggtcagcagaatcttggcccctcccttccccccagcctcttggttcttctgggctctgatccagcctcagcgtcactgtcttccacgcccctctttgattctcgtttatgtcaaaagccttgtgaggatgaggctgtgattatccccattttacagatgaggaaactgtggctccaggatgacacaactggccagaggtcacatcagaagcagagctgggtcacttgactccacccaatatccctaaatgcaaacatcccctacagaccgaggctggcaccttagagctggagtccatgcccgctctgaccaggagaagccaacctggtcctccagagccaagagcttctgtccctttcccatctcctgaagcctccctgtcacctttaaagtccattcccacaaagacatcatgggatcaccacagaaaatcaagctctggggctaggctgaccccagctagatttttggctcttttataccccagctgggtggacaagcaccttaaacccgctgagcctcagcttcccgggctataaaatgggggtgatgacacctgcctgtagcattccaaggagggttaaatgtgatgctgcagccaagggtccccacagccaggctctttgcaggtgctgggttcagagtcccagagctgaggccgggagtaggggttcaagtggggtgccccaggcagggtccagtgccagccctctgtggagacagccatccggggccgaggcagccgcccaccgcagggcctgcctatctgcagccagcccagccctcacaaaggaacaataacaggaaaccatcccagggggaagtgggccagggccagctggaaaacctgaaggggaggcagccaggcctccctcgccagcggggtgtggctcccctccaaagacggtcggctgacaggctccacagagctccactcacgctcagccctggacggacaggcagtccaacggaacagaaacatccctcagcccacaggcacggtgagtgggggctcccacactcccctccaccccaaacccgccaccctgcgcccaagatgggagggtcctcagcttccccatctgtagaatgggcatcgtcccactcccatgacagagaggctc

SEQ ID NO: 35 - DNA, 455 bp, Homo sapiens; identical to SEQ ID NO: 9

SEQ ID NO: 36 - DNA, 888 bp, Homo sapiens
cgccttgctgtgccactttgggacttccctccctagcctgagcttcagttttcctgcctgttaggcagccccatgtcaactgcacttagtaggccgggtttgatgcccgacaagacgtgaagtggtggaggtgggcaggatcccagcgctaccatcttcttgaaccagtgatctcaacacatcggatttctgtttcctcatctgcaaaatgggatcagtgagctcaggtgggtcacaaattctacaggaactactttagccaagcccggccccctgaaagttcccctcggtgggctgttagggtgattgttttcatctgtggggctccctgatgcgtcccacccaccagccttggagagggtgggatgggagggtggggtgcttggggagacaagcctagagcctgggccctcccaccccactgcctccccccatcccagggccccccacccagtgacaaagcccgtggcacttcctctacccggttggcaggcggcctggcccagccccttctctaaggaagcgcatttcctgcctccctgggccggccgggctggatgagccgggagctccctgctgccggtcataccacagccttcatctgcgccctggggccaggactgctgctgtcactgccatccattggagcccagcaccccctccccgcccatccttcggacagcaactccagcccagccccgcgtccctgtgtccacttctcctgacccctcggccgccaccccagaaggctggagcagggacgccgtcgctccggccgcctgctcccctcgggtccccgtgcgagcccacgccggccccggtgcccgcccgcagccctgccactggacacaggataaggcccagcgcacaggcccccacgtggacacc

SEQ ID NO: 37 - DNA, 1037 bp, Homo sapiens
tttgcttctaggaagcagaagactgaggaaatgacttgggcgggtgcatcaatgcggccaaaaaagacacggacacgctcccctgggacctgagctggttcgcagtcttcccaaaggtgccaagcaagcgtcagttcccctcaggcgctccaggttcagtgccttgtgccgagggtctccggtgccttcctagacttctcgggacagtctgaaggggtcaggagcggcgggacagcgcgggaagagcaggcaaggggagacagccggactgcgcctcagtcctccgtgccaagaacaccgtcgcggaggcgcggccagcttcccttggatcggactttccgcccctagggccaggcggcggagcttcagccttgtcccttccccagtttcgggcggcccccagagctgagtaagccgggtggagggagtctgcaaggatttcctgagcgcgatgggcaggaggaggggcaagggcaagagggcgcggagcaaagaccctgaacctgccggggccgcgctcccgggcccgcgtcgccagcacctccccacgcgcgctcggccccgggccacccgccctcgtcggcccccgcccctctccgtagccgcagggaagcgagcctgggaggaagaagagggtaggtggggaggcggatgaggggtgggggaccccttgacgtcaccagaaggaggtgccggggtaggaagtgggctggggaaaggttataaatcgcccccgccctcggctgctcttcatcgaggtccgcgggaggctcggagcgcgccaggcggacactcctctcggctcctccccggcagcggcggcggctcggagcgggctccggggctcgggtgcagcggccagcgggcgcctggcggcgaggattacccggggaagtggttgtctcctggctggagccgcgagacgggcgctcagggcgcggggccggcggcggcgaacaagaggacggactctggcggccgggtcgttggccgcggggagcgcgggcaccgggcgagcaggccgcgtcgcgctcacc

SEQ ID NO: 38 - DNA, 399 bp, Homo sapiens
gtctcccaggcatgactccaacaatgcatcccatgggatttggggttccccagatctggggcttgtaggcctgactctcccctgtgcacacgtctcatacacgcatgcgtgcacccattgcctgccccgccccttgcacagggagtcagcagggaggactgggttatgccctgcttatcagcagcttcccagcttcctctgcctggattcttagaggcctggggtcctagaacgagctggtgcacgtggcttcccaaagatctctcagataatgagaggaaatgcagtcatcagtttgcagaaggctagggattctgggccatagctcagacctgcgcccaccatctccctccaggcagcccttggctggtccctgcgagcccgtggagactgccagtc

SEQ ID NO: 39 - DNA, 6 bp, Homo sapiens
gccacc

SEQ ID NO: 40 - DNA, 8834 bp, Artificial Sequence
  vector
tggaagggctaattcactcccaaagaagacaagatatccttgatctgtggatctaccacacacaaggctacttccctgattagcagaactacacaccagggccaggggtcagatatccactgacctttggatggtgctacaagctagtaccagttgagccagataaggtagaagaggccaataaaggagagaacaccagcttgttacaccctgtgagcctgcatgggatggatgacccggagagagaagtgttagagtggaggtttgacagccgcctagcatttcatcacgtggcccgagagctgcatccggagtacttcaagaactgctgatatcgagcttgctacaagggactttccgctggggactttccagggaggcgtggcctgggcgggactggggagtggcgagccctcagatcctgcatataagcagctgctttttgcctgtactgggtctctctggttagaccagatctgagcctgggagctctctggctaactagggaacccactgcttaagcctcaataaagcttgccttgagtgcttcaagtagtgtgtgcccgtctgttgtgtgactctggtaactagagatccctcagacccttttagtcagtgtggaaaatctctagcagtggcgcccgaacagggacttgaaagcgaaagggaaaccagaggagctctctcgacgcaggactcggcttgctgaagcgcgcacggcaagaggcgaggggcggcgactggtgagtacgccaaaaattttgactagcggaggctagaaggagagagatgggtgcgagagcgtcagtattaagcgggggagaattagatcgcgatgggaaaaaattcggttaaggccagggggaaagaaaaaatataaattaaaacatatagtatgggcaagcagggagctagaacgattcgcagttaatcctggcctgttagaaacatcagaaggctgtagacaaatactgggacagctacaaccatcccttcagacaggatcagaagaacttagatcattatataatacagtagcaaccctctattgtgtgcatcaaaggatagagataaaagacaccaaggaagctttagacaagatagaggaagagcaaaacaaaagtaagaccaccgcacagcaagcggccggccgctgatcttcagacctggaggaggagatatgagggacaattggagaagtgaattatataaatataaagtagtaaaaattgaaccattaggagtagcacccaccaaggcaaagagaagagtggtgcagagagaaaaaagagcagtgggaataggagctttgttccttgggttcttgggagcagcaggaagcactatgggcgcagcgtcaatgacgctgacggtacaggccagacaattattgtctggtatagtgcagcagcagaacaatttgctgagggctattgaggcgcaacagcatctgttgcaactcacagtctggggcatcaagcagctccaggcaagaatcctggctgtggaaagatacctaaaggatcaacagctcctggggatttggggttgctctggaaaactcatttgcaccactgctgtgccttggaatgctagttggagtaataaatctctggaacagatttggaatcacacgacctggatggagtgggacagagaaattaacaattacacaagcttaatacactccttaattgaagaatcgcaaaaccagcaagaaaagaatgaacaagaattattggaattagataaatgggcaagtttgtggaattggtttaacataacaaattggctgtggtatataaaattattcataatgatagtaggaggcttggtaggtttaagaatagtttttgctgtactttctatagtgaatagagttaggcagggatattcaccattatcgtttcagacccacctcccaaccccgaggggacccgacaggcccgaaggaatagaagaagaaggtggagagagagacagagacagatccattcgattagtgaacggatctcgacggtatcgcctttaaaagaaaaggggggattggggggtacagtgcaggggaaagaatagtagacataatagcaacagacatacaaactaaagaactacaaaaacaaattacaaaaattcaaaattttcgggtttattacagggacagcagagatccagtttatcgataagcttgggagttccgcgttacataacttacggtaaatggcccgcctggctgaccgcccaacgacccccgcccattgacgtcaataatgacgtatgttcccatagtaacgccaatagggactttccattgacgtcaatgggtggagtatttacggtaaactgcccacttggcagtacatcaagtgtatcatatgccaagtacgccccctattgacgtcaatgacggtaaatggcccgcctggcattatgcccagtacatgaccttacgggactttcctacttggcagtacatctacgtattagtcatcgctattaccatggtgatgcggttttggcagtacaccaatgggcgtggatagcggtttgactcacggggatttccaagtctccaccccattgacgtcaatgggagtttgttttggcaccaaaatcaacgggactttccaaaatgtcgtaacaactccgccccattgacgcaaatgggcggtaggcgtgtacggtgggaggtctatataagcagagctcgtttagtgaaccgtcagatcgcctggagacgccatccacgctgttttgacctccatagaagacaccgactctagctagaggatctaccggtcgccaccatggtgagcaagggcgccgagctgttcaccggcatcgtgcccatcctgatcgagctgaatggcgatgtgaatggccacaagttcagcgtgagcggcgagggcgagggcgatgccacctacggcaagctgaccctgaagttcatctgcaccaccggcaagctgcctgtgccctggcccaccctggtgaccaccctgagctacggcgtgcagtgcttctcacgctaccccgatcacatgaagcagcacgacttcttcaagagcgccatgcctgagggctacatccaggagcgcaccatcttcttcgaggatgacggcaactacaagtcgcgcgccgaggtgaagttcgagggcgataccctggtgaatcgcatcgagctgaccggcaccgatttcaaggaggatggcaacatcctgggcaataagatggagtacaactacaacgcccacaatgtgtacatcatgaccgacaaggccaagaatggcatcaaggtgaacttcaagatccgccacaacatcgaggatggcagcgtgcagctggccgaccactaccagcagaatacccccatcggcgatggccctgtgctgctgcccgataaccactacctgtccacccagagcgccctgtccaaggaccccaacgagaagcgcgatcacatgatctacttcggcttcgtgaccgccgccgccatcacccacggcatggatgagctgtacaagtccggactcagatctcgagctcaagcttcgaattctgcagtcgacggtaccgcgggcccgggatccaccggatctagataactgatcataattctaccgggtaggggaggcgcttttcccaaggcagtctggagcatgcgctttagcagccccgctgggcacttggcgctacacaagtggcctctggcctcgcacacattccacatccaccggtaggcgccaaccggctccgttctttggtggccccttcgcgccaccttctactcctcccctagtcaggaagttcccccccgccccgcagctcgcgtcgtgcaggacgtgacaaatggaagtagcacgtctcactagtctcgtgcagatggacagcaccgctgagcaatggaagcgggtaggcctttggggcagcggccaatagcagctttgctccttcgctttctgggctcagaggctgggaaggggtgggtccgggggcgggctcaggggcgggctcaggggcggggcgggcgcccgaaggtcctccggaggcccggcattctgcacgcttcaaaagcgcacgtctgccgcgctgttctcctcttcctcatctccgggcctttcgacctgcagcccaagcttaccatgaccgagtacaagcccacggtgcgcctcgccacccgcgacgacgtccccagggccgtacgcaccctcgccgccgcgttcgccgactaccccgccacgcgccacaccgtcgatccggaccgccacatcgagcgggtcaccgagctgcaagaactcttcctcacgcgcgtcgggctcgacatcggcaaggtgtgggtcgcggacgacggcgccgcggtggcggtctggaccacgccggagagcgtcgaagcgggggcggtgttcgccgagatcggcccgcgcatggccgagttgagcggttcccggctggccgcgcagcaacagatggaaggcctcctggcgccgcaccggcccaaggagcccgcgtggttcctggccaccgtcggcgtctcgcccgaccaccagggcaagggtctgggcagcgccgtcgtgctccccggagtggaggcggccgagcgcgccggggtgcccgccttcctggagacctccgcgccccgcaacctccccttctacgagcggctcggcttcaccgtcaccgccgacgtcgaggtgcccgaaggaccgcgcacctggtgcatgacccgcaagcccggtgcctgaccgcgtctggaacaatcaacctctggattacaaaatttgtgaaagattgactggtattcttaactatgttgctccttttacgctatgtggatacgctgctttaatgcctttgtatcatgctattgcttcccgtatggctttcattttctcctccttgtataaatcctggttgctgtctctttatgaggagttgtggcccgttgtcaggcaacgtggcgtggtgtgcactgtgtttgctgacgcaacccccactggttggggcattgccaccacctgtcagctcctttccgggactttcgctttccccctccctattgccacggcggaactcatcgccgcctgccttgcccgctgctggacaggggctcggctgttgggcactgacaattccgtggtgttgtcggggaagctgacgtcctttccatggctgctcgcctgtgttgccacctggattctgcgcgggacgtccttctgctacgtcccttcggccctcaatccagcggaccttccttcccgcggcctgctgccggctctgcggcctcttccgcgtcttcgccttcgccctcagacgagtcggatctccctttgggccgcctccccgcctggaattaattctgcagtcgagacctagaaaaacatggagcaatcacaagtagcaatacagcagctaccaatgctgattgtgcctggctagaagcacaagaggaggaggaggtgggtttttccagtcacacctcaggtacctttaagaccaatgacttacaaggcagctgtagatcttagccactttttaaaagaaaagaggggactggaagggctaattcactcccaacgaagacaagatatccttgatctgtggatctaccacacacaaggctacttccctgattagcagaactacacaccagggccaggggtcagatatccactgacctttggatggtgctacaagctagtaccagttgagccagataaggtagaagaggccaataaaggagagaacaccagcttgttacaccctgtgagcctgcatgggatggatgacccggagagagaagtgttagagtggaggtttgacagccgcctagcatttcatcacgtggcccgagagctgcatccggagtacttcaagaactgctgatatcgagcttgctacaagggactttccgctggggactttccagggaggcgtggcctgggcgggactggggagtggcgagccctcagatcctgcatataagcagctgctttttgcctgtactgggtctctctggttagaccagatctgagcctgggagctctctggctaactagggaacccactgcttaagcctcaataaagcttgccttgagtgcttcaagtagtgtgtgcccgtctgttgtgtgactctggtaactagagatccctcagacccttttagtcagtgtggaaaatctctagcagtagtagttcatgtcatcttattattcagtatttataacttgcaaagaaatgaatatcagagagtgagaggccttgacattgctagcgttttaccgtcgacctctagctagagcttggcgtaatcatggtcatagctgtttcctgtgtgaaattgttatccgctcacaattccacacaacatacgagccggaagcataaagtgtaaagcctggggtgcctaatgagtgagctaactcacattaattgcgttgcgctcactgcccgctttccagtcgggaaacctgtcgtgccagctgcattaatgaatcggccaacgcgcggggagaggcggtttgcgtattgggcgctcttccgcttcctcgctcactgactcgctgcgctcggtcgttcggctgcggcgagcggtatcagctcactcaaaggcggtaatacggttatccacagaatcaggggataacgcaggaaagaacatgtgagcaaaaggccagcaaaaggccaggaaccgtaaaaaggccgcgttgctggcgtttttccataggctccgcccccctgacgagcatcacaaaaatcgacgctcaagtcagaggtggcgaaacccgacaggactataaagataccaggcgtttccccctggaagctccctcgtgcgctctcctgttccgaccctgccgcttaccggatacctgtccgcctttctcccttcgggaagcgtggcgctttctcatagctcacgctgtaggtatctcagttcggtgtaggtcgttcgctccaagctgggctgtgtgcacgaaccccccgttcagcccgaccgctgcgccttatccggtaactatcgtcttgagtccaacccggtaagacacgacttatcgccactggcagcagccactggtaacaggattagcagagcgaggtatgtaggcggtgctacagagttcttgaagtggtggcctaactacggctacactagaagaacagtatttggtatctgcgctctgctgaagccagttaccttcggaaaaagagttggtagctcttgatccggcaaacaaaccaccgctggtagcggtttttttgtttgcaagcagcagattacgcgcagaaaaaaaggatctcaagaagatcctttgatcttttctacggggtctgacgctcagtggaacgaaaactcacgttaagggattttggtcatgagattatcaaaaaggatcttcacctagatccttttaaattaaaaatgaagttttaaatcaatctaaagtatatatgagtaaacttggtctgacagttaccaatgcttaatcagtgaggcacctatctcagcgatctgtctatttcgttcatccatagttgcctgactccccgtcgtgtagataactacgatacgggagggcttaccatctggccccagtgctgcaatgataccgcgagacccacgctcaccggctccagatttatcagcaataaaccagccagccggaagggccgagcgcagaagtggtcctgcaactttatccgcctccatccagtctattaattgttgccgggaagctagagtaagtagttcgccagttaatagtttgcgcaacgttgttgccattgctacaggcatcgtggtgtcacgctcgtcgtttggtatggcttcattcagctccggttcccaacgatcaaggcgagttacatgatcccccatgttgtgcaaaaaagcggttagctccttcggtcctccgatcgttgtcagaagtaagttggccgcagtgttatcactcatggttatggcagcactgcataattctcttactgtcatgccatccgtaagatgcttttctgtgactggtgagtactcaaccaagtcattctgagaatagtgtatgcggcgaccgagttgctcttgcccggcgtcaatacgggataataccgcgccacatagcagaactttaaaagtgctcatcattggaaaacgttcttcggggcgaaaactctcaaggatcttaccgctgttgagatccagttcgatgtaacccactcgtgcacccaactgatcttcagcatcttttactttcaccagcgtttctgggtgagcaaaaacaggaaggcaaaatgccgcaaaaaagggaataagggcgacacggaaatgttgaatactcatactcttcctttttcaatattattgaagcatttatcagggttattgtctcatgagcggatacatatttgaatgtatttagaaaaataaacaaataggggttccgcgcacatttccccgaaaagtgccacctgacgtcgacggatcgggagatcaacttgtttattgcagcttataatggttacaaataaagcaatagcatcacaaatttcacaaataaagcatttttttcactgcattctagttgtggtttgtccaaactcatcaatgtatcttatcatgtctggatcaactggataactcaagctaaccaaaatcatcccaaacttcccaccccataccctattaccactgccaattacctagtggtttcatttactctaaacctgtgattcctctgaattattttcattttaaagaaattgtatttgttaaatatgtactacaaacttagtagtttttaaagaaattgtatttgttaaatatgtactacaaacttagtagt

SEQ ID NO: 41 - DNA, 11329 bp, Artificial Sequence
  vector
tggaagggctaattcactcccaaagaagacaagatatccttgatctgtggatctaccacacacaaggctacttccctgattagcagaactacacaccagggccaggggtcagatatccactgacctttggatggtgctacaagctagtaccagttgagccagataaggtagaagaggccaataaaggagagaacaccagcttgttacaccctgtgagcctgcatgggatggatgacccggagagagaagtgttagagtggaggtttgacagccgcctagcatttcatcacgtggcccgagagctgcatccggagtacttcaagaactgctgatatcgagcttgctacaagggactttccgctggggactttccagggaggcgtggcctgggcgggactggggagtggcgagccctcagatcctgcatataagcagctgctttttgcctgtactgggtctctctggttagaccagatctgagcctgggagctctctggctaactagggaacccactgcttaagcctcaataaagcttgccttgagtgcttcaagtagtgtgtgcccgtctgttgtgtgactctggtaactagagatccctcagacccttttagtcagtgtggaaaatctctagcagtggcgcccgaacagggacttgaaagcgaaagggaaaccagaggagctctctcgacgcaggactcggcttgctgaagcgcgcacggcaagaggcgaggggcggcgactggtgagtacgccaaaaattttgactagcggaggctagaaggagagagatgggtgcgagagcgtcagtattaagcgggggagaattagatcgcgatgggaaaaaattcggttaaggccagggggaaagaaaaaatataaattaaaacatatagtatgggcaagcagggagctagaacgattcgcagttaatcctggcctgttagaaacatcagaaggctgtagacaaatactgggacagctacaaccatcccttcagacaggatcagaagaacttagatcattatataatacagtagcaaccctctattgtgtgcatcaaaggatagagataaaagacaccaaggaagctttagacaagatagaggaagagcaaaacaaaagtaagaccaccgcacagcaagcggccggccgctgatcttcagacctggaggaggagatatgagggacaattggagaagtgaattatataaatataaagtagtaaaaattgaaccattaggagtagcacccaccaaggcaaagagaagagtggtgcagagagaaaaaagagcagtgggaataggagctttgttccttgggttcttgggagcagcaggaagcactatgggcgcagcgtcaatgacgctgacggtacaggccagacaattattgtctggtatagtgcagcagcagaacaatttgctgagggctattgaggcgcaacagcatctgttgcaactcacagtctggggcatcaagcagctccaggcaagaatcctggctgtggaaagatacctaaaggatcaacagctcctggggatttggggttgctctggaaaactcatttgcaccactgctgtgccttggaatgctagttggagtaataaatctctggaacagatttggaatcacacgacctggatggagtgggacagagaaattaacaattacacaagcttaatacactccttaattgaagaatcgcaaaaccagcaagaaaagaatgaacaagaattattggaattagataaatgggcaagtttgtggaattggtttaacataacaaattggctgtggtatataaaattattcataatgatagtaggaggcttggtaggtttaagaatagtttttgctgtactttctatagtgaatagagttaggcagggatattcaccattatcgtttcagacccacctcccaaccccgaggggacccgacaggcccgaaggaatagaagaagaaggtggagagagagacagagacagatccattcgattagtgaacggatctcgacggtatcgcctttaaaagaaaaggggggattggggggtacagtgcaggggaaagaatagtagacataatagcaacagacatacaaactaaagaattacaaaaacaaattacaaaaattcaaaattttcgggtttattacagggacagcagagatccagtttatcgataagcttgggagttccgcgttacataacttacggtaaatggcccgcctggctgaccgcccaacgacccccgcccattgacgtcaataatgacgtatgttcccatagtaacgccaatagggactttccattgacgtcaatgggtggagtatttacggtaaactgcccacttggcagtacatcaagtgtatcatatgccaagtacgccccctattgacgtcaatgacggtaaatggcccgcctggcattatgcccagtacatgaccttatgggactttcctacttggcagtacatctacgtattagtcatcgctattaccatggtgatgcggttttggcagtacatcaatgggcgtggatagcggtttgactcacggggatttccaagtctccaccccattgacgtcaatgggagtttgttttggcaccaaaatcaacgggactttccaaaatgtcgtaacaactccgccccattgacgcaaatgggcggtaggcgtgtacggtgggaggtctatataagcagagctcgtttagtgaaccgtcagatcgcctggagacgccatccacgctgttttgacctccatagaagacaccgactctactagaggatcgctagcgctaccggactcagatctcgagctcaagcttcgaattctgcagtcgacggtaccgcgggcccggatgcagatcgagctgtccacctgcttttttctgtgcctgctgcggttctgcttcagcgccacccggcggtactacctgggcgccgtggagctgtcctgggactacatgcagagcgacctgggcgagctgcccgtggacgcccggttcccccccagagtgcccaagagcttccccttcaacaccagcgtggtgtacaagaaaaccctgttcgtggagttcaccgaccacctgttcaatatcgccaagcccaggcccccctggatgggcctgctgggccccaccatccaggccgaggtgtacgacaccgtggtgatcaccctgaagaacatggccagccaccccgtgagcctgcacgccgtgggcgtgagctactggaaggccagcgagggcgccgagtacgacgaccagaccagccagcgggagaaagaagatgacaaggtgttccctggcggcagccacacctacgtgtggcaggtgctgaaagaaaacggccccatggcctccgaccccctgtgcctgacctacagctacctgagccacgtggacctggtgaaggacctgaacagcggcctgatcggcgctctgctcgtctgccgggagggcagcctggccaaagagaaaacccagaccctgcacaagttcatcctgctgttcgccgtgttcgacgagggcaagagctggcacagcgagacaaagaacagcctgatgcaggaccgggacgccgcctctgccagagcctggcccaagatgcacaccgtgaacggctacgtgaacagaagcctgcccggcctgattggctgccaccggaagagcgtgtactggcacgtgatcggcatgggcaccacacccgaggtgcacagcatctttctggaagggcacacctttctggtccggaaccaccggcaggccagcctggaaatcagccctatcaccttcctgaccgcccagacactgctgatggacctgggccagttcctgctgttttgccacatcagctctcaccagcacgacggcatggaagcctacgtgaaggtggactcttgccccgaggaaccccagctgcggatgaagaacaacgaggaagccgaggactacgacgacgacctgaccgacagcgagatggacgtggtgcggttcgacgacgacaacagccccagcttcatccagatcagaagcgtggccaagaagcaccccaagacctgggtgcactatatcgccgccgaggaagaggactgggactacgcccccctggtgctggcccccgacgacagaagctacaagagccagtacctgaacaatggcccccagcggatcggccggaagtacaagaaagtgcggttcatggcctacaccgacgagacattcaagacccgggaggccatccagcacgagagcggcatcctgggccccctgctgtacggcgaagtgggcgacacactgctgatcatcttcaagaaccaggctagccggccctacaacatctacccccacggcatcaccgacgtgcggcccctgtacagcaggcggctgcccaagggcgtgaagcacctgaaggacttccccatcctgcccggcgagatcttcaagtacaagtggaccgtgaccgtggaggacggccccaccaagagcgaccccagatgcctgacccggtactacagcagcttcgtgaacatggaacgggacctggcctccgggctgatcggacctctgctgatctgctacaaagaaagcgtggaccagcggggcaaccagatcatgagcgacaagcggaacgtgatcctgttcagcgtgttcgatgagaaccggtcctggtatctgaccgagaacatccagcggtttctgcccaaccctgccggcgtgcagctggaagatcccgagttccaggccagcaacatcatgcactccatcaatggctacgtgttcgactctctgcagctctccgtgtgtctgcacgaggtggcctactggtacatcctgagcatcggcgcccagaccgacttcctgagcgtgttcttcagcggctacaccttcaagcacaagatggtgtacgaggacaccctgaccctgttccctttcagcggcgagacagtgttcatgagcatggaaaaccccggcctgtggattctgggctgccacaacagcgacttccggaaccggggcatgaccgccctgctgaaggtgtccagctgcgacaagaacaccggcgactactacgaggacagctacgaggatatcagcgcctacctgctgtccaagaacaacgccatcgaaccccggagcttcagccagaacccccccgtgctgacgcgtcaccagcgggagatcacccggacaaccctgcagtccgaccaggaagagatcgattacgacgacaccatcagcgtggagatgaagaaagaggatttcgatatctacgacgaggacgagaaccagagccccagaagcttccagaagaaaacccggcactacttcattgccgccgtggagaggctgtgggactacggcatgagttctagcccccacgtgctgcggaaccgggcccagagcggcagcgtgccccagttcaagaaagtggtgttccaggaattcacagacggcagcttcacccagcctctgtatagaggcgagctgaacgagcacctggggctgctggggccctacatcagggccgaagtggaggacaacatcatggtgaccttccggaatcaggccagcagaccctactccttctacagcagcctgatcagctacgaagaggaccagcggcagggcgccgaaccccggaagaacttcgtgaagcccaacgaaaccaagacctacttctggaaagtgcagcaccacatggcccccaccaaggacgagttcgactgcaaggcctgggcctacttcagcgacgtggatctggaaaaggacgtgcactctggactgattggcccactcctggtctgccacactaacaccctcaaccccgcccacggccgccaggtgaccgtgcaggaattcgccctgttcttcaccatcttcgacgagacaaagtcctggtacttcaccgagaatatggaacggaactgcagagccccctgcaacatccagatggaagatcctaccttcaaagagaactaccggttccacgccatcaacggctacatcatggacaccctgcctggcctggtgatggcccaggaccagagaatccggtggtatctgctgtccatgggcagcaacgagaatatccacagcatccacttcagcggccacgtgttcaccgtgcggaagaaagaagagtacaagatggccctgtacaacctgtaccccggcgtgttcgagacagtggagatgctgcccagcaaggccggcatctggcgggtggagtgtctgatcggcgagcacctgcacgctggcatgagcaccctgtttctggtgtacagcaacaagtgccagaccccactgggcatggcctctggccacatccgggacttccagatcaccgcctccggccagtacggccagtgggcccccaagctggccagactgcactacagcggcagcatcaacgcctggtccaccaaagagcccttcagctggatcaaggtggacctgctggcccctatgatcatccacggcattaagacccagggcgccaggcagaagttcagcagcctgtacatcagccagttcatcatcatgtacagcctggacggcaagaagtggcagacctaccggggcaacagcaccggcaccctgatggtgttcttcggcaatgtggacagcagcggcatcaagcacaacatcttcaacccccccatcattgcccggtacatccggctgcaccccacccactacagcattagatccacactgagaatggaactgatgggctgcgacctgaactcctgcagcatgcctctgggcatggaaagcaaggccatcagcgacgcccagatcacagccagcagctacttcaccaacatgttcgccacctggtccccctccaaggccaggctgcacctgcagggccggtccaacgcctggcggcctcaggtcaacaaccccaaagaatggctgcaggtggactttcagaaaaccatgaaggtgaccggcgtgaccacccagggcgtgaaaagcctgctgaccagcatgtacgtgaaagagtttctgatcagcagctctcaggatggccaccagtggaccctgttctttcagaacggcaaggtgaaagtgttccagggcaaccaggactccttcacccccgtggtgaactccctggacccccccctgctgacccgctacctgagaatccacccccagtcttgggtgcaccagatcgccctcaggatggaagtcctgggatgtgaggcccaggatctgtactgatgacgtctggaacaatcaacctctggattacaaaatttgtgaaagattgactggtattcttaactatgttgctccttttacgctatgtggatacgctgctttaatgcctttgtatcatgctattgcttcccgtatggctttcattttctcctccttgtataaatcctggttgctgtctctttatgaggagttgtggcccgttgtcaggcaacgtggcgtggtgtgcactgtgtttgctgacgcaacccccactggttggggcattgccaccacctgtcagctcctttccgggactttcgctttccccctccctattgccacggcggaactcatcgccgcctgccttgcccgctgctggacaggggctcggctgttgggcactgacaattccgtggtgttgtcggggaagctgacgtcctttccatggctgctcgcctgtgttgccacctggattctgcgcgggacgtccttctgctacgtcccttcggccctcaatccagcggaccttccttcccgcggcctgctgccggctctgcggcctcttccgcgtcttcgccttcgccctcagacgagtcggatctccctttgggccgcctccccgcctggaattaattctgcagtcgagacctagaaaaacatggagcaatcacaagtagcaatacagcagctaccaatgctgattgtgcctggctagaagcacaagaggaggaggaggtgggttttccagtcacacctcaggtacctttaagaccaatgacttacaaggcagctgtagatcttagccactttttaaaagaaaagaggggactggaagggctaattcactcccaacgaagacaagatatccttgatctgtggatctaccacacacaaggctacttccctgattagcagaactacacaccagggccaggggtcagatatccactgacctttggatggtgctacaagctagtaccagttgagccagataaggtagaagaggccaataaaggagagaacaccagcttgttacaccctgtgagcctgcatgggatggatgacccggagagagaagtgttagagtggaggtttgacagccgcctagcatttcatcacgtggcccgagagctgcatccggagtacttcaagaactgctgatatcgagcttgctacaagggactttccgctggggactttccagggaggcgtggcctgggcgggactggggagtggcgagccctcagatcctgcatataagcagctgctttttgcctgtactgggtctctctggttagaccagatctgagcctgggagctctctggctaactagggaacccactgcttaagcctcaataaagcttgccttgagtgcttcaagtagtgtgtgcccgtctgttgtgtgactctggtaactagagatccctcagacccttttagtcagtgtggaaaatctctagcagtagtagttcatgtcatcttattattcagtatttataacttgcaaagaaatgaatatcagagagtgagaggccttgacattgctagcgttttaccgtcgacctctagctagagcttggcgtaatcatggtcatagctgtttcctgtgtgaaattgttatccgctcacaattccacacaacatacgagccggaagcataaagtgtaaagcctggggtgcctaatgagtgagctaactcacattaattgcgttgcgctcactgcccgctttccagtcgggaaacctgtcgtgccagctgcattaatgaatcggccaacgcgcggggagaggcggtttgcgtattgggcgctcttccgcttcctcgctcactgactcgctgcgctcggtcgttcggctgcggcgagcggtatcagctcactcaaaggcggtaatacggttatccacagaatcaggggataacgcaggaaagaacatgtgagcaaaaggccagcaaaaggccaggaaccgtaaaaaggccgcgttgctggcgtttttccataggctccgcccccctgacgagcatcacaaaaatcgacgctcaagtcagaggtggcgaaacccgacaggactataaagataccaggcgtttccccctggaagctccctcgtgcgctctcctgttccgaccctgccgcttaccggatacctgtccgcctttctcccttcgggaagcgtggcgctttctcatagctcacgctgtaggtatctcagttcggtgtaggtcgttcgctccaagctgggctgtgtgcacgaaccccccgttcagcccgaccgctgcgccttatccggtaactatcgtcttgagtccaacccggtaagacacgacttatcgccactggcagcagccactggtaacaggattagcagagcgaggtatgtaggcggtgctacagagttcttgaagtggtggcctaactacggctacactagaagaacagtatttggtatctgcgctctgctgaagccagttaccttcggaaaaagagttggtagctcttgatccggcaaacaaaccaccgctggtagcggtggtttttttgtttgcaagcagcagattacgcgcagaaaaaaaggatctcaagaagatcctttgatcttttctacggggtctgacgctcagtggaacgaaaactcacgttaagggattttggtcatgagattatcaaaaaggatcttcacctagatccttttaaattaaaaatgaagttttaaatcaatctaaagtatatatgagtaaacttggtctgacagttaccaatgcttaatcagtgaggcacctatctcagcgatctgtctatttcgttcatccatagttgcctgactccccgtcgtgtagataactacgatacgggagggcttaccatctggccccagtgctgcaatgataccgcgagacccacgctcaccggctccagatttatcagcaataaaccagccagccggaagggccgagcgcagaagtggtcctgcaactttatccgcctccatccagtctattaattgttgccgggaagctagagtaagtagttcgccagttaatagtttgcgcaacgttgttgccattgctacaggcatcgtggtgtcacgctcgtcgtttggtatggcttcattcagctccggttcccaacgatcaaggcgagttacatgatcccccatgttgtgcaaaaaagcggttagctccttcggtcctccgatcgttgtcagaagtaagttggccgcagtgttatcactcatggttatggcagcactgcataattctcttactgtcatgccatccgtaagatgcttttctgtgactggtgagtactcaaccaagtcattctgagaatagtgtatgcggcgaccgagttgctcttgcccggcgtcaatacgggataataccgcgccacatagcagaactttaaaagtgctcatcattggaaaacgttcttcggggcgaaaactctcaaggatcttaccgctgttgagatccagttcgatgtaacccactcgtgcacccaactgatcttcagcatcttttactttcaccagcgtttctgggtgagcaaaaacaggaaggcaaaatgccgcaaaaaagggaataagggcgacacggaaatgttgaatactcatactcttcctttttcaatattattgaagcatttatcagggttattgtctcatgagcggatacatatttgaatgtatttagaaaaataaacaaataggggttccgcgcacatttccccgaaaagtgccacctgacgtcgacggatcgggagatcaacttgtttattgcagcttataatggttacaaataaagcaatagcatcacaaatttcacaaataaagcatttttttcactgcattctagttgtggtttgtccaaactcatcaatgtatcttatcatgtctggatcaactggataactcaagctaaccaaaatcatcccaaacttcccaccccataccctattaccactgccaattacctgtggtttcatttactctaaacctgtgattcctctgaattattttcattttaaagaaattgtatttgttaaatatgtactacaaacttagtagtttttaaagaaattgtatttgttaaatatgtactacaaacttagtagt

SEQ ID NO: 42 - DNA, 11220 bp, Artificial Sequence
  vector
tggaagggctaattcactcccaaagaagacaagatatccttgatctgtggatctaccacacacaaggctacttccctgattagcagaactacacaccagggccaggggtcagatatccactgacctttggatggtgctacaagctagtaccagttgagccagataaggtagaagaggccaataaaggagagaacaccagcttgttacaccctgtgagcctgcatgggatggatgacccggagagagaagtgttagagtggaggtttgacagccgcctagcatttcatcacgtggcccgagagctgcatccggagtacttcaagaactgctgatatcgagcttgctacaagggactttccgctggggactttccagggaggcgtggcctgggcgggactggggagtggcgagccctcagatcctgcatataagcagctgctttttgcctgtactgggtctctctggttagaccagatctgagcctgggagctctctggctaactagggaacccactgcttaagcctcaataaagcttgccttgagtgcttcaagtagtgtgtgcccgtctgttgtgtgactctggtaactagagatccctcagacccttttagtcagtgtggaaaatctctagcagtggcgcccgaacagggacttgaaagcgaaagggaaaccagaggagctctctcgacgcaggactcggcttgctgaagcgcgcacggcaagaggcgaggggcggcgactggtgagtacgccaaaaattttgactagcggaggctagaaggagagagatgggtgcgagagcgtcagtattaagcgggggagaattagatcgcgatgggaaaaaattcggttaaggccagggggaaagaaaaaatataaattaaaacatatagtatgggcaagcagggagctagaacgattcgcagttaatcctggcctgttagaaacatcagaaggctgtagacaaatactgggacagctacaaccatcccttcagacaggatcagaagaacttagatcattatataatacagtagcaaccctctattgtgtgcatcaaaggatagagataaaagacaccaaggaagctttagacaagatagaggaagagcaaaacaaaagtaagaccaccgcacagcaagcggccggccgctgatcttcagacctggaggaggagatatgagggacaattggagaagtgaattatataaatataaagtagtaaaaattgaaccattaggagtagcacccaccaaggcaaagagaagagtggtgcagagagaaaaaagagcagtgggaataggagctttgttccttgggttcttgggagcagcaggaagcactatgggcgcagcgtcaatgacgctgacggtacaggccagacaattattgtctggtatagtgcagcagcagaacaatttgctgagggctattgaggcgcaacagcatctgttgcaactcacagtctggggcatcaagcagctccaggcaagaatcctggctgtggaaagatacctaaaggatcaacagctcctggggatttggggttgctctggaaaactcatttgcaccactgctgtgccttggaatgctagttggagtaataaatctctggaacagatttggaatcacacgacctggatggagtgggacagagaaattaacaattacacaagcttaatacactccttaattgaagaatcgcaaaaccagcaagaaaagaatgaacaagaattattggaattagataaatgggcaagtttgtggaattggtttaacataacaaattggctgtggtatataaaattattcataatgatagtaggaggcttggtaggtttaagaatagtttttgctgtactttctatagtgaatagagttaggcagggatattcaccattatcgtttcagacccacctcccaaccccgaggggggacccgacaggcccgaaggaatagaagaagaaggtggagagagagacagagacagatccattcgattagtgaacggatctcgacggtcgccaaatggcagtattcatccacaattttaaaagaaaaggggggattggggggtacagtgcaggggaaagaatagtagacataatagcaacagacatacaaactaaagaattacaaaaacaaattacaaaaattcaaaattttcgggtttattacagggacagcagagatccagtttggatcgataagcttgatatcgaattcctgcgcggccgcttcgaacgcgcgcgatgcatcatatgcgtacgcggtctagaactagtgagacataaaaggaaaatgaagcgagcaacaattaaaaaaaattccccgcacacaacaatacaatctatttaaactgtggctcatacttttcataccaatggtatgactttttttctggagtcccctcttctgattcttgaactccggggctggcagcttgcaaaggggaagcggactccagcactgcacgggcaggtttagcaaaggtctctaatgggtattttctttttcttagccctgcccccgaattgtcagacggcgggcgtctgcctctgaagttagcagtgatttcctttcgggcctggccttatctccggctgcacgttgcctgttggtgactaataacacaataacattgtctggggctggaataaagtcggagctgtttacccccactctaataggggttcaatataaaaagccggcagagagctgtccaagtcagacgcgcctcagcgctggatccatgcagatcgagctgtccacctgcttttttctgtgcctgctgcggttctgcttcagcgccacccggcggtactacctgggcgccgtggagctgtcctgggactacatgcagagcgacctgggcgagctgcccgtggacgcccggttcccccccagagtgcccaagagcttccccttcaacaccagcgtggtgtacaagaaaaccctgttcgtggagttcaccgaccacctgttcaatatcgccaagcccaggcccccctggatgggcctgctgggccccaccatccaggccgaggtgtacgacaccgtggtgatcaccctgaagaacatggccagccaccccgtgagcctgcacgccgtgggcgtgagctactggaaggccagcgagggcgccgagtacgacgaccagaccagccagcgggagaaagaagatgacaaggtgttccctggcggcagccacacctacgtgtggcaggtgctgaaagaaaacggccccatggcctccgaccccctgtgcctgacctacagctacctgagccacgtggacctggtgaaggacctgaacagcggcctgatcggcgctctgctcgtctgccgggagggcagcctggccaaagagaaaacccagaccctgcacaagttcatcctgctgttcgccgtgttcgacgagggcaagagctggcacagcgagacaaagaacagcctgatgcaggaccgggacgccgcctctgccagagcctggcccaagatgcacaccgtgaacggctacgtgaacagaagcctgcccggcctgattggctgccaccggaagagcgtgtactggcacgtgatcggcatgggcaccacacccgaggtgcacagcatctttctggaagggcacacctttctggtccggaaccaccggcaggccagcctggaaatcagccctatcaccttcctgaccgcccagacactgctgatggacctgggccagttcctgctgttttgccacatcagctctcaccagcacgacggcatggaagcctacgtgaaggtggactcttgccccgaggaaccccagctgcggatgaagaacaacgaggaagccgaggactacgacgacgacctgaccgacagcgagatggacgtggtgcggttcgacgacgacaacagccccagcttcatccagatcagaagcgtggccaagaagcaccccaagacctgggtgcactatatcgccgccgaggaagaggactgggactacgcccccctggtgctggcccccgacgacagaagctacaagagccagtacctgaacaatggcccccagcggatcggccggaagtacaagaaagtgcggttcatggcctacaccgacgagacattcaagacccgggaggccatccagcacgagagcggcatcctgggccccctgctgtacggcgaagtgggcgacacactgctgatcatcttcaagaaccaggctagccggccctacaacatctacccccacggcatcaccgacgtgcggcccctgtacagcaggcggctgcccaagggcgtgaagcacctgaaggacttccccatcctgcccggcgagatcttcaagtacaagtggaccgtgaccgtggaggacggccccaccaagagcgaccccagatgcctgacccggtactacagcagcttcgtgaacatggaacgggacctggcctccgggctgatcggacctctgctgatctgctacaaagaaagcgtggaccagcggggcaaccagatcatgagcgacaagcggaacgtgatcctgttcagcgtgttcgatgagaaccggtcctggtatctgaccgagaacatccagcggtttctgcccaaccctgccggcgtgcagctggaagatcccgagttccaggccagcaacatcatgcactccatcaatggctacgtgttcgactctctgcagctctccgtgtgtctgcacgaggtggcctactggtacatcctgagcatcggcgcccagaccgacttcctgagcgtgttcttcagcggctacaccttcaagcacaagatggtgtacgaggacaccctgaccctgttccctttcagcggcgagacagtgttcatgagcatggaaaaccccggcctgtggattctgggctgccacaacagcgacttccggaaccggggcatgaccgccctgctgaaggtgtccagctgcgacaagaacaccggcgactactacgaggacagctacgaggatatcagcgcctacctgctgtccaagaacaacgccatcgaaccccggagcttcagccagaacccccccgtgctgacgcgtcaccagcgggagatcacccggacaaccctgcagtccgaccaggaagagatcgattacgacgacaccatcagcgtggagatgaagaaagaggatttcgatatctacgacgaggacgagaaccagagccccagaagcttccagaagaaaacccggcactacttcattgccgccgtggagaggctgtgggactacggcatgagttctagcccccacgtgctgcggaaccgggcccagagcggcagcgtgccccagttcaagaaagtggtgttccaggaattcacagacggcagcttcacccagcctctgtatagaggcgagctgaacgagcacctggggctgctggggccctacatcagggccgaagtggaggacaacatcatggtgaccttccggaatcaggccagcagaccctactccttctacagcagcctgatcagctacgaagaggaccagcggcagggcgccgaaccccggaagaacttcgtgaagcccaacgaaaccaagacctacttctggaaagtgcagcaccacatggcccccaccaaggacgagttcgactgcaaggcctgggcctacttcagcgacgtggatctggaaaaggacgtgcactctggactgattggcccactcctggtctgccacactaacaccctcaaccccgcccacggccgccaggtgaccgtgcaggaattcgccctgttcttcaccatcttcgacgagacaaagtcctggtacttcaccgagaatatggaacggaactgcagagccccctgcaacatccagatggaagatcctaccttcaaagagaactaccggttccacgccatcaacggctacatcatggacaccctgcctggcctggtgatggcccaggaccagagaatccggtggtatctgctgtccatgggcagcaacgagaatatccacagcatccacttcagcggccacgtgttcaccgtgcggaagaaagaagagtacaagatggccctgtacaacctgtaccccggcgtgttcgagacagtggagatgctgcccagcaaggccggcatctggcgggtggagtgtctgatcggcgagcacctgcacgctggcatgagcaccctgtttctggtgtacagcaacaagtgccagaccccactgggcatggcctctggccacatccgggacttccagatcaccgcctccggccagtacggccagtgggcccccaagctggccagactgcactacagcggcagcatcaacgcctggtccaccaaagagcccttcagctggatcaaggtggacctgctggcccctatgatcatccacggcattaagacccagggcgccaggcagaagttcagcagcctgtacatcagccagttcatcatcatgtacagcctggacggcaagaagtggcagacctaccggggcaacagcaccggcaccctgatggtgttcttcggcaatgtggacagcagcggcatcaagcacaacatcttcaacccccccatcattgcccggtacatccggctgcaccccacccactacagcattagatccacactgagaatggaactgatgggctgcgacctgaactcctgcagcatgcctctgggcatggaaagcaaggccatcagcgacgcccagatcacagccagcagctacttcaccaacatgttcgccacctggtccccctccaaggccaggctgcacctgcagggccggtccaacgcctggcggcctcaggtcaacaaccccaaagaatggctgcaggtggactttcagaaaaccatgaaggtgaccggcgtgaccacccagggcgtgaaaagcctgctgaccagcatgtacgtgaaagagtttctgatcagcagctctcaggatggccaccagtggaccctgttctttcagaacggcaaggtgaaagtgttccagggcaaccaggactccttcacccccgtggtgaactccctggacccccccctgctgacccgctacctgagaatccacccccagtcttgggtgcaccagatcgccctcaggatggaagtcctgggatgtgaggcccaggatctgtactgatgacgtctggaacaatcaacctctggattacaaaatttgtgaaagattgactggtattcttaactatgttgctccttttacgctatgtggatacgctgctttaatgcctttgtatcatgctattgcttcccgtatggctttcattttctcctccttgtataaatcctggttgctgtctctttatgaggagttgtggcccgttgtcaggcaacgtggcgtggtgtgcactgtgtttgctgacgcaacccccactggttggggcattgccaccacctgtcagctcctttccgggactttcgctttccccctccctattgccacggcggaactcatcgccgcctgccttgcccgctgctggacaggggctcggctgttgggcactgacaattccgtggtgttgtcggggaagctgacgtcctttccatggctgctcgcctgtgttgccacctggattctgcgcgggacgtccttctgctacgtcccttcggccctcaatccagcggaccttccttcccgcggcctgctgccggctctgcggcctcttccgcgtcttcgccttcgccctcagacgagtcggatctccctttgggccgcctccccgcctggaattaattctgcagtcgagacctagaaaaacatggagcaatcacaagtagcaatacagcagctaccaatgctgattgtgcctggctagaagcacaagaggaggaggaggtgggttttccagtcacacctcaggtacctttaagaccaatgacttacaaggcagctgtagatcttagccactttttaaaagaaaagaggggactggaagggctaattcactcccaacgaagacaagatatccttgatctgtggatctaccacacacaaggctacttccctgattagcagaactacacaccagggccaggggtcagatatccactgacctttggatggtgctacaagctagtaccagttgagccagataaggtagaagaggccaataaaggagagaacaccagcttgttacaccctgtgagcctgcatgggatggatgacccggagagagaagtgttagagtggaggtttgacagccgcctagcatttcatcacgtggcccgagagctgcatccggagtacttcaagaactgctgatatcgagcttgctacaagggactttccgctggggactttccagggaggcgtggcctgggcgggactggggagtggcgagccctcagatcctgcatataagcagctgctttttgcctgtactgggtctctctggttagaccagatctgagcctgggagctctctggctaactagggaacccactgcttaagcctcaataaagcttgccttgagtgcttcaagtagtgtgtgcccgtctgttgtgtgactctggtaactagagatccctcagacccttttagtcagtgtggaaaatctctagcagtagtagttcatgtcatcttattattcagtatttataacttgcaaagaaatgaatatcagagagtgagaggccttgacattgctagcgttttaccgtcgacctctagctagagcttggcgtaatcatggtcatagctgtttcctgtgtgaaattgttatccgctcacaattccacacaacatacgagccggaagcataaagtgtaaagcctggggtgcctaatgagtgagctaactcacattaattgcgttgcgctcactgcccgctttccagtcgggaaacctgtcgtgccagctgcattaatgaatcggccaacgcgcggggagaggcggtttgcgtattgggcgctcttccgcttcctcgctcactgactcgctgcgctcggtcgttcggctgcggcgagcggtatcagctcactcaaaggcggtaatacggttatccacagaatcaggggataacgcaggaaagaacatgtgagcaaaaggccagcaaaaggccaggaaccgtaaaaaggccgcgttgctggcgtttttccataggctccgcccccctgacgagcatcacaaaaatcgacgctcaagtcagaggtggcgaaacccgacaggactataaagataccaggcgtttccccctggaagctccctcgtgcgctctcctgttccgaccctgccgcttaccggatacctgtccgcctttctcccttcgggaagcgtggcgctttctcatagctcacgctgtaggtatctcagttcggtgtaggtcgttcgctccaagctgggctgtgtgcacgaaccccccgttcagcccgaccgctgcgccttatccggtaactatcgtcttgagtccaacccggtaagacacgacttatcgccactggcagcagccactggtaacaggattagcagagcgaggtatgtaggcggtgctacagagttcttgaagtggtggcctaactacggctacactagaagaacagtatttggtatctgcgctctgctgaagccagttaccttcggaaaaagagttggtagctcttgatccggcaaacaaaccaccgctggtagcggtggtttttttgtttgcaagcagcagattacgcgcagaaaaaaaggatctcaagaagatcctttgatcttttctacggggtctgacgctcagtggaacgaaaactcacgttaagggattttggtcatgagattatcaaaaaggatcttcacctagatccttttaaattaaaaatgaagttttaaatcaatctaaagtatatatgagtaaacttggtctgacagttaccaatgcttaatcagtgaggcacctatctcagcgatctgtctatttcgttcatccatagttgcctgactccccgtcgtgtagataactacgatacgggagggcttaccatctggccccagtgctgcaatgataccgcgagacccacgctcaccggctccagatttatcagcaataaaccagccagccggaagggccgagcgcagaagtggtcctgcaactttatccgcctccatccagtctattaattgttgccgggaagctagagtaagtagttcgccagttaatagtttgcgcaacgttgttgccattgctacaggcatcgtggtgtcacgctcgtcgtttggtatggcttcattcagctccggttcccaacgatcaaggcgagttacatgatcccccatgttgtgcaaaaaagcggttagctccttcggtcctccgatcgttgtcagaagtaagttggccgcagtgttatcactcatggttatggcagcactgcataattctcttactgtcatgccatccgtaagatgcttttctgtgactggtgagtactcaaccaagtcattctgagaatagtgtatgcggcgaccgagttgctcttgcccggcgtcaatacgggataataccgcgccacatagcagaactttaaaagtgctcatcattggaaaacgttcttcggggcgaaaactctcaaggatcttaccgctgttgagatccagttcgatgtaacccactcgtgcacccaactgatcttcagcatcttttactttcaccagcgtttctgggtgagcaaaaacaggaaggcaaaatgccgcaaaaaagggaataagggcgacacggaaatgttgaatactcatactcttcctttttcaatattattgaagcatttatcagggttattgtctcatgagcggatacatatttgaatgtatttagaaaaataaacaaataggggttccgcgcacatttccccgaaaagtgccacctgacgtcgacggatcgggagatcaacttgtttattgcagcttataatggttacaaataaagcaatagcatcacaaatttcacaaataaagcatttttttcactgcattctagttgtggtttgtccaaactcatcaatgtatcttatcatgtctggatcaactggataactcaagctaaccaaaatcatcccaaacttcccaccccataccctattaccactgccaattacctgtggtttcatttactctaaacctgtgattcctctgaattattttcattttaaagaaattgtatttgttaaatatgtactacaaacttagtagtttttaaagaaattgtatttgttaaatatgtactacaaacttagtagt

SEQ ID NO: 43 - DNA, 11236 bp, Artificial Sequence
  vector
tggaagggctaattcactcccaaagaagacaagatatccttgatctgtggatctaccacacacaaggctacttccctgattagcagaactacacaccagggccaggggtcagatatccactgacctttggatggtgctacaagctagtaccagttgagccagataaggtagaagaggccaataaaggagagaacaccagcttgttacaccctgtgagcctgcatgggatggatgacccggagagagaagtgttagagtggaggtttgacagccgcctagcatttcatcacgtggcccgagagctgcatccggagtacttcaagaactgctgatatcgagcttgctacaagggactttccgctggggactttccagggaggcgtggcctgggcgggactggggagtggcgagccctcagatcctgcatataagcagctgctttttgcctgtactgggtctctctggttagaccagatctgagcctgggagctctctggctaactagggaacccactgcttaagcctcaataaagcttgccttgagtgcttcaagtagtgtgtgcccgtctgttgtgtgactctggtaactagagatccctcagacccttttagtcagtgtggaaaatctctagcagtggcgcccgaacagggacttgaaagcgaaagggaaaccagaggagctctctcgacgcaggactcggcttgctgaagcgcgcacggcaagaggcgaggggcggcgactggtgagtacgccaaaaattttgactagcggaggctagaaggagagagatgggtgcgagagcgtcagtattaagcgggggagaattagatcgcgatgggaaaaaattcggttaaggccagggggaaagaaaaaatataaattaaaacatatagtatgggcaagcagggagctagaacgattcgcagttaatcctggcctgttagaaacatcagaaggctgtagacaaatactgggacagctacaaccatcccttcagacaggatcagaagaacttagatcattatataatacagtagcaaccctctattgtgtgcatcaaaggatagagataaaagacaccaaggaagctttagacaagatagaggaagagcaaaacaaaagtaagaccaccgcacagcaagcggccggccgctgatcttcagacctggaggaggagatatgagggacaattggagaagtgaattatataaatataaagtagtaaaaattgaaccattaggagtagcacccaccaaggcaaagagaagagtggtgcagagagaaaaaagagcagtgggaataggagctttgttccttgggttcttgggagcagcaggaagcactatgggcgcagcgtcaatgacgctgacggtacaggccagacaattattgtctggtatagtgcagcagcagaacaatttgctgagggctattgaggcgcaacagcatctgttgcaactcacagtctggggcatcaagcagctccaggcaagaatcctggctgtggaaagatacctaaaggatcaacagctcctggggatttggggttgctctggaaaactcatttgcaccactgctgtgccttggaatgctagttggagtaataaatctctggaacagatttggaatcacacgacctggatggagtgggacagagaaattaacaattacacaagcttaatacactccttaattgaagaatcgcaaaaccagcaagaaaagaatgaacaagaattattggaattagataaatgggcaagtttgtggaattggtttaacataacaaattggctgtggtatataaaattattcataatgatagtaggaggcttggtaggtttaagaatagtttttgctgtactttctatagtgaatagagttaggcagggatattcaccattatcgtttcagacccacctcccaaccccgaggggggacccgacaggcccgaaggaatagaagaagaaggtggagagagagacagagacagatccattcgattagtgaacggatctcgacggtcgccaaatggcagtattcatccacaattttaaaagaaaaggggggattggggggtacagtgcaggggaaagaatagtagacataatagcaacagacatacaaactaaagaattacaaaaacaaattacaaaaattcaaaattttcgggtttattacagggacagcagagatccagtttggatcgataagcttgatatcgaattcctgcgcggccgcttcgaacgcgcgcgatgcatcatatgcgtacgcggtctagaactagtgagacataaaaggaaaatgaagcgagcaacaattaaaaaaaattccccgcacacaacaatacaatctatttaaactgtggctcatacttttcataccaatggtatgactttttttctggagtcccctcttctgattcttgaactccggggctggcagcttgcaaaggggaagcggactccagcactgcacgggcaggtttagcaaaggtctctaatgggtattttctttttcttagccctgcccccgaattgtcagacggcgggcgtctgcctctgaagttagcagtgatttcctttcgggcctggccttatctccggctgcacgttgcctgttggtgactaataacacaataacattgtctggggctggaataaagtcggagctgtttacccccactctaataggggttcaatataaaaagccggcagagagctgtccaagtcagacgcgcctcagcgctggatctcgggctcgaggccaccatgcagatcgagctgtccacctgcttttttctgtgcctgctgcggttctgcttcagcgccacccggcggtactacctgggcgccgtggagctgtcctgggactacatgcagagcgacctgggcgagctgcccgtggacgcccggttcccccccagagtgcccaagagcttccccttcaacaccagcgtggtgtacaagaaaaccctgttcgtggagttcaccgaccacctgttcaatatcgccaagcccaggcccccctggatgggcctgctgggccccaccatccaggccgaggtgtacgacaccgtggtgatcaccctgaagaacatggccagccaccccgtgagcctgcacgccgtgggcgtgagctactggaaggccagcgagggcgccgagtacgacgaccagaccagccagcgggagaaagaagatgacaaggtgttccctggcggcagccacacctacgtgtggcaggtgctgaaagaaaacggccccatggcctccgaccccctgtgcctgacctacagctacctgagccacgtggacctggtgaaggacctgaacagcggcctgatcggcgctctgctcgtctgccgggagggcagcctggccaaagagaaaacccagaccctgcacaagttcatcctgctgttcgccgtgttcgacgagggcaagagctggcacagcgagacaaagaacagcctgatgcaggaccgggacgccgcctctgccagagcctggcccaagatgcacaccgtgaacggctacgtgaacagaagcctgcccggcctgattggctgccaccggaagagcgtgtactggcacgtgatcggcatgggcaccacacccgaggtgcacagcatctttctggaagggcacacctttctggtccggaaccaccggcaggccagcctggaaatcagccctatcaccttcctgaccgcccagacactgctgatggacctgggccagttcctgctgttttgccacatcagctctcaccagcacgacggcatggaagcctacgtgaaggtggactcttgccccgaggaaccccagctgcggatgaagaacaacgaggaagccgaggactacgacgacgacctgaccgacagcgagatggacgtggtgcggttcgacgacgacaacagccccagcttcatccagatcagaagcgtggccaagaagcaccccaagacctgggtgcactatatcgccgccgaggaagaggactgggactacgcccccctggtgctggcccccgacgacagaagctacaagagccagtacctgaacaatggcccccagcggatcggccggaagtacaagaaagtgcggttcatggcctacaccgacgagacattcaagacccgggaggccatccagcacgagagcggcatcctgggccccctgctgtacggcgaagtgggcgacacactgctgatcatcttcaagaaccaggctagccggccctacaacatctacccccacggcatcaccgacgtgcggcccctgtacagcaggcggctgcccaagggcgtgaagcacctgaaggacttccccatcctgcccggcgagatcttcaagtacaagtggaccgtgaccgtggaggacggccccaccaagagcgaccccagatgcctgacccggtactacagcagcttcgtgaacatggaacgggacctggcctccgggctgatcggacctctgctgatctgctacaaagaaagcgtggaccagcggggcaaccagatcatgagcgacaagcggaacgtgatcctgttcagcgtgttcgatgagaaccggtcctggtatctgaccgagaacatccagcggtttctgcccaaccctgccggcgtgcagctggaagatcccgagttccaggccagcaacatcatgcactccatcaatggctacgtgttcgactctctgcagctctccgtgtgtctgcacgaggtggcctactggtacatcctgagcatcggcgcccagaccgacttcctgagcgtgttcttcagcggctacaccttcaagcacaagatggtgtacgaggacaccctgaccctgttccctttcagcggcgagacagtgttcatgagcatggaaaaccccggcctgtggattctgggctgccacaacagcgacttccggaaccggggcatgaccgccctgctgaaggtgtccagctgcgacaagaacaccggcgactactacgaggacagctacgaggatatcagcgcctacctgctgtccaagaacaacgccatcgaaccccggagcttcagccagaacccccccgtgctgacgcgtcaccagcgggagatcacccggacaaccctgcagtccgaccaggaagagatcgattacgacgacaccatcagcgtggagatgaagaaagaggatttcgatatctacgacgaggacgagaaccagagccccagaagcttccagaagaaaacccggcactacttcattgccgccgtggagaggctgtgggactacggcatgagttctagcccccacgtgctgcggaaccgggcccagagcggcagcgtgccccagttcaagaaagtggtgttccaggaattcacagacggcagcttcacccagcctctgtatagaggcgagctgaacgagcacctggggctgctggggccctacatcagggccgaagtggaggacaacatcatggtgaccttccggaatcaggccagcagaccctactccttctacagcagcctgatcagctacgaagaggaccagcggcagggcgccgaaccccggaagaacttcgtgaagcccaacgaaaccaagacctacttctggaaagtgcagcaccacatggcccccaccaaggacgagttcgactgcaaggcctgggcctacttcagcgacgtggatctggaaaaggacgtgcactctggactgattggcccactcctggtctgccacactaacaccctcaaccccgcccacggccgccaggtgaccgtgcaggaattcgccctgttcttcaccatcttcgacgagacaaagtcctggtacttcaccgagaatatggaacggaactgcagagccccctgcaacatccagatggaagatcctaccttcaaagagaactaccggttccacgccatcaacggctacatcatggacaccctgcctggcctggtgatggcccaggaccagagaatccggtggtatctgctgtccatgggcagcaacgagaatatccacagcatccacttcagcggccacgtgttcaccgtgcggaagaaagaagagtacaagatggccctgtacaacctgtaccccggcgtgttcgagacagtggagatgctgcccagcaaggccggcatctggcgggtggagtgtctgatcggcgagcacctgcacgctggcatgagcaccctgtttctggtgtacagcaacaagtgccagaccccactgggcatggcctctggccacatccgggacttccagatcaccgcctccggccagtacggccagtgggcccccaagctggccagactgcactacagcggcagcatcaacgcctggtccaccaaagagcccttcagctggatcaaggtggacctgctggcccctatgatcatccacggcattaagacccagggcgccaggcagaagttcagcagcctgtacatcagccagttcatcatcatgtacagcctggacggcaagaagtggcagacctaccggggcaacagcaccggcaccctgatggtgttcttcggcaatgtggacagcagcggcatcaagcacaacatcttcaacccccccatcattgcccggtacatccggctgcaccccacccactacagcattagatccacactgagaatggaactgatgggctgcgacctgaactcctgcagcatgcctctgggcatggaaagcaaggccatcagcgacgcccagatcacagccagcagctacttcaccaacatgttcgccacctggtccccctccaaggccaggctgcacctgcagggccggtccaacgcctggcggcctcaggtcaacaaccccaaagaatggctgcaggtggactttcagaaaaccatgaaggtgaccggcgtgaccacccagggcgtgaaaagcctgctgaccagcatgtacgtgaaagagtttctgatcagcagctctcaggatggccaccagtggaccctgttctttcagaacggcaaggtgaaagtgttccagggcaaccaggactccttcacccccgtggtgaactccctggacccccccctgctgacccgctacctgagaatccacccccagtcttgggtgcaccagatcgccctcaggatggaagtcctgggatgtgaggcccaggatctgtactgatgacgtctggaacaatcaacctctggattacaaaatttgtgaaagattgactggtattcttaactatgttgctccttttacgctatgtggatacgctgctttaatgcctttgtatcatgctattgcttcccgtatggctttcattttctcctccttgtataaatcctggttgctgtctctttatgaggagttgtggcccgttgtcaggcaacgtggcgtggtgtgcactgtgtttgctgacgcaacccccactggttggggcattgccaccacctgtcagctcctttccgggactttcgctttccccctccctattgccacggcggaactcatcgccgcctgccttgcccgctgctggacaggggctcggctgttgggcactgacaattccgtggtgttgtcggggaagctgacgtcctttccatggctgctcgcctgtgttgccacctggattctgcgcgggacgtccttctgctacgtcccttcggccctcaatccagcggaccttccttcccgcggcctgctgccggctctgcggcctcttccgcgtcttcgccttcgccctcagacgagtcggatctccctttgggccgcctccccgcctggaattaattctgcagtcgagacctagaaaaacatggagcaatcacaagtagcaatacagcagctaccaatgctgattgtgcctggctagaagcacaagaggaggaggaggtgggttttccagtcacacctcaggtacctttaagaccaatgacttacaaggcagctgtagatcttagccactttttaaaagaaaagaggggactggaagggctaattcactcccaacgaagacaagatatccttgatctgtggatctaccacacacaaggctacttccctgattagcagaactacacaccagggccaggggtcagatatccactgacctttggatggtgctacaagctagtaccagttgagccagataaggtagaagaggccaataaaggagagaacaccagcttgttacaccctgtgagcctgcatgggatggatgacccggagagagaagtgttagagtggaggtttgacagccgcctagcatttcatcacgtggcccgagagctgcatccggagtacttcaagaactgctgatatcgagcttgctacaagggactttccgctggggactttccagggaggcgtggcctgggcgggactggggagtggcgagccctcagatcctgcatataagcagctgctttttgcctgtactgggtctctctggttagaccagatctgagcctgggagctctctggctaactagggaacccactgcttaagcctcaataaagcttgccttgagtgcttcaagtagtgtgtgcccgtctgttgtgtgactctggtaactagagatccctcagacccttttagtcagtgtggaaaatctctagcagtagtagttcatgtcatcttattattcagtatttataacttgcaaagaaatgaatatcagagagtgagaggccttgacattgctagcgttttaccgtcgacctctagctagagcttggcgtaatcatggtcatagctgtttcctgtgtgaaattgttatccgctcacaattccacacaacatacgagccggaagcataaagtgtaaagcctggggtgcctaatgagtgagctaactcacattaattgcgttgcgctcactgcccgctttccagtcgggaaacctgtcgtgccagctgcattaatgaatcggccaacgcgcggggagaggcggtttgcgtattgggcgctcttccgcttcctcgctcactgactcgctgcgctcggtcgttcggctgcggcgagcggtatcagctcactcaaaggcggtaatacggttatccacagaatcaggggataacgcaggaaagaacatgtgagcaaaaggccagcaaaaggccaggaaccgtaaaaaggccgcgttgctggcgtttttccataggctccgcccccctgacgagcatcacaaaaatcgacgctcaagtcagaggtggcgaaacccgacaggactataaagataccaggcgtttccccctggaagctccctcgtgcgctctcctgttccgaccctgccgcttaccggatacctgtccgcctttctcccttcgggaagcgtggcgctttctcatagctcacgctgtaggtatctcagttcggtgtaggtcgttcgctccaagctgggctgtgtgcacgaaccccccgttcagcccgaccgctgcgccttatccggtaactatcgtcttgagtccaacccggtaagacacgacttatcgccactggcagcagccactggtaacaggattagcagagcgaggtatgtaggcggtgctacagagttcttgaagtggtggcctaactacggctacactagaagaacagtatttggtatctgcgctctgctgaagccagttaccttcggaaaaagagttggtagctcttgatccggcaaacaaaccaccgctggtagcggtggtttttttgtttgcaagcagcagattacgcgcagaaaaaaaggatctcaagaagatcctttgatcttttctacggggtctgacgctcagtggaacgaaaactcacgttaagggattttggtcatgagattatcaaaaaggatcttcacctagatccttttaaattaaaaatgaagttttaaatcaatctaaagtatatatgagtaaacttggtctgacagttaccaatgcttaatcagtgaggcacctatctcagcgatctgtctatttcgttcatccatagttgcctgactccccgtcgtgtagataactacgatacgggagggcttaccatctggccccagtgctgcaatgataccgcgagacccacgctcaccggctccagatttatcagcaataaaccagccagccggaagggccgagcgcagaagtggtcctgcaactttatccgcctccatccagtctattaattgttgccgggaagctagagtaagtagttcgccagttaatagtttgcgcaacgttgttgccattgctacaggcatcgtggtgtcacgctcgtcgtttggtatggcttcattcagctccggttcccaacgatcaaggcgagttacatgatcccccatgttgtgcaaaaaagcggttagctccttcggtcctccgatcgttgtcagaagtaagttggccgcagtgttatcactcatggttatggcagcactgcataattctcttactgtcatgccatccgtaagatgcttttctgtgactggtgagtactcaaccaagtcattctgagaatagtgtatgcggcgaccgagttgctcttgcccggcgtcaatacgggataataccgcgccacatagcagaactttaaaagtgctcatcattggaaaacgttcttcggggcgaaaactctcaaggatcttaccgctgttgagatccagttcgatgtaacccactcgtgcacccaactgatcttcagcatcttttactttcaccagcgtttctgggtgagcaaaaacaggaaggcaaaatgccgcaaaaaagggaataagggcgacacggaaatgttgaatactcatactcttcctttttcaatattattgaagcatttatcagggttattgtctcatgagcggatacatatttgaatgtatttagaaaaataaacaaataggggttccgcgcacatttccccgaaaagtgccacctgacgtcgacggatcgggagatcaacttgtttattgcagcttataatggttacaaataaagcaatagcatcacaaatttcacaaataaagcatttttttcactgcattctagttgtggtttgtccaaactcatcaatgtatcttatcatgtctggatcaactggataactcaagctaaccaaaatcatcccaaacttcccaccccataccctattaccactgccaattacctgtggtttcatttactctaaacctgtgattcctctgaattattttcattttaaagaaattgtatttgttaaatatgtactacaaacttagtagtttttaaagaaattgtatttgttaaatatgtactacaaacttagtagt

SEQ ID NO: 44 - DNA, 11177 bp, Artificial Sequence
  vector
tggaagggctaattcactcccaaagaagacaagatatccttgatctgtggatctaccacacacaaggctacttccctgattagcagaactacacaccagggccaggggtcagatatccactgacctttggatggtgctacaagctagtaccagttgagccagataaggtagaagaggccaataaaggagagaacaccagcttgttacaccctgtgagcctgcatgggatggatgacccggagagagaagtgttagagtggaggtttgacagccgcctagcatttcatcacgtggcccgagagctgcatccggagtacttcaagaactgctgatatcgagcttgctacaagggactttccgctggggactttccagggaggcgtggcctgggcgggactggggagtggcgagccctcagatcctgcatataagcagctgctttttgcctgtactgggtctctctggttagaccagatctgagcctgggagctctctggctaactagggaacccactgcttaagcctcaataaagcttgccttgagtgcttcaagtagtgtgtgcccgtctgttgtgtgactctggtaactagagatccctcagacccttttagtcagtgtggaaaatctctagcagtggcgcccgaacagggacttgaaagcgaaagggaaaccagaggagctctctcgacgcaggactcggcttgctgaagcgcgcacggcaagaggcgaggggcggcgactggtgagtacgccaaaaattttgactagcggaggctagaaggagagagatgggtgcgagagcgtcagtattaagcgggggagaattagatcgcgatgggaaaaaattcggttaaggccagggggaaagaaaaaatataaattaaaacatatagtatgggcaagcagggagctagaacgattcgcagttaatcctggcctgttagaaacatcagaaggctgtagacaaatactgggacagctacaaccatcccttcagacaggatcagaagaacttagatcattatataatacagtagcaaccctctattgtgtgcatcaaaggatagagataaaagacaccaaggaagctttagacaagatagaggaagagcaaaacaaaagtaagaccaccgcacagcaagcggccggccgctgatcttcagacctggaggaggagatatgagggacaattggagaagtgaattatataaatataaagtagtaaaaattgaaccattaggagtagcacccaccaaggcaaagagaagagtggtgcagagagaaaaaagagcagtgggaataggagctttgttccttgggttcttgggagcagcaggaagcactatgggcgcagcgtcaatgacgctgacggtacaggccagacaattattgtctggtatagtgcagcagcagaacaatttgctgagggctattgaggcgcaacagcatctgttgcaactcacagtctggggcatcaagcagctccaggcaagaatcctggctgtggaaagatacctaaaggatcaacagctcctggggatttggggttgctctggaaaactcatttgcaccactgctgtgccttggaatgctagttggagtaataaatctctggaacagatttggaatcacacgacctggatggagtgggacagagaaattaacaattacacaagcttaatacactccttaattgaagaatcgcaaaaccagcaagaaaagaatgaacaagaattattggaattagataaatgggcaagtttgtggaattggtttaacataacaaattggctgtggtatataaaattattcataatgatagtaggaggcttggtaggtttaagaatagtttttgctgtactttctatagtgaatagagttaggcagggatattcaccattatcgtttcagacccacctcccaaccccgaggggggacccgacaggcccgaaggaatagaagaagaaggtggagagagagacagagacagatccattcgattagtgaacggatctcgacggtcgccaaatggcagtattcatccacaattttaaaagaaaaggggggattggggggtacagtgcaggggaaagaatagtagacataatagcaacagacatacaaactaaagaattacaaaaacaaattacaaaaattcaaaattttcgggtttattacagggacagcagagatccagtttggatcgataagcttgatatcgaattcctgcgcggccgcttcgaacgcgcgcgatgcatcatatgcgtacgcggtctagaattcctgcagggcccactagtctcccaggcatgactccaacaatgcatcccatgggatttggggttccccagatctggggcttgtaggcctgactctcccctgtgcacacgtctcatacacgcatgcgtgcacccattgcctgccccgccccttgcacagggagtcagcagggaggactgggttatgccctgcttatcagcagcttcccagcttcctctgcctggattcttagaggcctggggtcctagaacgagctggtgcacgtggcttcccaaagatctctcagataatgagaggaaatgcagtcatcagtttgcagaaggctagggattctgggccatagctcagacctgcgcccaccatctccctccaggcagcccttggctggtccctgcgagcccgtggagactgccagtcagcgctggatccatgcagatcgagctgtccacctgcttttttctgtgcctgctgcggttctgcttcagcgccacccggcggtactacctgggcgccgtggagctgtcctgggactacatgcagagcgacctgggcgagctgcccgtggacgcccggttcccccccagagtgcccaagagcttccccttcaacaccagcgtggtgtacaagaaaaccctgttcgtggagttcaccgaccacctgttcaatatcgccaagcccaggcccccctggatgggcctgctgggccccaccatccaggccgaggtgtacgacaccgtggtgatcaccctgaagaacatggccagccaccccgtgagcctgcacgccgtgggcgtgagctactggaaggccagcgagggcgccgagtacgacgaccagaccagccagcgggagaaagaagatgacaaggtgttccctggcggcagccacacctacgtgtggcaggtgctgaaagaaaacggccccatggcctccgaccccctgtgcctgacctacagctacctgagccacgtggacctggtgaaggacctgaacagcggcctgatcggcgctctgctcgtctgccgggagggcagcctggccaaagagaaaacccagaccctgcacaagttcatcctgctgttcgccgtgttcgacgagggcaagagctggcacagcgagacaaagaacagcctgatgcaggaccgggacgccgcctctgccagagcctggcccaagatgcacaccgtgaacggctacgtgaacagaagcctgcccggcctgattggctgccaccggaagagcgtgtactggcacgtgatcggcatgggcaccacacccgaggtgcacagcatctttctggaagggcacacctttctggtccggaaccaccggcaggccagcctggaaatcagccctatcaccttcctgaccgcccagacactgctgatggacctgggccagttcctgctgttttgccacatcagctctcaccagcacgacggcatggaagcctacgtgaaggtggactcttgccccgaggaaccccagctgcggatgaagaacaacgaggaagccgaggactacgacgacgacctgaccgacagcgagatggacgtggtgcggttcgacgacgacaacagccccagcttcatccagatcagaagcgtggccaagaagcaccccaagacctgggtgcactatatcgccgccgaggaagaggactgggactacgcccccctggtgctggcccccgacgacagaagctacaagagccagtacctgaacaatggcccccagcggatcggccggaagtacaagaaagtgcggttcatggcctacaccgacgagacattcaagacccgggaggccatccagcacgagagcggcatcctgggccccctgctgtacggcgaagtgggcgacacactgctgatcatcttcaagaaccaggctagccggccctacaacatctacccccacggcatcaccgacgtgcggcccctgtacagcaggcggctgcccaagggcgtgaagcacctgaaggacttccccatcctgcccggcgagatcttcaagtacaagtggaccgtgaccgtggaggacggccccaccaagagcgaccccagatgcctgacccggtactacagcagcttcgtgaacatggaacgggacctggcctccgggctgatcggacctctgctgatctgctacaaagaaagcgtggaccagcggggcaaccagatcatgagcgacaagcggaacgtgatcctgttcagcgtgttcgatgagaaccggtcctggtatctgaccgagaacatccagcggtttctgcccaaccctgccggcgtgcagctggaagatcccgagttccaggccagcaacatcatgcactccatcaatggctacgtgttcgactctctgcagctctccgtgtgtctgcacgaggtggcctactggtacatcctgagcatcggcgcccagaccgacttcctgagcgtgttcttcagcggctacaccttcaagcacaagatggtgtacgaggacaccctgaccctgttccctttcagcggcgagacagtgttcatgagcatggaaaaccccggcctgtggattctgggctgccacaacagcgacttccggaaccggggcatgaccgccctgctgaaggtgtccagctgcgacaagaacaccggcgactactacgaggacagctacgaggatatcagcgcctacctgctgtccaagaacaacgccatcgaaccccggagcttcagccagaacccccccgtgctgacgcgtcaccagcgggagatcacccggacaaccctgcagtccgaccaggaagagatcgattacgacgacaccatcagcgtggagatgaagaaagaggatttcgatatctacgacgaggacgagaaccagagccccagaagcttccagaagaaaacccggcactacttcattgccgccgtggagaggctgtgggactacggcatgagttctagcccccacgtgctgcggaaccgggcccagagcggcagcgtgccccagttcaagaaagtggtgttccaggaattcacagacggcagcttcacccagcctctgtatagaggcgagctgaacgagcacctggggctgctggggccctacatcagggccgaagtggaggacaacatcatggtgaccttccggaatcaggccagcagaccctactccttctacagcagcctgatcagctacgaagaggaccagcggcagggcgccgaaccccggaagaacttcgtgaagcccaacgaaaccaagacctacttctggaaagtgcagcaccacatggcccccaccaaggacgagttcgactgcaaggcctgggcctacttcagcgacgtggatctggaaaaggacgtgcactctggactgattggcccactcctggtctgccacactaacaccctcaaccccgcccacggccgccaggtgaccgtgcaggaattcgccctgttcttcaccatcttcgacgagacaaagtcctggtacttcaccgagaatatggaacggaactgcagagccccctgcaacatccagatggaagatcctaccttcaaagagaactaccggttccacgccatcaacggctacatcatggacaccctgcctggcctggtgatggcccaggaccagagaatccggtggtatctgctgtccatgggcagcaacgagaatatccacagcatccacttcagcggccacgtgttcaccgtgcggaagaaagaagagtacaagatggccctgtacaacctgtaccccggcgtgttcgagacagtggagatgctgcccagcaaggccggcatctggcgggtggagtgtctgatcggcgagcacctgcacgctggcatgagcaccctgtttctggtgtacagcaacaagtgccagaccccactgggcatggcctctggccacatccgggacttccagatcaccgcctccggccagtacggccagtgggcccccaagctggccagactgcactacagcggcagcatcaacgcctggtccaccaaagagcccttcagctggatcaaggtggacctgctggcccctatgatcatccacggcattaagacccagggcgccaggcagaagttcagcagcctgtacatcagccagttcatcatcatgtacagcctggacggcaagaagtggcagacctaccggggcaacagcaccggcaccctgatggtgttcttcggcaatgtggacagcagcggcatcaagcacaacatcttcaacccccccatcattgcccggtacatccggctgcaccccacccactacagcattagatccacactgagaatggaactgatgggctgcgacctgaactcctgcagcatgcctctgggcatggaaagcaaggccatcagcgacgcccagatcacagccagcagctacttcaccaacatgttcgccacctggtccccctccaaggccaggctgcacctgcagggccggtccaacgcctggcggcctcaggtcaacaaccccaaagaatggctgcaggtggactttcagaaaaccatgaaggtgaccggcgtgaccacccagggcgtgaaaagcctgctgaccagcatgtacgtgaaagagtttctgatcagcagctctcaggatggccaccagtggaccctgttctttcagaacggcaaggtgaaagtgttccagggcaaccaggactccttcacccccgtggtgaactccctggacccccccctgctgacccgctacctgagaatccacccccagtcttgggtgcaccagatcgccctcaggatggaagtcctgggatgtgaggcccaggatctgtactgatgacgtctggaacaatcaacctctggattacaaaatttgtgaaagattgactggtattcttaactatgttgctccttttacgctatgtggatacgctgctttaatgcctttgtatcatgctattgcttcccgtatggctttcattttctcctccttgtataaatcctggttgctgtctctttatgaggagttgtggcccgttgtcaggcaacgtggcgtggtgtgcactgtgtttgctgacgcaacccccactggttggggcattgccaccacctgtcagctcctttccgggactttcgctttccccctccctattgccacggcggaactcatcgccgcctgccttgcccgctgctggacaggggctcggctgttgggcactgacaattccgtggtgttgtcggggaagctgacgtcctttccatggctgctcgcctgtgttgccacctggattctgcgcgggacgtccttctgctacgtcccttcggccctcaatccagcggaccttccttcccgcggcctgctgccggctctgcggcctcttccgcgtcttcgccttcgccctcagacgagtcggatctccctttgggccgcctccccgcctggaattaattctgcagtcgagacctagaaaaacatggagcaatcacaagtagcaatacagcagctaccaatgctgattgtgcctggctagaagcacaagaggaggaggaggtgggttttccagtcacacctcaggtacctttaagaccaatgacttacaaggcagctgtagatcttagccactttttaaaagaaaagaggggactggaagggctaattcactcccaacgaagacaagatatccttgatctgtggatctaccacacacaaggctacttccctgattagcagaactacacaccagggccaggggtcagatatccactgacctttggatggtgctacaagctagtaccagttgagccagataaggtagaagaggccaataaaggagagaacaccagcttgttacaccctgtgagcctgcatgggatggatgacccggagagagaagtgttagagtggaggtttgacagccgcctagcatttcatcacgtggcccgagagctgcatccggagtacttcaagaactgctgatatcgagcttgctacaagggactttccgctggggactttccagggaggcgtggcctgggcgggactggggagtggcgagccctcagatcctgcatataagcagctgctttttgcctgtactgggtctctctggttagaccagatctgagcctgggagctctctggctaactagggaacccactgcttaagcctcaataaagcttgccttgagtgcttcaagtagtgtgtgcccgtctgttgtgtgactctggtaactagagatccctcagacccttttagtcagtgtggaaaatctctagcagtagtagttcatgtcatcttattattcagtatttataacttgcaaagaaatgaatatcagagagtgagaggccttgacattgctagcgttttaccgtcgacctctagctagagcttggcgtaatcatggtcatagctgtttcctgtgtgaaattgttatccgctcacaattccacacaacatacgagccggaagcataaagtgtaaagcctggggtgcctaatgagtgagctaactcacattaattgcgttgcgctcactgcccgctttccagtcgggaaacctgtcgtgccagctgcattaatgaatcggccaacgcgcggggagaggcggtttgcgtattgggcgctcttccgcttcctcgctcactgactcgctgcgctcggtcgttcggctgcggcgagcggtatcagctcactcaaaggcggtaatacggttatccacagaatcaggggataacgcaggaaagaacatgtgagcaaaaggccagcaaaaggccaggaaccgtaaaaaggccgcgttgctggcgtttttccataggctccgcccccctgacgagcatcacaaaaatcgacgctcaagtcagaggtggcgaaacccgacaggactataaagataccaggcgtttccccctggaagctccctcgtgcgctctcctgttccgaccctgccgcttaccggatacctgtccgcctttctcccttcgggaagcgtggcgctttctcatagctcacgctgtaggtatctcagttcggtgtaggtcgttcgctccaagctgggctgtgtgcacgaaccccccgttcagcccgaccgctgcgccttatccggtaactatcgtcttgagtccaacccggtaagacacgacttatcgccactggcagcagccactggtaacaggattagcagagcgaggtatgtaggcggtgctacagagttcttgaagtggtggcctaactacggctacactagaagaacagtatttggtatctgcgctctgctgaagccagttaccttcggaaaaagagttggtagctcttgatccggcaaacaaaccaccgctggtagcggtggtttttttgtttgcaagcagcagattacgcgcagaaaaaaaggatctcaagaagatcctttgatcttttctacggggtctgacgctcagtggaacgaaaactcacgttaagggattttggtcatgagattatcaaaaaggatcttcacctagatccttttaaattaaaaatgaagttttaaatcaatctaaagtatatatgagtaaacttggtctgacagttaccaatgcttaatcagtgaggcacctatctcagcgatctgtctatttcgttcatccatagttgcctgactccccgtcgtgtagataactacgatacgggagggcttaccatctggccccagtgctgcaatgataccgcgagacccacgctcaccggctccagatttatcagcaataaaccagccagccggaagggccgagcgcagaagtggtcctgcaactttatccgcctccatccagtctattaattgttgccgggaagctagagtaagtagttcgccagttaatagtttgcgcaacgttgttgccattgctacaggcatcgtggtgtcacgctcgtcgtttggtatggcttcattcagctccggttcccaacgatcaaggcgagttacatgatcccccatgttgtgcaaaaaagcggttagctccttcggtcctccgatcgttgtcagaagtaagttggccgcagtgttatcactcatggttatggcagcactgcataattctcttactgtcatgccatccgtaagatgcttttctgtgactggtgagtactcaaccaagtcattctgagaatagtgtatgcggcgaccgagttgctcttgcccggcgtcaatacgggataataccgcgccacatagcagaactttaaaagtgctcatcattggaaaacgttcttcggggcgaaaactctcaaggatcttaccgctgttgagatccagttcgatgtaacccactcgtgcacccaactgatcttcagcatcttttactttcaccagcgtttctgggtgagcaaaaacaggaaggcaaaatgccgcaaaaaagggaataagggcgacacggaaatgttgaatactcatactcttcctttttcaatattattgaagcatttatcagggttattgtctcatgagcggatacatatttgaatgtatttagaaaaataaacaaataggggttccgcgcacatttccccgaaaagtgccacctgacgtcgacggatcgggagatcaacttgtttattgcagcttataatggttacaaataaagcaatagcatcacaaatttcacaaataaagcatttttttcactgcattctagttgtggtttgtccaaactcatcaatgtatcttatcatgtctggatcaactggataactcaagctaaccaaaatcatcccaaacttcccaccccataccctattaccactgccaattacctgtggtttcatttactctaaacctgtgattcctctgaattattttcattttaaagaaattgtatttgttaaatatgtactacaaacttagtagtttttaaagaaattgtatttgttaaatatgtactacaaacttagtagt

SEQ ID NO: 45 - DNA, 11196 bp, Artificial Sequence
  vector
tggaagggctaattcactcccaaagaagacaagatatccttgatctgtggatctaccacacacaaggctacttccctgattagcagaactacacaccagggccaggggtcagatatccactgacctttggatggtgctacaagctagtaccagttgagccagataaggtagaagaggccaataaaggagagaacaccagcttgttacaccctgtgagcctgcatgggatggatgacccggagagagaagtgttagagtggaggtttgacagccgcctagcatttcatcacgtggcccgagagctgcatccggagtacttcaagaactgctgatatcgagcttgctacaagggactttccgctggggactttccagggaggcgtggcctgggcgggactggggagtggcgagccctcagatcctgcatataagcagctgctttttgcctgtactgggtctctctggttagaccagatctgagcctgggagctctctggctaactagggaacccactgcttaagcctcaataaagcttgccttgagtgcttcaagtagtgtgtgcccgtctgttgtgtgactctggtaactagagatccctcagacccttttagtcagtgtggaaaatctctagcagtggcgcccgaacagggacttgaaagcgaaagggaaaccagaggagctctctcgacgcaggactcggcttgctgaagcgcgcacggcaagaggcgaggggcggcgactggtgagtacgccaaaaattttgactagcggaggctagaaggagagagatgggtgcgagagcgtcagtattaagcgggggagaattagatcgcgatgggaaaaaattcggttaaggccagggggaaagaaaaaatataaattaaaacatatagtatgggcaagcagggagctagaacgattcgcagttaatcctggcctgttagaaacatcagaaggctgtagacaaatactgggacagctacaaccatcccttcagacaggatcagaagaacttagatcattatataatacagtagcaaccctctattgtgtgcatcaaaggatagagataaaagacaccaaggaagctttagacaagatagaggaagagcaaaacaaaagtaagaccaccgcacagcaagcggccggccgctgatcttcagacctggaggaggagatatgagggacaattggagaagtgaattatataaatataaagtagtaaaaattgaaccattaggagtagcacccaccaaggcaaagagaagagtggtgcagagagaaaaaagagcagtgggaataggagctttgttccttgggttcttgggagcagcaggaagcactatgggcgcagcgtcaatgacgctgacggtacaggccagacaattattgtctggtatagtgcagcagcagaacaatttgctgagggctattgaggcgcaacagcatctgttgcaactcacagtctggggcatcaagcagctccaggcaagaatcctggctgtggaaagatacctaaaggatcaacagctcctggggatttggggttgctctggaaaactcatttgcaccactgctgtgccttggaatgctagttggagtaataaatctctggaacagatttggaatcacacgacctggatggagtgggacagagaaattaacaattacacaagcttaatacactccttaattgaagaatcgcaaaaccagcaagaaaagaatgaacaagaattattggaattagataaatgggcaagtttgtggaattggtttaacataacaaattggctgtggtatataaaattattcataatgatagtaggaggcttggtaggtttaagaatagtttttgctgtactttctatagtgaatagagttaggcagggatattcaccattatcgtttcagacccacctcccaaccccgaggggggacccgacaggcccgaaggaatagaagaagaaggtggagagagagacagagacagatccattcgattagtgaacggatctcgacggtcgccaaatggcagtattcatccacaattttaaaagaaaaggggggattggggggtacagtgcaggggaaagaatagtagacataatagcaacagacatacaaactaaagaattacaaaaacaaattacaaaaattcaaaattttcgggtttattacagggacagcagagatccagtttggatcgataagcttgatatcgaattcctgcgcggccgcttcgaacgcgcgcgatgcatcatatgcgtacgcggtctagaattcctgcagggcccactagtctcccaggcatgactccaacaatgcatcccatgggatttggggttccccagatctggggcttgtaggcctgactctcccctgtgcacacgtctcatacacgcatgcgtgcacccattgcctgccccgccccttgcacagggagtcagcagggaggactgggttatgccctgcttatcagcagcttcccagcttcctctgcctggattcttagaggcctggggtcctagaacgagctggtgcacgtggcttcccaaagatctctcagataatgagaggaaatgcagtcatcagtttgcagaaggctagggattctgggccatagctcagacctgcgcccaccatctccctccaggcagcccttggctggtccctgcgagcccgtggagactgccagtcagcgctgctggatctcgggctcgaggccaccatgcagatcgagctgtccacctgcttttttctgtgcctgctgcggttctgcttcagcgccacccggcggtactacctgggcgccgtggagctgtcctgggactacatgcagagcgacctgggcgagctgcccgtggacgcccggttcccccccagagtgcccaagagcttccccttcaacaccagcgtggtgtacaagaaaaccctgttcgtggagttcaccgaccacctgttcaatatcgccaagcccaggcccccctggatgggcctgctgggccccaccatccaggccgaggtgtacgacaccgtggtgatcaccctgaagaacatggccagccaccccgtgagcctgcacgccgtgggcgtgagctactggaaggccagcgagggcgccgagtacgacgaccagaccagccagcgggagaaagaagatgacaaggtgttccctggcggcagccacacctacgtgtggcaggtgctgaaagaaaacggccccatggcctccgaccccctgtgcctgacctacagctacctgagccacgtggacctggtgaaggacctgaacagcggcctgatcggcgctctgctcgtctgccgggagggcagcctggccaaagagaaaacccagaccctgcacaagttcatcctgctgttcgccgtgttcgacgagggcaagagctggcacagcgagacaaagaacagcctgatgcaggaccgggacgccgcctctgccagagcctggcccaagatgcacaccgtgaacggctacgtgaacagaagcctgcccggcctgattggctgccaccggaagagcgtgtactggcacgtgatcggcatgggcaccacacccgaggtgcacagcatctttctggaagggcacacctttctggtccggaaccaccggcaggccagcctggaaatcagccctatcaccttcctgaccgcccagacactgctgatggacctgggccagttcctgctgttttgccacatcagctctcaccagcacgacggcatggaagcctacgtgaaggtggactcttgccccgaggaaccccagctgcggatgaagaacaacgaggaagccgaggactacgacgacgacctgaccgacagcgagatggacgtggtgcggttcgacgacgacaacagccccagcttcatccagatcagaagcgtggccaagaagcaccccaagacctgggtgcactatatcgccgccgaggaagaggactgggactacgcccccctggtgctggcccccgacgacagaagctacaagagccagtacctgaacaatggcccccagcggatcggccggaagtacaagaaagtgcggttcatggcctacaccgacgagacattcaagacccgggaggccatccagcacgagagcggcatcctgggccccctgctgtacggcgaagtgggcgacacactgctgatcatcttcaagaaccaggctagccggccctacaacatctacccccacggcatcaccgacgtgcggcccctgtacagcaggcggctgcccaagggcgtgaagcacctgaaggacttccccatcctgcccggcgagatcttcaagtacaagtggaccgtgaccgtggaggacggccccaccaagagcgaccccagatgcctgacccggtactacagcagcttcgtgaacatggaacgggacctggcctccgggctgatcggacctctgctgatctgctacaaagaaagcgtggaccagcggggcaaccagatcatgagcgacaagcggaacgtgatcctgttcagcgtgttcgatgagaaccggtcctggtatctgaccgagaacatccagcggtttctgcccaaccctgccggcgtgcagctggaagatcccgagttccaggccagcaacatcatgcactccatcaatggctacgtgttcgactctctgcagctctccgtgtgtctgcacgaggtggcctactggtacatcctgagcatcggcgcccagaccgacttcctgagcgtgttcttcagcggctacaccttcaagcacaagatggtgtacgaggacaccctgaccctgttccctttcagcggcgagacagtgttcatgagcatggaaaaccccggcctgtggattctgggctgccacaacagcgacttccggaaccggggcatgaccgccctgctgaaggtgtccagctgcgacaagaacaccggcgactactacgaggacagctacgaggatatcagcgcctacctgctgtccaagaacaacgccatcgaaccccggagcttcagccagaacccccccgtgctgacgcgtcaccagcgggagatcacccggacaaccctgcagtccgaccaggaagagatcgattacgacgacaccatcagcgtggagatgaagaaagaggatttcgatatctacgacgaggacgagaaccagagccccagaagcttccagaagaaaacccggcactacttcattgccgccgtggagaggctgtgggactacggcatgagttctagcccccacgtgctgcggaaccgggcccagagcggcagcgtgccccagttcaagaaagtggtgttccaggaattcacagacggcagcttcacccagcctctgtatagaggcgagctgaacgagcacctggggctgctggggccctacatcagggccgaagtggaggacaacatcatggtgaccttccggaatcaggccagcagaccctactccttctacagcagcctgatcagctacgaagaggaccagcggcagggcgccgaaccccggaagaacttcgtgaagcccaacgaaaccaagacctacttctggaaagtgcagcaccacatggcccccaccaaggacgagttcgactgcaaggcctgggcctacttcagcgacgtggatctggaaaaggacgtgcactctggactgattggcccactcctggtctgccacactaacaccctcaaccccgcccacggccgccaggtgaccgtgcaggaattcgccctgttcttcaccatcttcgacgagacaaagtcctggtacttcaccgagaatatggaacggaactgcagagccccctgcaacatccagatggaagatcctaccttcaaagagaactaccggttccacgccatcaacggctacatcatggacaccctgcctggcctggtgatggcccaggaccagagaatccggtggtatctgctgtccatgggcagcaacgagaatatccacagcatccacttcagcggccacgtgttcaccgtgcggaagaaagaagagtacaagatggccctgtacaacctgtaccccggcgtgttcgagacagtggagatgctgcccagcaaggccggcatctggcgggtggagtgtctgatcggcgagcacctgcacgctggcatgagcaccctgtttctggtgtacagcaacaagtgccagaccccactgggcatggcctctggccacatccgggacttccagatcaccgcctccggccagtacggccagtgggcccccaagctggccagactgcactacagcggcagcatcaacgcctggtccaccaaagagcccttcagctggatcaaggtggacctgctggcccctatgatcatccacggcattaagacccagggcgccaggcagaagttcagcagcctgtacatcagccagttcatcatcatgtacagcctggacggcaagaagtggcagacctaccggggcaacagcaccggcaccctgatggtgttcttcggcaatgtggacagcagcggcatcaagcacaacatcttcaacccccccatcattgcccggtacatccggctgcaccccacccactacagcattagatccacactgagaatggaactgatgggctgcgacctgaactcctgcagcatgcctctgggcatggaaagcaaggccatcagcgacgcccagatcacagccagcagctacttcaccaacatgttcgccacctggtccccctccaaggccaggctgcacctgcagggccggtccaacgcctggcggcctcaggtcaacaaccccaaagaatggctgcaggtggactttcagaaaaccatgaaggtgaccggcgtgaccacccagggcgtgaaaagcctgctgaccagcatgtacgtgaaagagtttctgatcagcagctctcaggatggccaccagtggaccctgttctttcagaacggcaaggtgaaagtgttccagggcaaccaggactccttcacccccgtggtgaactccctggacccccccctgctgacccgctacctgagaatccacccccagtcttgggtgcaccagatcgccctcaggatggaagtcctgggatgtgaggcccaggatctgtactgatgacgtctggaacaatcaacctctggattacaaaatttgtgaaagattgactggtattcttaactatgttgctccttttacgctatgtggatacgctgctttaatgcctttgtatcatgctattgcttcccgtatggctttcattttctcctccttgtataaatcctggttgctgtctctttatgaggagttgtggcccgttgtcaggcaacgtggcgtggtgtgcactgtgtttgctgacgcaacccccactggttggggcattgccaccacctgtcagctcctttccgggactttcgctttccccctccctattgccacggcggaactcatcgccgcctgccttgcccgctgctggacaggggctcggctgttgggcactgacaattccgtggtgttgtcggggaagctgacgtcctttccatggctgctcgcctgtgttgccacctggattctgcgcgggacgtccttctgctacgtcccttcggccctcaatccagcggaccttccttcccgcggcctgctgccggctctgcggcctcttccgcgtcttcgccttcgccctcagacgagtcggatctccctttgggccgcctccccgcctggaattaattctgcagtcgagacctagaaaaacatggagcaatcacaagtagcaatacagcagctaccaatgctgattgtgcctggctagaagcacaagaggaggaggaggtgggttttccagtcacacctcaggtacctttaagaccaatgacttacaaggcagctgtagatcttagccactttttaaaagaaaagaggggactggaagggctaattcactcccaacgaagacaagatatccttgatctgtggatctaccacacacaaggctacttccctgattagcagaactacacaccagggccaggggtcagatatccactgacctttggatggtgctacaagctagtaccagttgagccagataaggtagaagaggccaataaaggagagaacaccagcttgttacaccctgtgagcctgcatgggatggatgacccggagagagaagtgttagagtggaggtttgacagccgcctagcatttcatcacgtggcccgagagctgcatccggagtacttcaagaactgctgatatcgagcttgctacaagggactttccgctggggactttccagggaggcgtggcctgggcgggactggggagtggcgagccctcagatcctgcatataagcagctgctttttgcctgtactgggtctctctggttagaccagatctgagcctgggagctctctggctaactagggaacccactgcttaagcctcaataaagcttgccttgagtgcttcaagtagtgtgtgcccgtctgttgtgtgactctggtaactagagatccctcagacccttttagtcagtgtggaaaatctctagcagtagtagttcatgtcatcttattattcagtatttataacttgcaaagaaatgaatatcagagagtgagaggccttgacattgctagcgttttaccgtcgacctctagctagagcttggcgtaatcatggtcatagctgtttcctgtgtgaaattgttatccgctcacaattccacacaacatacgagccggaagcataaagtgtaaagcctggggtgcctaatgagtgagctaactcacattaattgcgttgcgctcactgcccgctttccagtcgggaaacctgtcgtgccagctgcattaatgaatcggccaacgcgcggggagaggcggtttgcgtattgggcgctcttccgcttcctcgctcactgactcgctgcgctcggtcgttcggctgcggcgagcggtatcagctcactcaaaggcggtaatacggttatccacagaatcaggggataacgcaggaaagaacatgtgagcaaaaggccagcaaaaggccaggaaccgtaaaaaggccgcgttgctggcgtttttccataggctccgcccccctgacgagcatcacaaaaatcgacgctcaagtcagaggtggcgaaacccgacaggactataaagataccaggcgtttccccctggaagctccctcgtgcgctctcctgttccgaccctgccgcttaccggatacctgtccgcctttctcccttcgggaagcgtggcgctttctcatagctcacgctgtaggtatctcagttcggtgtaggtcgttcgctccaagctgggctgtgtgcacgaaccccccgttcagcccgaccgctgcgccttatccggtaactatcgtcttgagtccaacccggtaagacacgacttatcgccactggcagcagccactggtaacaggattagcagagcgaggtatgtaggcggtgctacagagttcttgaagtggtggcctaactacggctacactagaagaacagtatttggtatctgcgctctgctgaagccagttaccttcggaaaaagagttggtagctcttgatccggcaaacaaaccaccgctggtagcggtggtttttttgtttgcaagcagcagattacgcgcagaaaaaaaggatctcaagaagatcctttgatcttttctacggggtctgacgctcagtggaacgaaaactcacgttaagggattttggtcatgagattatcaaaaaggatcttcacctagatccttttaaattaaaaatgaagttttaaatcaatctaaagtatatatgagtaaacttggtctgacagttaccaatgcttaatcagtgaggcacctatctcagcgatctgtctatttcgttcatccatagttgcctgactccccgtcgtgtagataactacgatacgggagggcttaccatctggccccagtgctgcaatgataccgcgagacccacgctcaccggctccagatttatcagcaataaaccagccagccggaagggccgagcgcagaagtggtcctgcaactttatccgcctccatccagtctattaattgttgccgggaagctagagtaagtagttcgccagttaatagtttgcgcaacgttgttgccattgctacaggcatcgtggtgtcacgctcgtcgtttggtatggcttcattcagctccggttcccaacgatcaaggcgagttacatgatcccccatgttgtgcaaaaaagcggttagctccttcggtcctccgatcgttgtcagaagtaagttggccgcagtgttatcactcatggttatggcagcactgcataattctcttactgtcatgccatccgtaagatgcttttctgtgactggtgagtactcaaccaagtcattctgagaatagtgtatgcggcgaccgagttgctcttgcccggcgtcaatacgggataataccgcgccacatagcagaactttaaaagtgctcatcattggaaaacgttcttcggggcgaaaactctcaaggatcttaccgctgttgagatccagttcgatgtaacccactcgtgcacccaactgatcttcagcatcttttactttcaccagcgtttctgggtgagcaaaaacaggaaggcaaaatgccgcaaaaaagggaataagggcgacacggaaatgttgaatactcatactcttcctttttcaatattattgaagcatttatcagggttattgtctcatgagcggatacatatttgaatgtatttagaaaaataaacaaataggggttccgcgcacatttccccgaaaagtgccacctgacgtcgacggatcgggagatcaacttgtttattgcagcttataatggttacaaataaagcaatagcatcacaaatttcacaaataaagcatttttttcactgcattctagttgtggtttgtccaaactcatcaatgtatcttatcatgtctggatcaactggataactcaagctaaccaaaatcatcccaaacttcccaccccataccctattaccactgccaattacctgtggtttcatttactctaaacctgtgattcctctgaattattttcattttaaagaaattgtatttgttaaatatgtactacaaacttagtagtttttaaagaaattgtatttgttaaatatgtactacaaacttagtagt

SEQ ID NO: 46 - DNA, 8303 bp, Artificial Sequence
  vector
tggaagggctaattcactcccaaagaagacaagatatccttgatctgtggatctaccacacacaaggctacttccctgattagcagaactacacaccagggccaggggtcagatatccactgacctttggatggtgctacaagctagtaccagttgagccagataaggtagaagaggccaataaaggagagaacaccagcttgttacaccctgtgagcctgcatgggatggatgacccggagagagaagtgttagagtggaggtttgacagccgcctagcatttcatcacgtggcccgagagctgcatccggagtacttcaagaactgctgatatcgagcttgctacaagggactttccgctggggactttccagggaggcgtggcctgggcgggactggggagtggcgagccctcagatcctgcatataagcagctgctttttgcctgtactgggtctctctggttagaccagatctgagcctgggagctctctggctaactagggaacccactgcttaagcctcaataaagcttgccttgagtgcttcaagtagtgtgtgcccgtctgttgtgtgactctggtaactagagatccctcagacccttttagtcagtgtggaaaatctctagcagtggcgcccgaacagggacttgaaagcgaaagggaaaccagaggagctctctcgacgcaggactcggcttgctgaagcgcgcacggcaagaggcgaggggcggcgactggtgagtacgccaaaaattttgactagcggaggctagaaggagagagatgggtgcgagagcgtcagtattaagcgggggagaattagatcgcgatgggaaaaaattcggttaaggccagggggaaagaaaaaatataaattaaaacatatagtatgggcaagcagggagctagaacgattcgcagttaatcctggcctgttagaaacatcagaaggctgtagacaaatactgggacagctacaaccatcccttcagacaggatcagaagaacttagatcattatataatacagtagcaaccctctattgtgtgcatcaaaggatagagataaaagacaccaaggaagctttagacaagatagaggaagagcaaaacaaaagtaagaccaccgcacagcaagcggccggccgctgatcttcagacctggaggaggagatatgagggacaattggagaagtgaattatataaatataaagtagtaaaaattgaaccattaggagtagcacccaccaaggcaaagagaagagtggtgcagagagaaaaaagagcagtgggaataggagctttgttccttgggttcttgggagcagcaggaagcactatgggcgcagcgtcaatgacgctgacggtacaggccagacaattattgtctggtatagtgcagcagcagaacaatttgctgagggctattgaggcgcaacagcatctgttgcaactcacagtctggggcatcaagcagctccaggcaagaatcctggctgtggaaagatacctaaaggatcaacagctcctggggatttggggttgctctggaaaactcatttgcaccactgctgtgccttggaatgctagttggagtaataaatctctggaacagatttggaatcacacgacctggatggagtgggacagagaaattaacaattacacaagcttaatacactccttaattgaagaatcgcaaaaccagcaagaaaagaatgaacaagaattattggaattagataaatgggcaagtttgtggaattggtttaacataacaaattggctgtggtatataaaattattcataatgatagtaggaggcttggtaggtttaagaatagtttttgctgtactttctatagtgaatagagttaggcagggatattcaccattatcgtttcagacccacctcccaaccccgaggggggacccgacaggcccgaaggaatagaagaagaaggtggagagagagacagagacagatccattcgattagtgaacggatctcgacggtcgccaaatggcagtattcatccacaattttaaaagaaaaggggggattggggggtacagtgcaggggaaagaatagtagacataatagcaacagacatacaaactaaagaattacaaaaacaaattacaaaaattcaaaattttcgggtttattacagggacagcagagatccagtttggatcgataagcttgatatcgaattcctgcgcggccgcttcgaacgcgcgcgatgcatcatatgcgtacgcggtctagaattcctgcagggcccactagtctcccaggcatgactccaacaatgcatcccatgggatttggggttccccagatctggggcttgtaggcctgactctcccctgtgcacacgtctcatacacgcatgcgtgcacccattgcctgccccgccccttgcacagggagtcagcagggaggactgggttatgccctgcttatcagcagcttcccagcttcctctgcctggattcttagaggcctggggtcctagaacgagctggtgcacgtggcttcccaaagatctctcagataatgagaggaaatgcagtcatcagtttgcagaaggctagggattctgggccatagctcagacctgcgcccaccatctccctccaggcagcccttggctggtccctgcgagcccgtggagactgccagtcagcgctgctggatctcgggctcgaggccaccatggaagatgccaaaaacattaagaagggcccagcgccattctacccactcgaagacgggaccgccggcgagcagctgcacaaagccatgaagcgctacgccctggtgcccggcaccatcgcctttaccgacgcacatatcgaggtggacattacctacgccgagtacttcgagatgagcgttcggctggcagaagctatgaagcgctatgggctgaatacaaaccatcggatcgtggtgtgcagcgagaatagcttgcagttcttcatgcccgtgttgggtgccctgttcatcggtgtggctgtggccccagctaacgacatctacaacgagcgcgagctgctgaacagcatgggcatcagccagcccaccgtcgtattcgtgagcaagaaagggctgcaaaagatcctcaacgtgcaaaagaagctaccgatcatacaaaagatcatcatcatggatagcaagaccgactaccagggcttccaaagcatgtacaccttcgtgacttcccatttgccacccggcttcaacgagtacgacttcgtgcccgagagcttcgaccgggacaaaaccatcgccctgatcatgaacagtagtggcagtaccggattgcccaagggcgtagccctaccgcaccgcaccgcttgtgtccgattcagtcatgcccgcgaccccatcttcggcaaccagatcatccccgacaccgctatcctcagcgtggtgccatttcaccacggcttcggcatgttcaccacgctgggctacttgatctgcggctttcgggtcgtgctcatgtaccgcttcgaggaggagctattcttgcgcagcttgcaagactataagattcaatctgccctgctggtgcccacactatttagcttcttcgctaagagcactctcatcgacaagtacgacctaagcaacttgcacgagatcgccagcggcggggcgccgctcagcaaggaggtaggtgaggccgtggccaaacgcttccacctaccaggcatccgccagggctacggcctgacagaaacaaccagcgccattctgatcacccccgaaggggacgacaagcctggcgcagtaggcaaggtggtgcccttcttcgaggctaaggtggtggacttggacaccggtaagacactgggtgtgaaccagcgcggcgagctgtgcgtccgtggccccatgatcatgagcggctacgttaacaaccccgaggctacaaacgctctcatcgacaaggacggctggctgcacagcggcgacatcgcctactgggacgaggacgagcacttcttcatcgtggaccggctgaagagcctgatcaaatacaagggctaccaggtagccccagccgaactggagagcatcctgctgcaacaccccaacatcttcgacgccggggtcgccggcctgcccgacgacgatgccggcgagctgcccgccgcagtcgtcgtgctggaacacggtaaaaccatgaccgagaaggagatcgtggactatgtggccagccaggttacaaccgccaagaagctgcgcggtggtgttgtgttcgtggacgaggtgcctaaaggactgaccggcaagttggacgcccgcaagatccgcgagattctcattaaggccaagaagggcggcaagatcgccgtgtaaatgcagcctagggtatacgatatcaagcttatcgtcgacaatcaacctctggattacaaaatttgtgaaagattgactggtattcttaactatgttgctccttttacgctatgtggatacgctgctttaatgcctttgtatcatgctattgcttcccgtatggctttcattttctcctccttgtataaatcctggttgctgtctctttatgaggagttgtggcccgttgtcaggcaacgtggcgtggtgtgcactgtgtttgctgacgcaacccccactggttggggcattgccaccacctgtcagctcctttccgggactttcgctttccccctccctattgccacggcggaactcatcgccgcctgccttgcccgctgctggacaggggctcggctgttgggcactgacaattccgtggtgttgtcggggaagctgacgtcctttccatggctgctcgcctgtgttgccacctggattctgcgcgggacgtccttctgctacgtcccttcggccctcaatccagcggaccttccttcccgcggcctgctgccggctcaagataggtacctttaagaccaatgacttacaaggcagctgtagatcttagccactttttaaaagaaaagaggggactggaagggctaattcactcccaacgaagacaagatatccttgatctgtggatctaccacacacaaggctacttccctgattagcagaactacacaccagggccaggggtcagatatccactgacctttggatggtgctacaagctagtaccagttgagccagataaggtagaagaggccaataaaggagagaacaccagcttgttacaccctgtgagcctgcatgggatggatgacccggagagagaagtgttagagtggaggtttgacagccgcctagcatttcatcacgtggcccgagagctgcatccggagtacttcaagaactgctgatatcgagcttgctacaagggactttccgctggggactttccagggaggcgtggcctgggcgggactggggagtggcgagccctcagatcctgcatataagcagctgctttttgcctgtactgggtctctctggttagaccagatctgagcctgggagctctctggctaactagggaacccactgcttaagcctcaataaagcttgccttgagtgcttcaagtagtgtgtgcccgtctgttgtgtgactctggtaactagagatccctcagacccttttagtcagtgtggaaaatctctagcagtagtagttcatgtcatcttattattcagtatttataacttgcaaagaaatgaatatcagagagtgagaggccttgacattgctagcgttttaccgtcgacctctagctagagcttggcgtaatcatggtcatagctgtttcctgtgtgaaattgttatccgctcacaattccacacaacatacgagccggaagcataaagtgtaaagcctggggtgcctaatgagtgagctaactcacattaattgcgttgcgctcactgcccgctttccagtcgggaaacctgtcgtgccagctgcattaatgaatcggccaacgcgcggggagaggcggtttgcgtattgggcgctcttccgcttcctcgctcactgactcgctgcgctcggtcgttcggctgcggcgagcggtatcagctcactcaaaggcggtaatacggttatccacagaatcaggggataacgcaggaaagaacatgtgagcaaaaggccagcaaaaggccaggaaccgtaaaaaggccgcgttgctggcgtttttccataggctccgcccccctgacgagcatcacaaaaatcgacgctcaagtcagaggtggcgaaacccgacaggactataaagataccaggcgtttccccctggaagctccctcgtgcgctctcctgttccgaccctgccgcttaccggatacctgtccgcctttctcccttcgggaagcgtggcgctttctcatagctcacgctgtaggtatctcagttcggtgtaggtcgttcgctccaagctgggctgtgtgcacgaaccccccgttcagcccgaccgctgcgccttatccggtaactatcgtcttgagtccaacccggtaagacacgacttatcgccactggcagcagccactggtaacaggattagcagagcgaggtatgtaggcggtgctacagagttcttgaagtggtggcctaactacggctacactagaagaacagtatttggtatctgcgctctgctgaagccagttaccttcggaaaaagagttggtagctcttgatccggcaaacaaaccaccgctggtagcggtggtttttttgtttgcaagcagcagattacgcgcagaaaaaaaggatctcaagaagatcctttgatcttttctacggggtctgacgctcagtggaacgaaaactcacgttaagggattttggtcatgagattatcaaaaaggatcttcacctagatccttttaaattaaaaatgaagttttaaatcaatctaaagtatatatgagtaaacttggtctgacagttaccaatgcttaatcagtgaggcacctatctcagcgatctgtctatttcgttcatccatagttgcctgactccccgtcgtgtagataactacgatacgggagggcttaccatctggccccagtgctgcaatgataccgcgagacccacgctcaccggctccagatttatcagcaataaaccagccagccggaagggccgagcgcagaagtggtcctgcaactttatccgcctccatccagtctattaattgttgccgggaagctagagtaagtagttcgccagttaatagtttgcgcaacgttgttgccattgctacaggcatcgtggtgtcacgctcgtcgtttggtatggcttcattcagctccggttcccaacgatcaaggcgagttacatgatcccccatgttgtgcaaaaaagcggttagctccttcggtcctccgatcgttgtcagaagtaagttggccgcagtgttatcactcatggttatggcagcactgcataattctcttactgtcatgccatccgtaagatgcttttctgtgactggtgagtactcaaccaagtcattctgagaatagtgtatgcggcgaccgagttgctcttgcccggcgtcaatacgggataataccgcgccacatagcagaactttaaaagtgctcatcattggaaaacgttcttcggggcgaaaactctcaaggatcttaccgctgttgagatccagttcgatgtaacccactcgtgcacccaactgatcttcagcatcttttactttcaccagcgtttctgggtgagcaaaaacaggaaggcaaaatgccgcaaaaaagggaataagggcgacacggaaatgttgaatactcatactcttcctttttcaatattattgaagcatttatcagggttattgtctcatgagcggatacatatttgaatgtatttagaaaaataaacaaataggggttccgcgcacatttccccgaaaagtgccacctgacgtcgacggatcgggagatcaacttgtttattgcagcttataatggttacaaataaagcaatagcatcacaaatttcacaaataaagcatttttttcactgcattctagttgtggtttgtccaaactcatcaatgtatcttatcatgtctggatcaactggataactcaagctaaccaaaatcatcccaaacttcccaccccataccctattaccactgccaattacctgtggtttcatttactctaaacctgtgattcctctgaattattttcattttaaagaaattgtatttgttaaatatgtactacaaacttagtagtttttaaagaaattgtatttgttaaatatgtactacaaacttagtagt

SEQ ID NO: 47 - DNA, 8379 bp, Artificial Sequence
  vector
tggaagggctaattcactcccaaagaagacaagatatccttgatctgtggatctaccacacacaaggctacttccctgattagcagaactacacaccagggccaggggtcagatatccactgacctttggatggtgctacaagctagtaccagttgagccagataaggtagaagaggccaataaaggagagaacaccagcttgttacaccctgtgagcctgcatgggatggatgacccggagagagaagtgttagagtggaggtttgacagccgcctagcatttcatcacgtggcccgagagctgcatccggagtacttcaagaactgctgatatcgagcttgctacaagggactttccgctggggactttccagggaggcgtggcctgggcgggactggggagtggcgagccctcagatcctgcatataagcagctgctttttgcctgtactgggtctctctggttagaccagatctgagcctgggagctctctggctaactagggaacccactgcttaagcctcaataaagcttgccttgagtgcttcaagtagtgtgtgcccgtctgttgtgtgactctggtaactagagatccctcagacccttttagtcagtgtggaaaatctctagcagtggcgcccgaacagggacttgaaagcgaaagggaaaccagaggagctctctcgacgcaggactcggcttgctgaagcgcgcacggcaagaggcgaggggcggcgactggtgagtacgccaaaaattttgactagcggaggctagaaggagagagatgggtgcgagagcgtcagtattaagcgggggagaattagatcgcgatgggaaaaaattcggttaaggccagggggaaagaaaaaatataaattaaaacatatagtatgggcaagcagggagctagaacgattcgcagttaatcctggcctgttagaaacatcagaaggctgtagacaaatactgggacagctacaaccatcccttcagacaggatcagaagaacttagatcattatataatacagtagcaaccctctattgtgtgcatcaaaggatagagataaaagacaccaaggaagctttagacaagatagaggaagagcaaaacaaaagtaagaccaccgcacagcaagcggccggccgctgatcttcagacctggaggaggagatatgagggacaattggagaagtgaattatataaatataaagtagtaaaaattgaaccattaggagtagcacccaccaaggcaaagagaagagtggtgcagagagaaaaaagagcagtgggaataggagctttgttccttgggttcttgggagcagcaggaagcactatgggcgcagcgtcaatgacgctgacggtacaggccagacaattattgtctggtatagtgcagcagcagaacaatttgctgagggctattgaggcgcaacagcatctgttgcaactcacagtctggggcatcaagcagctccaggcaagaatcctggctgtggaaagatacctaaaggatcaacagctcctggggatttggggttgctctggaaaactcatttgcaccactgctgtgccttggaatgctagttggagtaataaatctctggaacagatttggaatcacacgacctggatggagtgggacagagaaattaacaattacacaagcttaatacactccttaattgaagaatcgcaaaaccagcaagaaaagaatgaacaagaattattggaattagataaatgggcaagtttgtggaattggtttaacataacaaattggctgtggtatataaaattattcataatgatagtaggaggcttggtaggtttaagaatagtttttgctgtactttctatagtgaatagagttaggcagggatattcaccattatcgtttcagacccacctcccaaccccgaggggggacccgacaggcccgaaggaatagaagaagaaggtggagagagagacagagacagatccattcgattagtgaacggatctcgacggtcgccaaatggcagtattcatccacaattttaaaagaaaaggggggattggggggtacagtgcaggggaaagaatagtagacataatagcaacagacatacaaactaaagaattacaaaaacaaattacaaaaattcaaaattttcgggtttattacagggacagcagagatccagtttggatcgataagcttgatatcgaattcctgcgcggccgcttcgaacgcgcgcgatgcatcatatggccctcacaaaggaacaataacaggaaaccatcccagggggaagtgggccagggccagctggaaaacctgaaggggcgtacgcggtctagaattcctgcagggcccactagtctcccaggcatgactccaacaatgcatcccatgggatttggggttccccagatctggggcttgtaggcctgactctcccctgtgcacacgtctcatacacgcatgcgtgcacccattgcctgccccgccccttgcacagggagtcagcagggaggactgggttatgccctgcttatcagcagcttcccagcttcctctgcctggattcttagaggcctggggtcctagaacgagctggtgcacgtggcttcccaaagatctctcagataatgagaggaaatgcagtcatcagtttgcagaaggctagggattctgggccatagctcagacctgcgcccaccatctccctccaggcagcccttggctggtccctgcgagcccgtggagactgccagtcagcgctgctggatctcgggctcgaggccaccatggaagatgccaaaaacattaagaagggcccagcgccattctacccactcgaagacgggaccgccggcgagcagctgcacaaagccatgaagcgctacgccctggtgcccggcaccatcgcctttaccgacgcacatatcgaggtggacattacctacgccgagtacttcgagatgagcgttcggctggcagaagctatgaagcgctatgggctgaatacaaaccatcggatcgtggtgtgcagcgagaatagcttgcagttcttcatgcccgtgttgggtgccctgttcatcggtgtggctgtggccccagctaacgacatctacaacgagcgcgagctgctgaacagcatgggcatcagccagcccaccgtcgtattcgtgagcaagaaagggctgcaaaagatcctcaacgtgcaaaagaagctaccgatcatacaaaagatcatcatcatggatagcaagaccgactaccagggcttccaaagcatgtacaccttcgtgacttcccatttgccacccggcttcaacgagtacgacttcgtgcccgagagcttcgaccgggacaaaaccatcgccctgatcatgaacagtagtggcagtaccggattgcccaagggcgtagccctaccgcaccgcaccgcttgtgtccgattcagtcatgcccgcgaccccatcttcggcaaccagatcatccccgacaccgctatcctcagcgtggtgccatttcaccacggcttcggcatgttcaccacgctgggctacttgatctgcggctttcgggtcgtgctcatgtaccgcttcgaggaggagctattcttgcgcagcttgcaagactataagattcaatctgccctgctggtgcccacactatttagcttcttcgctaagagcactctcatcgacaagtacgacctaagcaacttgcacgagatcgccagcggcggggcgccgctcagcaaggaggtaggtgaggccgtggccaaacgcttccacctaccaggcatccgccagggctacggcctgacagaaacaaccagcgccattctgatcacccccgaaggggacgacaagcctggcgcagtaggcaaggtggtgcccttcttcgaggctaaggtggtggacttggacaccggtaagacactgggtgtgaaccagcgcggcgagctgtgcgtccgtggccccatgatcatgagcggctacgttaacaaccccgaggctacaaacgctctcatcgacaaggacggctggctgcacagcggcgacatcgcctactgggacgaggacgagcacttcttcatcgtggaccggctgaagagcctgatcaaatacaagggctaccaggtagccccagccgaactggagagcatcctgctgcaacaccccaacatcttcgacgccggggtcgccggcctgcccgacgacgatgccggcgagctgcccgccgcagtcgtcgtgctggaacacggtaaaaccatgaccgagaaggagatcgtggactatgtggccagccaggttacaaccgccaagaagctgcgcggtggtgttgtgttcgtggacgaggtgcctaaaggactgaccggcaagttggacgcccgcaagatccgcgagattctcattaaggccaagaagggcggcaagatcgccgtgtaaatgcagcctagggtatacgatatcaagcttatcgtcgacaatcaacctctggattacaaaatttgtgaaagattgactggtattcttaactatgttgctccttttacgctatgtggatacgctgctttaatgcctttgtatcatgctattgcttcccgtatggctttcattttctcctccttgtataaatcctggttgctgtctctttatgaggagttgtggcccgttgtcaggcaacgtggcgtggtgtgcactgtgtttgctgacgcaacccccactggttggggcattgccaccacctgtcagctcctttccgggactttcgctttccccctccctattgccacggcggaactcatcgccgcctgccttgcccgctgctggacaggggctcggctgttgggcactgacaattccgtggtgttgtcggggaagctgacgtcctttccatggctgctcgcctgtgttgccacctggattctgcgcgggacgtccttctgctacgtcccttcggccctcaatccagcggaccttccttcccgcggcctgctgccggctcaagataggtacctttaagaccaatgacttacaaggcagctgtagatcttagccactttttaaaagaaaagaggggactggaagggctaattcactcccaacgaagacaagatatccttgatctgtggatctaccacacacaaggctacttccctgattagcagaactacacaccagggccaggggtcagatatccactgacctttggatggtgctacaagctagtaccagttgagccagataaggtagaagaggccaataaaggagagaacaccagcttgttacaccctgtgagcctgcatgggatggatgacccggagagagaagtgttagagtggaggtttgacagccgcctagcatttcatcacgtggcccgagagctgcatccggagtacttcaagaactgctgatatcgagcttgctacaagggactttccgctggggactttccagggaggcgtggcctgggcgggactggggagtggcgagccctcagatcctgcatataagcagctgctttttgcctgtactgggtctctctggttagaccagatctgagcctgggagctctctggctaactagggaacccactgcttaagcctcaataaagcttgccttgagtgcttcaagtagtgtgtgcccgtctgttgtgtgactctggtaactagagatccctcagacccttttagtcagtgtggaaaatctctagcagtagtagttcatgtcatcttattattcagtatttataacttgcaaagaaatgaatatcagagagtgagaggccttgacattgctagcgttttaccgtcgacctctagctagagcttggcgtaatcatggtcatagctgtttcctgtgtgaaattgttatccgctcacaattccacacaacatacgagccggaagcataaagtgtaaagcctggggtgcctaatgagtgagctaactcacattaattgcgttgcgctcactgcccgctttccagtcgggaaacctgtcgtgccagctgcattaatgaatcggccaacgcgcggggagaggcggtttgcgtattgggcgctcttccgcttcctcgctcactgactcgctgcgctcggtcgttcggctgcggcgagcggtatcagctcactcaaaggcggtaatacggttatccacagaatcaggggataacgcaggaaagaacatgtgagcaaaaggccagcaaaaggccaggaaccgtaaaaaggccgcgttgctggcgtttttccataggctccgcccccctgacgagcatcacaaaaatcgacgctcaagtcagaggtggcgaaacccgacaggactataaagataccaggcgtttccccctggaagctccctcgtgcgctctcctgttccgaccctgccgcttaccggatacctgtccgcctttctcccttcgggaagcgtggcgctttctcatagctcacgctgtaggtatctcagttcggtgtaggtcgttcgctccaagctgggctgtgtgcacgaaccccccgttcagcccgaccgctgcgccttatccggtaactatcgtcttgagtccaacccggtaagacacgacttatcgccactggcagcagccactggtaacaggattagcagagcgaggtatgtaggcggtgctacagagttcttgaagtggtggcctaactacggctacactagaagaacagtatttggtatctgcgctctgctgaagccagttaccttcggaaaaagagttggtagctcttgatccggcaaacaaaccaccgctggtagcggtggtttttttgtttgcaagcagcagattacgcgcagaaaaaaaggatctcaagaagatcctttgatcttttctacggggtctgacgctcagtggaacgaaaactcacgttaagggattttggtcatgagattatcaaaaaggatcttcacctagatccttttaaattaaaaatgaagttttaaatcaatctaaagtatatatgagtaaacttggtctgacagttaccaatgcttaatcagtgaggcacctatctcagcgatctgtctatttcgttcatccatagttgcctgactccccgtcgtgtagataactacgatacgggagggcttaccatctggccccagtgctgcaatgataccgcgagacccacgctcaccggctccagatttatcagcaataaaccagccagccggaagggccgagcgcagaagtggtcctgcaactttatccgcctccatccagtctattaattgttgccgggaagctagagtaagtagttcgccagttaatagtttgcgcaacgttgttgccattgctacaggcatcgtggtgtcacgctcgtcgtttggtatggcttcattcagctccggttcccaacgatcaaggcgagttacatgatcccccatgttgtgcaaaaaagcggttagctccttcggtcctccgatcgttgtcagaagtaagttggccgcagtgttatcactcatggttatggcagcactgcataattctcttactgtcatgccatccgtaagatgcttttctgtgactggtgagtactcaaccaagtcattctgagaatagtgtatgcggcgaccgagttgctcttgcccggcgtcaatacgggataataccgcgccacatagcagaactttaaaagtgctcatcattggaaaacgttcttcggggcgaaaactctcaaggatcttaccgctgttgagatccagttcgatgtaacccactcgtgcacccaactgatcttcagcatcttttactttcaccagcgtttctgggtgagcaaaaacaggaaggcaaaatgccgcaaaaaagggaataagggcgacacggaaatgttgaatactcatactcttcctttttcaatattattgaagcatttatcagggttattgtctcatgagcggatacatatttgaatgtatttagaaaaataaacaaataggggttccgcgcacatttccccgaaaagtgccacctgacgtcgacggatcgggagatcaacttgtttattgcagcttataatggttacaaataaagcaatagcatcacaaatttcacaaataaagcatttttttcactgcattctagttgtggtttgtccaaactcatcaatgtatcttatcatgtctggatcaactggataactcaagctaaccaaaatcatcccaaacttcccaccccataccctattaccactgccaattacctgtggtttcatttactctaaacctgtgattcctctgaattattttcattttaaagaaattgtatttgttaaatatgtactacaaacttagtagtttttaaagaaattgtatttgttaaatatgtactacaaacttagtagt

SEQ ID NO: 48 - DNA, 11272 bp, Artificial Sequence
  vector
tggaagggctaattcactcccaaagaagacaagatatccttgatctgtggatctaccacacacaaggctacttccctgattagcagaactacacaccagggccaggggtcagatatccactgacctttggatggtgctacaagctagtaccagttgagccagataaggtagaagaggccaataaaggagagaacaccagcttgttacaccctgtgagcctgcatgggatggatgacccggagagagaagtgttagagtggaggtttgacagccgcctagcatttcatcacgtggcccgagagctgcatccggagtacttcaagaactgctgatatcgagcttgctacaagggactttccgctggggactttccagggaggcgtggcctgggcgggactggggagtggcgagccctcagatcctgcatataagcagctgctttttgcctgtactgggtctctctggttagaccagatctgagcctgggagctctctggctaactagggaacccactgcttaagcctcaataaagcttgccttgagtgcttcaagtagtgtgtgcccgtctgttgtgtgactctggtaactagagatccctcagacccttttagtcagtgtggaaaatctctagcagtggcgcccgaacagggacttgaaagcgaaagggaaaccagaggagctctctcgacgcaggactcggcttgctgaagcgcgcacggcaagaggcgaggggcggcgactggtgagtacgccaaaaattttgactagcggaggctagaaggagagagatgggtgcgagagcgtcagtattaagcgggggagaattagatcgcgatgggaaaaaattcggttaaggccagggggaaagaaaaaatataaattaaaacatatagtatgggcaagcagggagctagaacgattcgcagttaatcctggcctgttagaaacatcagaaggctgtagacaaatactgggacagctacaaccatcccttcagacaggatcagaagaacttagatcattatataatacagtagcaaccctctattgtgtgcatcaaaggatagagataaaagacaccaaggaagctttagacaagatagaggaagagcaaaacaaaagtaagaccaccgcacagcaagcggccggccgctgatcttcagacctggaggaggagatatgagggacaattggagaagtgaattatataaatataaagtagtaaaaattgaaccattaggagtagcacccaccaaggcaaagagaagagtggtgcagagagaaaaaagagcagtgggaataggagctttgttccttgggttcttgggagcagcaggaagcactatgggcgcagcgtcaatgacgctgacggtacaggccagacaattattgtctggtatagtgcagcagcagaacaatttgctgagggctattgaggcgcaacagcatctgttgcaactcacagtctggggcatcaagcagctccaggcaagaatcctggctgtggaaagatacctaaaggatcaacagctcctggggatttggggttgctctggaaaactcatttgcaccactgctgtgccttggaatgctagttggagtaataaatctctggaacagatttggaatcacacgacctggatggagtgggacagagaaattaacaattacacaagcttaatacactccttaattgaagaatcgcaaaaccagcaagaaaagaatgaacaagaattattggaattagataaatgggcaagtttgtggaattggtttaacataacaaattggctgtggtatataaaattattcataatgatagtaggaggcttggtaggtttaagaatagtttttgctgtactttctatagtgaatagagttaggcagggatattcaccattatcgtttcagacccacctcccaaccccgaggggggacccgacaggcccgaaggaatagaagaagaaggtggagagagagacagagacagatccattcgattagtgaacggatctcgacggtcgccaaatggcagtattcatccacaattttaaaagaaaaggggggattggggggtacagtgcaggggaaagaatagtagacataatagcaacagacatacaaactaaagaattacaaaaacaaattacaaaaattcaaaattttcgggtttattacagggacagcagagatccagtttggatcgataagcttgatatcgaattcctgcgcggccgcttcgaacgcgcgcgatgcatcatatggccctcacaaaggaacaataacaggaaaccatcccagggggaagtgggccagggccagctggaaaacctgaaggggcgtacgcggtctagaattcctgcagggcccactagtctcccaggcatgactccaacaatgcatcccatgggatttggggttccccagatctggggcttgtaggcctgactctcccctgtgcacacgtctcatacacgcatgcgtgcacccattgcctgccccgccccttgcacagggagtcagcagggaggactgggttatgccctgcttatcagcagcttcccagcttcctctgcctggattcttagaggcctggggtcctagaacgagctggtgcacgtggcttcccaaagatctctcagataatgagaggaaatgcagtcatcagtttgcagaaggctagggattctgggccatagctcagacctgcgcccaccatctccctccaggcagcccttggctggtccctgcgagcccgtggagactgccagtcagcgctgctggatctcgggctcgaggccaccatgcagatcgagctgtccacctgcttttttctgtgcctgctgcggttctgcttcagcgccacccggcggtactacctgggcgccgtggagctgtcctgggactacatgcagagcgacctgggcgagctgcccgtggacgcccggttcccccccagagtgcccaagagcttccccttcaacaccagcgtggtgtacaagaaaaccctgttcgtggagttcaccgaccacctgttcaatatcgccaagcccaggcccccctggatgggcctgctgggccccaccatccaggccgaggtgtacgacaccgtggtgatcaccctgaagaacatggccagccaccccgtgagcctgcacgccgtgggcgtgagctactggaaggccagcgagggcgccgagtacgacgaccagaccagccagcgggagaaagaagatgacaaggtgttccctggcggcagccacacctacgtgtggcaggtgctgaaagaaaacggccccatggcctccgaccccctgtgcctgacctacagctacctgagccacgtggacctggtgaaggacctgaacagcggcctgatcggcgctctgctcgtctgccgggagggcagcctggccaaagagaaaacccagaccctgcacaagttcatcctgctgttcgccgtgttcgacgagggcaagagctggcacagcgagacaaagaacagcctgatgcaggaccgggacgccgcctctgccagagcctggcccaagatgcacaccgtgaacggctacgtgaacagaagcctgcccggcctgattggctgccaccggaagagcgtgtactggcacgtgatcggcatgggcaccacacccgaggtgcacagcatctttctggaagggcacacctttctggtccggaaccaccggcaggccagcctggaaatcagccctatcaccttcctgaccgcccagacactgctgatggacctgggccagttcctgctgttttgccacatcagctctcaccagcacgacggcatggaagcctacgtgaaggtggactcttgccccgaggaaccccagctgcggatgaagaacaacgaggaagccgaggactacgacgacgacctgaccgacagcgagatggacgtggtgcggttcgacgacgacaacagccccagcttcatccagatcagaagcgtggccaagaagcaccccaagacctgggtgcactatatcgccgccgaggaagaggactgggactacgcccccctggtgctggcccccgacgacagaagctacaagagccagtacctgaacaatggcccccagcggatcggccggaagtacaagaaagtgcggttcatggcctacaccgacgagacattcaagacccgggaggccatccagcacgagagcggcatcctgggccccctgctgtacggcgaagtgggcgacacactgctgatcatcttcaagaaccaggctagccggccctacaacatctacccccacggcatcaccgacgtgcggcccctgtacagcaggcggctgcccaagggcgtgaagcacctgaaggacttccccatcctgcccggcgagatcttcaagtacaagtggaccgtgaccgtggaggacggccccaccaagagcgaccccagatgcctgacccggtactacagcagcttcgtgaacatggaacgggacctggcctccgggctgatcggacctctgctgatctgctacaaagaaagcgtggaccagcggggcaaccagatcatgagcgacaagcggaacgtgatcctgttcagcgtgttcgatgagaaccggtcctggtatctgaccgagaacatccagcggtttctgcccaaccctgccggcgtgcagctggaagatcccgagttccaggccagcaacatcatgcactccatcaatggctacgtgttcgactctctgcagctctccgtgtgtctgcacgaggtggcctactggtacatcctgagcatcggcgcccagaccgacttcctgagcgtgttcttcagcggctacaccttcaagcacaagatggtgtacgaggacaccctgaccctgttccctttcagcggcgagacagtgttcatgagcatggaaaaccccggcctgtggattctgggctgccacaacagcgacttccggaaccggggcatgaccgccctgctgaaggtgtccagctgcgacaagaacaccggcgactactacgaggacagctacgaggatatcagcgcctacctgctgtccaagaacaacgccatcgaaccccggagcttcagccagaacccccccgtgctgacgcgtcaccagcgggagatcacccggacaaccctgcagtccgaccaggaagagatcgattacgacgacaccatcagcgtggagatgaagaaagaggatttcgatatctacgacgaggacgagaaccagagccccagaagcttccagaagaaaacccggcactacttcattgccgccgtggagaggctgtgggactacggcatgagttctagcccccacgtgctgcggaaccgggcccagagcggcagcgtgccccagttcaagaaagtggtgttccaggaattcacagacggcagcttcacccagcctctgtatagaggcgagctgaacgagcacctggggctgctggggccctacatcagggccgaagtggaggacaacatcatggtgaccttccggaatcaggccagcagaccctactccttctacagcagcctgatcagctacgaagaggaccagcggcagggcgccgaaccccggaagaacttcgtgaagcccaacgaaaccaagacctacttctggaaagtgcagcaccacatggcccccaccaaggacgagttcgactgcaaggcctgggcctacttcagcgacgtggatctggaaaaggacgtgcactctggactgattggcccactcctggtctgccacactaacaccctcaaccccgcccacggccgccaggtgaccgtgcaggaattcgccctgttcttcaccatcttcgacgagacaaagtcctggtacttcaccgagaatatggaacggaactgcagagccccctgcaacatccagatggaagatcctaccttcaaagagaactaccggttccacgccatcaacggctacatcatggacaccctgcctggcctggtgatggcccaggaccagagaatccggtggtatctgctgtccatgggcagcaacgagaatatccacagcatccacttcagcggccacgtgttcaccgtgcggaagaaagaagagtacaagatggccctgtacaacctgtaccccggcgtgttcgagacagtggagatgctgcccagcaaggccggcatctggcgggtggagtgtctgatcggcgagcacctgcacgctggcatgagcaccctgtttctggtgtacagcaacaagtgccagaccccactgggcatggcctctggccacatccgggacttccagatcaccgcctccggccagtacggccagtgggcccccaagctggccagactgcactacagcggcagcatcaacgcctggtccaccaaagagcccttcagctggatcaaggtggacctgctggcccctatgatcatccacggcattaagacccagggcgccaggcagaagttcagcagcctgtacatcagccagttcatcatcatgtacagcctggacggcaagaagtggcagacctaccggggcaacagcaccggcaccctgatggtgttcttcggcaatgtggacagcagcggcatcaagcacaacatcttcaacccccccatcattgcccggtacatccggctgcaccccacccactacagcattagatccacactgagaatggaactgatgggctgcgacctgaactcctgcagcatgcctctgggcatggaaagcaaggccatcagcgacgcccagatcacagccagcagctacttcaccaacatgttcgccacctggtccccctccaaggccaggctgcacctgcagggccggtccaacgcctggcggcctcaggtcaacaaccccaaagaatggctgcaggtggactttcagaaaaccatgaaggtgaccggcgtgaccacccagggcgtgaaaagcctgctgaccagcatgtacgtgaaagagtttctgatcagcagctctcaggatggccaccagtggaccctgttctttcagaacggcaaggtgaaagtgttccagggcaaccaggactccttcacccccgtggtgaactccctggacccccccctgctgacccgctacctgagaatccacccccagtcttgggtgcaccagatcgccctcaggatggaagtcctgggatgtgaggcccaggatctgtactgatgacgtctggaacaatcaacctctggattacaaaatttgtgaaagattgactggtattcttaactatgttgctccttttacgctatgtggatacgctgctttaatgcctttgtatcatgctattgcttcccgtatggctttcattttctcctccttgtataaatcctggttgctgtctctttatgaggagttgtggcccgttgtcaggcaacgtggcgtggtgtgcactgtgtttgctgacgcaacccccactggttggggcattgccaccacctgtcagctcctttccgggactttcgctttccccctccctattgccacggcggaactcatcgccgcctgccttgcccgctgctggacaggggctcggctgttgggcactgacaattccgtggtgttgtcggggaagctgacgtcctttccatggctgctcgcctgtgttgccacctggattctgcgcgggacgtccttctgctacgtcccttcggccctcaatccagcggaccttccttcccgcggcctgctgccggctctgcggcctcttccgcgtcttcgccttcgccctcagacgagtcggatctccctttgggccgcctccccgcctggaattaattctgcagtcgagacctagaaaaacatggagcaatcacaagtagcaatacagcagctaccaatgctgattgtgcctggctagaagcacaagaggaggaggaggtgggttttccagtcacacctcaggtacctttaagaccaatgacttacaaggcagctgtagatcttagccactttttaaaagaaaagaggggactggaagggctaattcactcccaacgaagacaagatatccttgatctgtggatctaccacacacaaggctacttccctgattagcagaactacacaccagggccaggggtcagatatccactgacctttggatggtgctacaagctagtaccagttgagccagataaggtagaagaggccaataaaggagagaacaccagcttgttacaccctgtgagcctgcatgggatggatgacccggagagagaagtgttagagtggaggtttgacagccgcctagcatttcatcacgtggcccgagagctgcatccggagtacttcaagaactgctgatatcgagcttgctacaagggactttccgctggggactttccagggaggcgtggcctgggcgggactggggagtggcgagccctcagatcctgcatataagcagctgctttttgcctgtactgggtctctctggttagaccagatctgagcctgggagctctctggctaactagggaacccactgcttaagcctcaataaagcttgccttgagtgcttcaagtagtgtgtgcccgtctgttgtgtgactctggtaactagagatccctcagacccttttagtcagtgtggaaaatctctagcagtagtagttcatgtcatcttattattcagtatttataacttgcaaagaaatgaatatcagagagtgagaggccttgacattgctagcgttttaccgtcgacctctagctagagcttggcgtaatcatggtcatagctgtttcctgtgtgaaattgttatccgctcacaattccacacaacatacgagccggaagcataaagtgtaaagcctggggtgcctaatgagtgagctaactcacattaattgcgttgcgctcactgcccgctttccagtcgggaaacctgtcgtgccagctgcattaatgaatcggccaacgcgcggggagaggcggtttgcgtattgggcgctcttccgcttcctcgctcactgactcgctgcgctcggtcgttcggctgcggcgagcggtatcagctcactcaaaggcggtaatacggttatccacagaatcaggggataacgcaggaaagaacatgtgagcaaaaggccagcaaaaggccaggaaccgtaaaaaggccgcgttgctggcgtttttccataggctccgcccccctgacgagcatcacaaaaatcgacgctcaagtcagaggtggcgaaacccgacaggactataaagataccaggcgtttccccctggaagctccctcgtgcgctctcctgttccgaccctgccgcttaccggatacctgtccgcctttctcccttcgggaagcgtggcgctttctcatagctcacgctgtaggtatctcagttcggtgtaggtcgttcgctccaagctgggctgtgtgcacgaaccccccgttcagcccgaccgctgcgccttatccggtaactatcgtcttgagtccaacccggtaagacacgacttatcgccactggcagcagccactggtaacaggattagcagagcgaggtatgtaggcggtgctacagagttcttgaagtggtggcctaactacggctacactagaagaacagtatttggtatctgcgctctgctgaagccagttaccttcggaaaaagagttggtagctcttgatccggcaaacaaaccaccgctggtagcggtggtttttttgtttgcaagcagcagattacgcgcagaaaaaaaggatctcaagaagatcctttgatcttttctacggggtctgacgctcagtggaacgaaaactcacgttaagggattttggtcatgagattatcaaaaaggatcttcacctagatccttttaaattaaaaatgaagttttaaatcaatctaaagtatatatgagtaaacttggtctgacagttaccaatgcttaatcagtgaggcacctatctcagcgatctgtctatttcgttcatccatagttgcctgactccccgtcgtgtagataactacgatacgggagggcttaccatctggccccagtgctgcaatgataccgcgagacccacgctcaccggctccagatttatcagcaataaaccagccagccggaagggccgagcgcagaagtggtcctgcaactttatccgcctccatccagtctattaattgttgccgggaagctagagtaagtagttcgccagttaatagtttgcgcaacgttgttgccattgctacaggcatcgtggtgtcacgctcgtcgtttggtatggcttcattcagctccggttcccaacgatcaaggcgagttacatgatcccccatgttgtgcaaaaaagcggttagctccttcggtcctccgatcgttgtcagaagtaagttggccgcagtgttatcactcatggttatggcagcactgcataattctcttactgtcatgccatccgtaagatgcttttctgtgactggtgagtactcaaccaagtcattctgagaatagtgtatgcggcgaccgagttgctcttgcccggcgtcaatacgggataataccgcgccacatagcagaactttaaaagtgctcatcattggaaaacgttcttcggggcgaaaactctcaaggatcttaccgctgttgagatccagttcgatgtaacccactcgtgcacccaactgatcttcagcatcttttactttcaccagcgtttctgggtgagcaaaaacaggaaggcaaaatgccgcaaaaaagggaataagggcgacacggaaatgttgaatactcatactcttcctttttcaatattattgaagcatttatcagggttattgtctcatgagcggatacatatttgaatgtatttagaaaaataaacaaataggggttccgcgcacatttccccgaaaagtgccacctgacgtcgacggatcgggagatcaacttgtttattgcagcttataatggttacaaataaagcaatagcatcacaaatttcacaaataaagcatttttttcactgcattctagttgtggtttgtccaaactcatcaatgtatcttatcatgtctggatcaactggataactcaagctaaccaaaatcatcccaaacttcccaccccataccctattaccactgccaattacctgtggtttcatttactctaaacctgtgattcctctgaattattttcattttaaagaaattgtatttgttaaatatgtactacaaacttagtagtttttaaagaaattgtatttgttaaatatgtactacaaacttagtagt

SEQ ID NO: 49 - DNA, 10725 bp, Artificial Sequence
  Vector
acgcgtgtagtcttatgcaatactcttgtagtcttgcaacatggtaacgatgagttagcaacatgccttacaaggagagaaaaagcaccgtgcatgccgattggtggaagtaaggtggtacgatcgtgccttattaggaaggcaacagacgggtctgacatggattggacgaaccactgaattgccgcattgcagagatattgtatttaagtgcctagctcgatacaataaacgggtctctctggttagaccagatctgagcctgggagctctctggctaactagggaacccactgcttaagcctcaataaagcttgccttgagtgcttcaagtagtgtgtgcccgtctgttgtgtgactctggtaactagagatccctcagacccttttagtcagtgtggaaaatctctagcagtggcgcccgaacagggacctgaaagcgaaagggaaaccagagctctctcgacgcaggactcggcttgctgaagcgcgcacggcaagaggcgaggggcggcgactggtgagtacgccaaaaattttgactagcggaggctagaaggagagagatgggtgcgagagcgtcagtattaagcgggggagaattagatcgcgatgggaaaaaattcggttaaggccagggggaaagaaaaaatataaattaaaacatatagtatgggcaagcagggagctagaacgattcgcagttaatcctggcctgttagaaacatcagaaggctgtagacaaatactgggacagctacaaccatcccttcagacaggatcagaagaacttagatcattatataatacagtagcaaccctctattgtgtgcatcaaaggatagagataaaagacaccaaggaagctttagacaagatagaggaagagcaaaacaaaagtaagaccaccgcacagcaagcggccactgatcttcagacctggaggaggagatatgagggacaattggagaagtgaattatataaatataaagtagtaaaaattgaaccattaggagtagcacccaccaaggcaaagagaagagtggtgcagagagaaaaaagagcagtgggaataggagctttgttccttgggttcttgggagcagcaggaagcactatgggcgcagcctcaatgacgctgacggtacaggccagacaattattgtctggtatagtgcagcagcagaacaatttgctgagggctattgaggcgcaacagcatctgttgcaactcacagtctggggcatcaagcagctccaggcaagaatcctggctgtggaaagatacctaaaggatcaacagctcctggggatttggggttgctctggaaaactcatttgcaccactgctgtgccttggaatgctagttggagtaataaatctctggaacagattggaatcacacgacctggatggagtgggacagagaaattaacaattacacaagcttaatacactccttaattgaagaatcgcaaaaccagcaagaaaagaatgaacaagaattattggaattagataaatgggcaagtttgtggaattggtttaacataacaaattggctgtggtatataaaattattcataatgatagtaggaggcttggtaggtttaagaatagtttttgctgtactttctatagtgaatagagttaggcagggatattcaccattatcgtttcagacccacctcccaaccccgaggggacccgacaggcccgaaggaatagaagaagaaggtggagagagagacagagacagatccattcgattagtgaacggatctcgacggttaacttttaaaagaaaaggggggattggggggtacagtgcaggggaaagaatagtagacataatagcaacagacatacaaactaaagaattacaaaaacaaattacaaaaattcaaaattttatcgatagcgcggccgcttcgaacgcgcgcgatgcatcatatgcgtacgcggtctagaattcctgcagggcccactagtctcccaggcatgactccaacaatgcatcccatgggatttggggttccccagatctggggcttgtaggcctgactctcccctgtgcacacgtctcatacacgcatgcgtgcacccattgcctgccccgccccttgcacagggagtcagcagggaggactgggttatgccctgcttatcagcagcttcccagcttcctctgcctggattcttagaggcctggggtcctagaacgagctggtgcacgtggcttcccaaagatctctcagataatgagaggaaatgcagtcatcagtttgcagaaggctagggattctgggccatagctcagacctgcgcccaccatctccctccaggcagcccttggctggtccctgcgagcccgtggagactgccagtcagcgctgctggatctcgggctcgaggccaccatgcagatcgagctgtccacctgcttttttctgtgcctgctgcggttctgcttcagcgccacccggcggtactacctgggcgccgtggagctgtcctgggactacatgcagagcgacctgggcgagctgcccgtggacgcccggttcccccccagagtgcccaagagcttccccttcaacaccagcgtggtgtacaagaaaaccctgttcgtggagttcaccgaccacctgttcaatatcgccaagcccaggcccccctggatgggcctgctgggccccaccatccaggccgaggtgtacgacaccgtggtgatcaccctgaagaacatggccagccaccccgtgagcctgcacgccgtgggcgtgagctactggaaggccagcgagggcgccgagtacgacgaccagaccagccagcgggagaaagaagatgacaaggtgttccctggcggcagccacacctacgtgtggcaggtgctgaaagaaaacggccccatggcctccgaccccctgtgcctgacctacagctacctgagccacgtggacctggtgaaggacctgaacagcggcctgatcggcgctctgctcgtctgccgggagggcagcctggccaaagagaaaacccagaccctgcacaagttcatcctgctgttcgccgtgttcgacgagggcaagagctggcacagcgagacaaagaacagcctgatgcaggaccgggacgccgcctctgccagagcctggcccaagatgcacaccgtgaacggctacgtgaacagaagcctgcccggcctgattggctgccaccggaagagcgtgtactggcacgtgatcggcatgggcaccacacccgaggtgcacagcatctttctggaagggcacacctttctggtccggaaccaccggcaggccagcctggaaatcagccctatcaccttcctgaccgcccagacactgctgatggacctgggccagttcctgctgttttgccacatcagctctcaccagcacgacggcatggaagcctacgtgaaggtggactcttgccccgaggaaccccagctgcggatgaagaacaacgaggaagccgaggactacgacgacgacctgaccgacagcgagatggacgtggtgcggttcgacgacgacaacagccccagcttcatccagatcagaagcgtggccaagaagcaccccaagacctgggtgcactatatcgccgccgaggaagaggactgggactacgcccccctggtgctggcccccgacgacagaagctacaagagccagtacctgaacaatggcccccagcggatcggccggaagtacaagaaagtgcggttcatggcctacaccgacgagacattcaagacccgggaggccatccagcacgagagcggcatcctgggccccctgctgtacggcgaagtgggcgacacactgctgatcatcttcaagaaccaggctagccggccctacaacatctacccccacggcatcaccgacgtgcggcccctgtacagcaggcggctgcccaagggcgtgaagcacctgaaggacttccccatcctgcccggcgagatcttcaagtacaagtggaccgtgaccgtggaggacggccccaccaagagcgaccccagatgcctgacccggtactacagcagcttcgtgaacatggaacgggacctggcctccgggctgatcggacctctgctgatctgctacaaagaaagcgtggaccagcggggcaaccagatcatgagcgacaagcggaacgtgatcctgttcagcgtgttcgatgagaaccggtcctggtatctgaccgagaacatccagcggtttctgcccaaccctgccggcgtgcagctggaagatcccgagttccaggccagcaacatcatgcactccatcaatggctacgtgttcgactctctgcagctctccgtgtgtctgcacgaggtggcctactggtacatcctgagcatcggcgcccagaccgacttcctgagcgtgttcttcagcggctacaccttcaagcacaagatggtgtacgaggacaccctgaccctgttccctttcagcggcgagacagtgttcatgagcatggaaaaccccggcctgtggattctgggctgccacaacagcgacttccggaaccggggcatgaccgccctgctgaaggtgtccagctgcgacaagaacaccggcgactactacgaggacagctacgaggatatcagcgcctacctgctgtccaagaacaacgccatcgaaccccggagcttcagccagaacccccccgtgctgacgcgtcaccagcgggagatcacccggacaaccctgcagtccgaccaggaagagatcgattacgacgacaccatcagcgtggagatgaagaaagaggatttcgatatctacgacgaggacgagaaccagagccccagaagcttccagaagaaaacccggcactacttcattgccgccgtggagaggctgtgggactacggcatgagttctagcccccacgtgctgcggaaccgggcccagagcggcagcgtgccccagttcaagaaagtggtgttccaggaattcacagacggcagcttcacccagcctctgtatagaggcgagctgaacgagcacctggggctgctggggccctacatcagggccgaagtggaggacaacatcatggtgaccttccggaatcaggccagcagaccctactccttctacagcagcctgatcagctacgaagaggaccagcggcagggcgccgaaccccggaagaacttcgtgaagcccaacgaaaccaagacctacttctggaaagtgcagcaccacatggcccccaccaaggacgagttcgactgcaaggcctgggcctacttcagcgacgtggatctggaaaaggacgtgcactctggactgattggcccactcctggtctgccacactaacaccctcaaccccgcccacggccgccaggtgaccgtgcaggaattcgccctgttcttcaccatcttcgacgagacaaagtcctggtacttcaccgagaatatggaacggaactgcagagccccctgcaacatccagatggaagatcctaccttcaaagagaactaccggttccacgccatcaacggctacatcatggacaccctgcctggcctggtgatggcccaggaccagagaatccggtggtatctgctgtccatgggcagcaacgagaatatccacagcatccacttcagcggccacgtgttcaccgtgcggaagaaagaagagtacaagatggccctgtacaacctgtaccccggcgtgttcgagacagtggagatgctgcccagcaaggccggcatctggcgggtggagtgtctgatcggcgagcacctgcacgctggcatgagcaccctgtttctggtgtacagcaacaagtgccagaccccactgggcatggcctctggccacatccgggacttccagatcaccgcctccggccagtacggccagtgggcccccaagctggccagactgcactacagcggcagcatcaacgcctggtccaccaaagagcccttcagctggatcaaggtggacctgctggcccctatgatcatccacggcattaagacccagggcgccaggcagaagttcagcagcctgtacatcagccagttcatcatcatgtacagcctggacggcaagaagtggcagacctaccggggcaacagcaccggcaccctgatggtgttcttcggcaatgtggacagcagcggcatcaagcacaacatcttcaacccccccatcattgcccggtacatccggctgcaccccacccactacagcattagatccacactgagaatggaactgatgggctgcgacctgaactcctgcagcatgcctctgggcatggaaagcaaggccatcagcgacgcccagatcacagccagcagctacttcaccaacatgttcgccacctggtccccctccaaggccaggctgcacctgcagggccggtccaacgcctggcggcctcaggtcaacaaccccaaagaatggctgcaggtggactttcagaaaaccatgaaggtgaccggcgtgaccacccagggcgtgaaaagcctgctgaccagcatgtacgtgaaagagtttctgatcagcagctctcaggatggccaccagtggaccctgttctttcagaacggcaaggtgaaagtgttccagggcaaccaggactccttcacccccgtggtgaactccctggacccccccctgctgacccgctacctgagaatccacccccagtcttgggtgcaccagatcgccctcaggatggaagtcctgggatgtgaggcccaggatctgtactgatgacgtctggaacgcgtcgacaatcaacctctggattacaaaatttgtgaaagattgactggtattcttaactatgttgctccttttacgctatgtggatacgctgctttaatgcctttgtatcatgctattgcttcccgtatggctttcattttctcctccttgtataaatcctggttgctgtctctttatgaggagttgtggcccgttgtcaggcaacgtggcgtggtgtgcactgtgtttgctgacgcaacccccactggttggggcattgccaccacctgtcagctcctttccgggactttcgctttccccctccctattgccacggcggaactcatcgccgcctgccttgcccgctgctggacaggggctcggctgttgggcactgacaattccgtggtgttgtcggggaaatcatcgtcctttccttggctgctcgcctgtgttgccacctggattctgcgcgggacgtccttctgctacgtcccttcggccctcaatccagcggaccttccttcccgcggcctgctgccggctctgcggcctcttccgcgtcttcgccttcgccctcagacgagtcggatctccctttgggccgcctccccgcctggtacctttaagaccaatgacttacaaggcagctgtagatcttagccactttttaaaagaaaaggggggactggaagggctaattcactcccaacgaaaataagatctgctttttgcttgtactgggtctctctggttagaccagatctgagcctgggagctctctggctaactagggaacccactgcttaagcctcaataaagcttgccttgagtgcttcaagtagtgtgtgcccgtctgttgtgtgactctggtaactagagatccctcagacccttttagtcagtgtggaaaatctctagcagtagtagttcatgtcatcttattattcagtatttataacttgcaaagaaatgaatatcagagagtgagaggaacttgtttattgcagcttataatggttacaaataaagcaatagcatcacaaatttcacaaataaagcatttttttcactgcattctagttgtggtttgtccaaactcatcaatgtatcttatcatgtctggctctagctatcccgcccctaactccgcccagttccgcccattctccgccccatggctgactaattttttttatttatgcagaggccgaggccgcctcggcctctgagctattccagaagtagtgaggaggcttttttggaggcctagacttttgcagagacggcccaaattcgtaatcatggtcatagctgtttcctgtgtgaaattgttatccgctcacaattccacacaacatacgagccggaagcataaagtgtaaagcctggggtgcctaatgagtgagctaactcacattaattgcgttgcgctcactgcccgctttccagtcgggaaacctgtcgtgccagctgcattaatgaatcggccaacgcgcggggagaggcggtttgcgtattgggcgctcttccgcttcctcgctcactgactcgctgcgctcggtcgttcggctgcggcgagcggtatcagctcactcaaaggcggtaatacggttatccacagaatcaggggataacgcaggaaagaacatgtgagcaaaaggccagcaaaaggccaggaaccgtaaaaaggccgcgttgctggcgtttttccataggctccgcccccctgacgagcatcacaaaaatcgacgctcaagtcagaggtggcgaaacccgacaggactataaagataccaggcgtttccccctggaagctccctcgtgcgctctcctgttccgaccctgccgcttaccggatacctgtccgcctttctcccttcgggaagcgtggcgctttctcatagctcacgctgtaggtatctcagttcggtgtaggtcgttcgctccaagctgggctgtgtgcacgaaccccccgttcagcccgaccgctgcgccttatccggtaactatcgtcttgagtccaacccggtaagacacgacttatcgccactggcagcagccactggtaacaggattagcagagcgaggtatgtaggcggtgctacagagttcttgaagtggtggcctaactacggctacactagaaggacagtatttggtatctgcgctctgctgaagccagttaccttcggaaaaagagttggtagctcttgatccggcaaacaaaccaccgctggtagcggtggtttttttgtttgcaagcagcagattacgcgcagaaaaaaaggatctcaagaagatcctttgatcttttctacggggtctgacgctcagtggaacgaaaactcacgttaagggattttggtcatgagattatcaaaaaggatcttcacctagatccttttaaattaaaaatgaagttttaaatcaatctaaagtatatatgagtaaacttggtctgacagttaccaatgcttaatcagtgaggcacctatctcagcgatctgtctatttcgttcatccatagttgcctgactccccgtcgtgtagataactacgatacgggagggcttaccatctggccccagtgctgcaatgataccgcgagacccacgctcaccggctccagatttatcagcaataaaccagccagccggaagggccgagcgcagaagtggtcctgcaactttatccgcctccatccagtctattaattgttgccgggaagctagagtaagtagttcgccagttaatagtttgcgcaacgttgttgccattgctacaggcatcgtggtgtcacgctcgtcgtttggtatggcttcattcagctccggttcccaacgatcaaggcgagttacatgatcccccatgttgtgcaaaaaagcggttagctccttcggtcctccgatcgttgtcagaagtaagttggccgcagtgttatcactcatggttatggcagcactgcataattctcttactgtcatgccatccgtaagatgcttttctgtgactggtgagtactcaaccaagtcattctgagaatagtgtatgcggcgaccgagttgctcttgcccggcgtcaatacgggataataccgcgccacatagcagaactttaaaagtgctcatcattggaaaacgttcttcggggcgaaaactctcaaggatcttaccgctgttgagatccagttcgatgtaacccactcgtgcacccaactgatcttcagcatcttttactttcaccagcgtttctgggtgagcaaaaacaggaaggcaaaatgccgcaaaaaagggaataagggcgacacggaaatgttgaatactcatactcttcctttttcaatattattgaagcatttatcagggttattgtctcatgagcggatacatatttgaatgtatttagaaaaataaacaaataggggttccgcgcacatttccccgaaaagtgccacctgacgtctaagaaaccattattatcatgacattaacctataaaaataggcgtatcacgaggccctttcgtctcgcgcgtttcggtgatgacggtgaaaacctctgacacatgcagctcccggagacggtcacagcttgtctgtaagcggatgccgggagcagacaagcccgtcagggcgcgtcagcgggtgttggcgggtgtcggggctggcttaactatgcggcatcagagcagattgtactgagagtgcaccatatatgcggtgtgaaataccgcacagatgcgtaaggagaaaataccgcatcaggcgccattcgccattcaggctgcgcaactgttgggaagggcgatcggtgcgggcctcttcgctattacgccagctggcgaaagggggatgtgctgcaaggcgattaagttgggtaacgccagggttttcccagtcacgacgttgtaaaacgacggccagtgccaagctg

SEQ ID NO: 50 - DNA, 10895 bp, Artificial Sequence
  Vector
acgcgtgtagtcttatgcaatactcttgtagtcttgcaacatggtaacgatgagttagcaacatgccttacaaggagagaaaaagcaccgtgcatgccgattggtggaagtaaggtggtacgatcgtgccttattaggaaggcaacagacgggtctgacatggattggacgaaccactgaattgccgcattgcagagatattgtatttaagtgcctagctcgatacaataaacgggtctctctggttagaccagatctgagcctgggagctctctggctaactagggaacccactgcttaagcctcaataaagcttgccttgagtgcttcaagtagtgtgtgcccgtctgttgtgtgactctggtaactagagatccctcagacccttttagtcagtgtggaaaatctctagcagtggcgcccgaacagggacctgaaagcgaaagggaaaccagagctctctcgacgcaggactcggcttgctgaagcgcgcacggcaagaggcgaggggcggcgactggtgagtacgccaaaaattttgactagcggaggctagaaggagagagatgggtgcgagagcgtcagtattaagcgggggagaattagatcgcgatgggaaaaaattcggttaaggccagggggaaagaaaaaatataaattaaaacatatagtatgggcaagcagggagctagaacgattcgcagttaatcctggcctgttagaaacatcagaaggctgtagacaaatactgggacagctacaaccatcccttcagacaggatcagaagaacttagatcattatataatacagtagcaaccctctattgtgtgcatcaaaggatagagataaaagacaccaaggaagctttagacaagatagaggaagagcaaaacaaaagtaagaccaccgcacagcaagcggccactgatcttcagacctggaggaggagatatgagggacaattggagaagtgaattatataaatataaagtagtaaaaattgaaccattaggagtagcacccaccaaggcaaagagaagagtggtgcagagagaaaaaagagcagtgggaataggagctttgttccttgggttcttgggagcagcaggaagcactatgggcgcagcctcaatgacgctgacggtacaggccagacaattattgtctggtatagtgcagcagcagaacaatttgctgagggctattgaggcgcaacagcatctgttgcaactcacagtctggggcatcaagcagctccaggcaagaatcctggctgtggaaagatacctaaaggatcaacagctcctggggatttggggttgctctggaaaactcatttgcaccactgctgtgccttggaatgctagttggagtaataaatctctggaacagattggaatcacacgacctggatggagtgggacagagaaattaacaattacacaagcttaatacactccttaattgaagaatcgcaaaaccagcaagaaaagaatgaacaagaattattggaattagataaatgggcaagtttgtggaattggtttaacataacaaattggctgtggtatataaaattattcataatgatagtaggaggcttggtaggtttaagaatagtttttgctgtactttctatagtgaatagagttaggcagggatattcaccattatcgtttcagacccacctcccaaccccgaggggacccgacaggcccgaaggaatagaagaagaaggtggagagagagacagagacagatccattcgattagtgaacggatctcgacggttaacttttaaaagaaaaggggggattggggggtacagtgcaggggaaagaatagtagacataatagcaacagacatacaaactaaagaattacaaaaacaaattacaaaaattcaaaattttatcgatagcgcggccgcttcgaacgcgcgcgatgcatcatatgagggaactccctgtgctgggcctacccagctgaccccatcgctggaaacaatgggggtcaggcaacacttccccactctctcccgccgggctgtgctcacttccttcctgctggctgcctgaggaagtgtccctgccctgggacagtctggcctagcctttgtttccccgcgtacgcggtctagaattcctgcagggcccactagtctcccaggcatgactccaacaatgcatcccatgggatttggggttccccagatctggggcttgtaggcctgactctcccctgtgcacacgtctcatacacgcatgcgtgcacccattgcctgccccgccccttgcacagggagtcagcagggaggactgggttatgccctgcttatcagcagcttcccagcttcctctgcctggattcttagaggcctggggtcctagaacgagctggtgcacgtggcttcccaaagatctctcagataatgagaggaaatgcagtcatcagtttgcagaaggctagggattctgggccatagctcagacctgcgcccaccatctccctccaggcagcccttggctggtccctgcgagcccgtggagactgccagtcagcgctgctggatctcgggctcgaggccaccatgcagatcgagctgtccacctgcttttttctgtgcctgctgcggttctgcttcagcgccacccggcggtactacctgggcgccgtggagctgtcctgggactacatgcagagcgacctgggcgagctgcccgtggacgcccggttcccccccagagtgcccaagagcttccccttcaacaccagcgtggtgtacaagaaaaccctgttcgtggagttcaccgaccacctgttcaatatcgccaagcccaggcccccctggatgggcctgctgggccccaccatccaggccgaggtgtacgacaccgtggtgatcaccctgaagaacatggccagccaccccgtgagcctgcacgccgtgggcgtgagctactggaaggccagcgagggcgccgagtacgacgaccagaccagccagcgggagaaagaagatgacaaggtgttccctggcggcagccacacctacgtgtggcaggtgctgaaagaaaacggccccatggcctccgaccccctgtgcctgacctacagctacctgagccacgtggacctggtgaaggacctgaacagcggcctgatcggcgctctgctcgtctgccgggagggcagcctggccaaagagaaaacccagaccctgcacaagttcatcctgctgttcgccgtgttcgacgagggcaagagctggcacagcgagacaaagaacagcctgatgcaggaccgggacgccgcctctgccagagcctggcccaagatgcacaccgtgaacggctacgtgaacagaagcctgcccggcctgattggctgccaccggaagagcgtgtactggcacgtgatcggcatgggcaccacacccgaggtgcacagcatctttctggaagggcacacctttctggtccggaaccaccggcaggccagcctggaaatcagccctatcaccttcctgaccgcccagacactgctgatggacctgggccagttcctgctgttttgccacatcagctctcaccagcacgacggcatggaagcctacgtgaaggtggactcttgccccgaggaaccccagctgcggatgaagaacaacgaggaagccgaggactacgacgacgacctgaccgacagcgagatggacgtggtgcggttcgacgacgacaacagccccagcttcatccagatcagaagcgtggccaagaagcaccccaagacctgggtgcactatatcgccgccgaggaagaggactgggactacgcccccctggtgctggcccccgacgacagaagctacaagagccagtacctgaacaatggcccccagcggatcggccggaagtacaagaaagtgcggttcatggcctacaccgacgagacattcaagacccgggaggccatccagcacgagagcggcatcctgggccccctgctgtacggcgaagtgggcgacacactgctgatcatcttcaagaaccaggctagccggccctacaacatctacccccacggcatcaccgacgtgcggcccctgtacagcaggcggctgcccaagggcgtgaagcacctgaaggacttccccatcctgcccggcgagatcttcaagtacaagtggaccgtgaccgtggaggacggccccaccaagagcgaccccagatgcctgacccggtactacagcagcttcgtgaacatggaacgggacctggcctccgggctgatcggacctctgctgatctgctacaaagaaagcgtggaccagcggggcaaccagatcatgagcgacaagcggaacgtgatcctgttcagcgtgttcgatgagaaccggtcctggtatctgaccgagaacatccagcggtttctgcccaaccctgccggcgtgcagctggaagatcccgagttccaggccagcaacatcatgcactccatcaatggctacgtgttcgactctctgcagctctccgtgtgtctgcacgaggtggcctactggtacatcctgagcatcggcgcccagaccgacttcctgagcgtgttcttcagcggctacaccttcaagcacaagatggtgtacgaggacaccctgaccctgttccctttcagcggcgagacagtgttcatgagcatggaaaaccccggcctgtggattctgggctgccacaacagcgacttccggaaccggggcatgaccgccctgctgaaggtgtccagctgcgacaagaacaccggcgactactacgaggacagctacgaggatatcagcgcctacctgctgtccaagaacaacgccatcgaaccccggagcttcagccagaacccccccgtgctgacgcgtcaccagcgggagatcacccggacaaccctgcagtccgaccaggaagagatcgattacgacgacaccatcagcgtggagatgaagaaagaggatttcgatatctacgacgaggacgagaaccagagccccagaagcttccagaagaaaacccggcactacttcattgccgccgtggagaggctgtgggactacggcatgagttctagcccccacgtgctgcggaaccgggcccagagcggcagcgtgccccagttcaagaaagtggtgttccaggaattcacagacggcagcttcacccagcctctgtatagaggcgagctgaacgagcacctggggctgctggggccctacatcagggccgaagtggaggacaacatcatggtgaccttccggaatcaggccagcagaccctactccttctacagcagcctgatcagctacgaagaggaccagcggcagggcgccgaaccccggaagaacttcgtgaagcccaacgaaaccaagacctacttctggaaagtgcagcaccacatggcccccaccaaggacgagttcgactgcaaggcctgggcctacttcagcgacgtggatctggaaaaggacgtgcactctggactgattggcccactcctggtctgccacactaacaccctcaaccccgcccacggccgccaggtgaccgtgcaggaattcgccctgttcttcaccatcttcgacgagacaaagtcctggtacttcaccgagaatatggaacggaactgcagagccccctgcaacatccagatggaagatcctaccttcaaagagaactaccggttccacgccatcaacggctacatcatggacaccctgcctggcctggtgatggcccaggaccagagaatccggtggtatctgctgtccatgggcagcaacgagaatatccacagcatccacttcagcggccacgtgttcaccgtgcggaagaaagaagagtacaagatggccctgtacaacctgtaccccggcgtgttcgagacagtggagatgctgcccagcaaggccggcatctggcgggtggagtgtctgatcggcgagcacctgcacgctggcatgagcaccctgtttctggtgtacagcaacaagtgccagaccccactgggcatggcctctggccacatccgggacttccagatcaccgcctccggccagtacggccagtgggcccccaagctggccagactgcactacagcggcagcatcaacgcctggtccaccaaagagcccttcagctggatcaaggtggacctgctggcccctatgatcatccacggcattaagacccagggcgccaggcagaagttcagcagcctgtacatcagccagttcatcatcatgtacagcctggacggcaagaagtggcagacctaccggggcaacagcaccggcaccctgatggtgttcttcggcaatgtggacagcagcggcatcaagcacaacatcttcaacccccccatcattgcccggtacatccggctgcaccccacccactacagcattagatccacactgagaatggaactgatgggctgcgacctgaactcctgcagcatgcctctgggcatggaaagcaaggccatcagcgacgcccagatcacagccagcagctacttcaccaacatgttcgccacctggtccccctccaaggccaggctgcacctgcagggccggtccaacgcctggcggcctcaggtcaacaaccccaaagaatggctgcaggtggactttcagaaaaccatgaaggtgaccggcgtgaccacccagggcgtgaaaagcctgctgaccagcatgtacgtgaaagagtttctgatcagcagctctcaggatggccaccagtggaccctgttctttcagaacggcaaggtgaaagtgttccagggcaaccaggactccttcacccccgtggtgaactccctggacccccccctgctgacccgctacctgagaatccacccccagtcttgggtgcaccagatcgccctcaggatggaagtcctgggatgtgaggcccaggatctgtactgatgacgtctggaacgcgtcgacaatcaacctctggattacaaaatttgtgaaagattgactggtattcttaactatgttgctccttttacgctatgtggatacgctgctttaatgcctttgtatcatgctattgcttcccgtatggctttcattttctcctccttgtataaatcctggttgctgtctctttatgaggagttgtggcccgttgtcaggcaacgtggcgtggtgtgcactgtgtttgctgacgcaacccccactggttggggcattgccaccacctgtcagctcctttccgggactttcgctttccccctccctattgccacggcggaactcatcgccgcctgccttgcccgctgctggacaggggctcggctgttgggcactgacaattccgtggtgttgtcggggaaatcatcgtcctttccttggctgctcgcctgtgttgccacctggattctgcgcgggacgtccttctgctacgtcccttcggccctcaatccagcggaccttccttcccgcggcctgctgccggctctgcggcctcttccgcgtcttcgccttcgccctcagacgagtcggatctccctttgggccgcctccccgcctggtacctttaagaccaatgacttacaaggcagctgtagatcttagccactttttaaaagaaaaggggggactggaagggctaattcactcccaacgaaaataagatctgctttttgcttgtactgggtctctctggttagaccagatctgagcctgggagctctctggctaactagggaacccactgcttaagcctcaataaagcttgccttgagtgcttcaagtagtgtgtgcccgtctgttgtgtgactctggtaactagagatccctcagacccttttagtcagtgtggaaaatctctagcagtagtagttcatgtcatcttattattcagtatttataacttgcaaagaaatgaatatcagagagtgagaggaacttgtttattgcagcttataatggttacaaataaagcaatagcatcacaaatttcacaaataaagcatttttttcactgcattctagttgtggtttgtccaaactcatcaatgtatcttatcatgtctggctctagctatcccgcccctaactccgcccagttccgcccattctccgccccatggctgactaattttttttatttatgcagaggccgaggccgcctcggcctctgagctattccagaagtagtgaggaggcttttttggaggcctagacttttgcagagacggcccaaattcgtaatcatggtcatagctgtttcctgtgtgaaattgttatccgctcacaattccacacaacatacgagccggaagcataaagtgtaaagcctggggtgcctaatgagtgagctaactcacattaattgcgttgcgctcactgcccgctttccagtcgggaaacctgtcgtgccagctgcattaatgaatcggccaacgcgcggggagaggcggtttgcgtattgggcgctcttccgcttcctcgctcactgactcgctgcgctcggtcgttcggctgcggcgagcggtatcagctcactcaaaggcggtaatacggttatccacagaatcaggggataacgcaggaaagaacatgtgagcaaaaggccagcaaaaggccaggaaccgtaaaaaggccgcgttgctggcgtttttccataggctccgcccccctgacgagcatcacaaaaatcgacgctcaagtcagaggtggcgaaacccgacaggactataaagataccaggcgtttccccctggaagctccctcgtgcgctctcctgttccgaccctgccgcttaccggatacctgtccgcctttctcccttcgggaagcgtggcgctttctcatagctcacgctgtaggtatctcagttcggtgtaggtcgttcgctccaagctgggctgtgtgcacgaaccccccgttcagcccgaccgctgcgccttatccggtaactatcgtcttgagtccaacccggtaagacacgacttatcgccactggcagcagccactggtaacaggattagcagagcgaggtatgtaggcggtgctacagagttcttgaagtggtggcctaactacggctacactagaaggacagtatttggtatctgcgctctgctgaagccagttaccttcggaaaaagagttggtagctcttgatccggcaaacaaaccaccgctggtagcggtggtttttttgtttgcaagcagcagattacgcgcagaaaaaaaggatctcaagaagatcctttgatcttttctacggggtctgacgctcagtggaacgaaaactcacgttaagggattttggtcatgagattatcaaaaaggatcttcacctagatccttttaaattaaaaatgaagttttaaatcaatctaaagtatatatgagtaaacttggtctgacagttaccaatgcttaatcagtgaggcacctatctcagcgatctgtctatttcgttcatccatagttgcctgactccccgtcgtgtagataactacgatacgggagggcttaccatctggccccagtgctgcaatgataccgcgagacccacgctcaccggctccagatttatcagcaataaaccagccagccggaagggccgagcgcagaagtggtcctgcaactttatccgcctccatccagtctattaattgttgccgggaagctagagtaagtagttcgccagttaatagtttgcgcaacgttgttgccattgctacaggcatcgtggtgtcacgctcgtcgtttggtatggcttcattcagctccggttcccaacgatcaaggcgagttacatgatcccccatgttgtgcaaaaaagcggttagctccttcggtcctccgatcgttgtcagaagtaagttggccgcagtgttatcactcatggttatggcagcactgcataattctcttactgtcatgccatccgtaagatgcttttctgtgactggtgagtactcaaccaagtcattctgagaatagtgtatgcggcgaccgagttgctcttgcccggcgtcaatacgggataataccgcgccacatagcagaactttaaaagtgctcatcattggaaaacgttcttcggggcgaaaactctcaaggatcttaccgctgttgagatccagttcgatgtaacccactcgtgcacccaactgatcttcagcatcttttactttcaccagcgtttctgggtgagcaaaaacaggaaggcaaaatgccgcaaaaaagggaataagggcgacacggaaatgttgaatactcatactcttcctttttcaatattattgaagcatttatcagggttattgtctcatgagcggatacatatttgaatgtatttagaaaaataaacaaataggggttccgcgcacatttccccgaaaagtgccacctgacgtctaagaaaccattattatcatgacattaacctataaaaataggcgtatcacgaggccctttcgtctcgcgcgtttcggtgatgacggtgaaaacctctgacacatgcagctcccggagacggtcacagcttgtctgtaagcggatgccgggagcagacaagcccgtcagggcgcgtcagcgggtgttggcgggtgtcggggctggcttaactatgcggcatcagagcagattgtactgagagtgcaccatatatgcggtgtgaaataccgcacagatgcgtaaggagaaaataccgcatcaggcgccattcgccattcaggctgcgcaactgttgggaagggcgatcggtgcgggcctcttcgctattacgccagctggcgaaagggggatgtgctgcaaggcgattaagttgggtaacgccagggttttcccagtcacgacgttgtaaaacgacggccagtgccaagctg

SEQ ID NO: 51 - DNA, 11195 bp, Artificial Sequence
  Vector
acgcgtgtagtcttatgcaatactcttgtagtcttgcaacatggtaacgatgagttagcaacatgccttacaaggagagaaaaagcaccgtgcatgccgattggtggaagtaaggtggtacgatcgtgccttattaggaaggcaacagacgggtctgacatggattggacgaaccactgaattgccgcattgcagagatattgtatttaagtgcctagctcgatacaataaacgggtctctctggttagaccagatctgagcctgggagctctctggctaactagggaacccactgcttaagcctcaataaagcttgccttgagtgcttcaagtagtgtgtgcccgtctgttgtgtgactctggtaactagagatccctcagacccttttagtcagtgtggaaaatctctagcagtggcgcccgaacagggacctgaaagcgaaagggaaaccagagctctctcgacgcaggactcggcttgctgaagcgcgcacggcaagaggcgaggggcggcgactggtgagtacgccaaaaattttgactagcggaggctagaaggagagagatgggtgcgagagcgtcagtattaagcgggggagaattagatcgcgatgggaaaaaattcggttaaggccagggggaaagaaaaaatataaattaaaacatatagtatgggcaagcagggagctagaacgattcgcagttaatcctggcctgttagaaacatcagaaggctgtagacaaatactgggacagctacaaccatcccttcagacaggatcagaagaacttagatcattatataatacagtagcaaccctctattgtgtgcatcaaaggatagagataaaagacaccaaggaagctttagacaagatagaggaagagcaaaacaaaagtaagaccaccgcacagcaagcggccactgatcttcagacctggaggaggagatatgagggacaattggagaagtgaattatataaatataaagtagtaaaaattgaaccattaggagtagcacccaccaaggcaaagagaagagtggtgcagagagaaaaaagagcagtgggaataggagctttgttccttgggttcttgggagcagcaggaagcactatgggcgcagcctcaatgacgctgacggtacaggccagacaattattgtctggtatagtgcagcagcagaacaatttgctgagggctattgaggcgcaacagcatctgttgcaactcacagtctggggcatcaagcagctccaggcaagaatcctggctgtggaaagatacctaaaggatcaacagctcctggggatttggggttgctctggaaaactcatttgcaccactgctgtgccttggaatgctagttggagtaataaatctctggaacagattggaatcacacgacctggatggagtgggacagagaaattaacaattacacaagcttaatacactccttaattgaagaatcgcaaaaccagcaagaaaagaatgaacaagaattattggaattagataaatgggcaagtttgtggaattggtttaacataacaaattggctgtggtatataaaattattcataatgatagtaggaggcttggtaggtttaagaatagtttttgctgtactttctatagtgaatagagttaggcagggatattcaccattatcgtttcagacccacctcccaaccccgaggggacccgacaggcccgaaggaatagaagaagaaggtggagagagagacagagacagatccattcgattagtgaacggatctcgacggttaacttttaaaagaaaaggggggattggggggtacagtgcaggggaaagaatagtagacataatagcaacagacatacaaactaaagaattacaaaaacaaattacaaaaattcaaaattttatcgatagcgcggccgcttcgaacgcgcgcgatgcatcatatggacaggcttctgagtgtagggagctggtctgccagtctttcggaggtttgaacttgtcaaggctagggcaggatcaccatatccagcctggacttgcagttctgtggggtgcctccccatacccccataagatgccaaacatgaggccctgtcatcctccatggtccccctctactggctgttcaaggcccagggctctcccatgccagatagcatcctgtctcctaccaccactgtcccagcctgagggaactccctgtgctgggcctacccagctgaccccatcgctggaaacaatgggggtcaggcaacacttccccactctctcccgccgggctgtgctcacttccttcctgctggctgcctgaggaagtgtccctgccctgggacagtctggcctagcctttgtttccccgggggtccccacccatggagctttcaaggcttctggcccctgtgaagccagcacacgtacgcggtctagaattcctgcagggcccactagtctcccaggcatgactccaacaatgcatcccatgggatttggggttccccagatctggggcttgtaggcctgactctcccctgtgcacacgtctcatacacgcatgcgtgcacccattgcctgccccgccccttgcacagggagtcagcagggaggactgggttatgccctgcttatcagcagcttcccagcttcctctgcctggattcttagaggcctggggtcctagaacgagctggtgcacgtggcttcccaaagatctctcagataatgagaggaaatgcagtcatcagtttgcagaaggctagggattctgggccatagctcagacctgcgcccaccatctccctccaggcagcccttggctggtccctgcgagcccgtggagactgccagtcagcgctgctggatctcgggctcgaggccaccatgcagatcgagctgtccacctgcttttttctgtgcctgctgcggttctgcttcagcgccacccggcggtactacctgggcgccgtggagctgtcctgggactacatgcagagcgacctgggcgagctgcccgtggacgcccggttcccccccagagtgcccaagagcttccccttcaacaccagcgtggtgtacaagaaaaccctgttcgtggagttcaccgaccacctgttcaatatcgccaagcccaggcccccctggatgggcctgctgggccccaccatccaggccgaggtgtacgacaccgtggtgatcaccctgaagaacatggccagccaccccgtgagcctgcacgccgtgggcgtgagctactggaaggccagcgagggcgccgagtacgacgaccagaccagccagcgggagaaagaagatgacaaggtgttccctggcggcagccacacctacgtgtggcaggtgctgaaagaaaacggccccatggcctccgaccccctgtgcctgacctacagctacctgagccacgtggacctggtgaaggacctgaacagcggcctgatcggcgctctgctcgtctgccgggagggcagcctggccaaagagaaaacccagaccctgcacaagttcatcctgctgttcgccgtgttcgacgagggcaagagctggcacagcgagacaaagaacagcctgatgcaggaccgggacgccgcctctgccagagcctggcccaagatgcacaccgtgaacggctacgtgaacagaagcctgcccggcctgattggctgccaccggaagagcgtgtactggcacgtgatcggcatgggcaccacacccgaggtgcacagcatctttctggaagggcacacctttctggtccggaaccaccggcaggccagcctggaaatcagccctatcaccttcctgaccgcccagacactgctgatggacctgggccagttcctgctgttttgccacatcagctctcaccagcacgacggcatggaagcctacgtgaaggtggactcttgccccgaggaaccccagctgcggatgaagaacaacgaggaagccgaggactacgacgacgacctgaccgacagcgagatggacgtggtgcggttcgacgacgacaacagccccagcttcatccagatcagaagcgtggccaagaagcaccccaagacctgggtgcactatatcgccgccgaggaagaggactgggactacgcccccctggtgctggcccccgacgacagaagctacaagagccagtacctgaacaatggcccccagcggatcggccggaagtacaagaaagtgcggttcatggcctacaccgacgagacattcaagacccgggaggccatccagcacgagagcggcatcctgggccccctgctgtacggcgaagtgggcgacacactgctgatcatcttcaagaaccaggctagccggccctacaacatctacccccacggcatcaccgacgtgcggcccctgtacagcaggcggctgcccaagggcgtgaagcacctgaaggacttccccatcctgcccggcgagatcttcaagtacaagtggaccgtgaccgtggaggacggccccaccaagagcgaccccagatgcctgacccggtactacagcagcttcgtgaacatggaacgggacctggcctccgggctgatcggacctctgctgatctgctacaaagaaagcgtggaccagcggggcaaccagatcatgagcgacaagcggaacgtgatcctgttcagcgtgttcgatgagaaccggtcctggtatctgaccgagaacatccagcggtttctgcccaaccctgccggcgtgcagctggaagatcccgagttccaggccagcaacatcatgcactccatcaatggctacgtgttcgactctctgcagctctccgtgtgtctgcacgaggtggcctactggtacatcctgagcatcggcgcccagaccgacttcctgagcgtgttcttcagcggctacaccttcaagcacaagatggtgtacgaggacaccctgaccctgttccctttcagcggcgagacagtgttcatgagcatggaaaaccccggcctgtggattctgggctgccacaacagcgacttccggaaccggggcatgaccgccctgctgaaggtgtccagctgcgacaagaacaccggcgactactacgaggacagctacgaggatatcagcgcctacctgctgtccaagaacaacgccatcgaaccccggagcttcagccagaacccccccgtgctgacgcgtcaccagcgggagatcacccggacaaccctgcagtccgaccaggaagagatcgattacgacgacaccatcagcgtggagatgaagaaagaggatttcgatatctacgacgaggacgagaaccagagccccagaagcttccagaagaaaacccggcactacttcattgccgccgtggagaggctgtgggactacggcatgagttctagcccccacgtgctgcggaaccgggcccagagcggcagcgtgccccagttcaagaaagtggtgttccaggaattcacagacggcagcttcacccagcctctgtatagaggcgagctgaacgagcacctggggctgctggggccctacatcagggccgaagtggaggacaacatcatggtgaccttccggaatcaggccagcagaccctactccttctacagcagcctgatcagctacgaagaggaccagcggcagggcgccgaaccccggaagaacttcgtgaagcccaacgaaaccaagacctacttctggaaagtgcagcaccacatggcccccaccaaggacgagttcgactgcaaggcctgggcctacttcagcgacgtggatctggaaaaggacgtgcactctggactgattggcccactcctggtctgccacactaacaccctcaaccccgcccacggccgccaggtgaccgtgcaggaattcgccctgttcttcaccatcttcgacgagacaaagtcctggtacttcaccgagaatatggaacggaactgcagagccccctgcaacatccagatggaagatcctaccttcaaagagaactaccggttccacgccatcaacggctacatcatggacaccctgcctggcctggtgatggcccaggaccagagaatccggtggtatctgctgtccatgggcagcaacgagaatatccacagcatccacttcagcggccacgtgttcaccgtgcggaagaaagaagagtacaagatggccctgtacaacctgtaccccggcgtgttcgagacagtggagatgctgcccagcaaggccggcatctggcgggtggagtgtctgatcggcgagcacctgcacgctggcatgagcaccctgtttctggtgtacagcaacaagtgccagaccccactgggcatggcctctggccacatccgggacttccagatcaccgcctccggccagtacggccagtgggcccccaagctggccagactgcactacagcggcagcatcaacgcctggtccaccaaagagcccttcagctggatcaaggtggacctgctggcccctatgatcatccacggcattaagacccagggcgccaggcagaagttcagcagcctgtacatcagccagttcatcatcatgtacagcctggacggcaagaagtggcagacctaccggggcaacagcaccggcaccctgatggtgttcttcggcaatgtggacagcagcggcatcaagcacaacatcttcaacccccccatcattgcccggtacatccggctgcaccccacccactacagcattagatccacactgagaatggaactgatgggctgcgacctgaactcctgcagcatgcctctgggcatggaaagcaaggccatcagcgacgcccagatcacagccagcagctacttcaccaacatgttcgccacctggtccccctccaaggccaggctgcacctgcagggccggtccaacgcctggcggcctcaggtcaacaaccccaaagaatggctgcaggtggactttcagaaaaccatgaaggtgaccggcgtgaccacccagggcgtgaaaagcctgctgaccagcatgtacgtgaaagagtttctgatcagcagctctcaggatggccaccagtggaccctgttctttcagaacggcaaggtgaaagtgttccagggcaaccaggactccttcacccccgtggtgaactccctggacccccccctgctgacccgctacctgagaatccacccccagtcttgggtgcaccagatcgccctcaggatggaagtcctgggatgtgaggcccaggatctgtactgatgacgtctggaacgcgtcgacaatcaacctctggattacaaaatttgtgaaagattgactggtattcttaactatgttgctccttttacgctatgtggatacgctgctttaatgcctttgtatcatgctattgcttcccgtatggctttcattttctcctccttgtataaatcctggttgctgtctctttatgaggagttgtggcccgttgtcaggcaacgtggcgtggtgtgcactgtgtttgctgacgcaacccccactggttggggcattgccaccacctgtcagctcctttccgggactttcgctttccccctccctattgccacggcggaactcatcgccgcctgccttgcccgctgctggacaggggctcggctgttgggcactgacaattccgtggtgttgtcggggaaatcatcgtcctttccttggctgctcgcctgtgttgccacctggattctgcgcgggacgtccttctgctacgtcccttcggccctcaatccagcggaccttccttcccgcggcctgctgccggctctgcggcctcttccgcgtcttcgccttcgccctcagacgagtcggatctccctttgggccgcctccccgcctggtacctttaagaccaatgacttacaaggcagctgtagatcttagccactttttaaaagaaaaggggggactggaagggctaattcactcccaacgaaaataagatctgctttttgcttgtactgggtctctctggttagaccagatctgagcctgggagctctctggctaactagggaacccactgcttaagcctcaataaagcttgccttgagtgcttcaagtagtgtgtgcccgtctgttgtgtgactctggtaactagagatccctcagacccttttagtcagtgtggaaaatctctagcagtagtagttcatgtcatcttattattcagtatttataacttgcaaagaaatgaatatcagagagtgagaggaacttgtttattgcagcttataatggttacaaataaagcaatagcatcacaaatttcacaaataaagcatttttttcactgcattctagttgtggtttgtccaaactcatcaatgtatcttatcatgtctggctctagctatcccgcccctaactccgcccagttccgcccattctccgccccatggctgactaattttttttatttatgcagaggccgaggccgcctcggcctctgagctattccagaagtagtgaggaggcttttttggaggcctagacttttgcagagacggcccaaattcgtaatcatggtcatagctgtttcctgtgtgaaattgttatccgctcacaattccacacaacatacgagccggaagcataaagtgtaaagcctggggtgcctaatgagtgagctaactcacattaattgcgttgcgctcactgcccgctttccagtcgggaaacctgtcgtgccagctgcattaatgaatcggccaacgcgcggggagaggcggtttgcgtattgggcgctcttccgcttcctcgctcactgactcgctgcgctcggtcgttcggctgcggcgagcggtatcagctcactcaaaggcggtaatacggttatccacagaatcaggggataacgcaggaaagaacatgtgagcaaaaggccagcaaaaggccaggaaccgtaaaaaggccgcgttgctggcgtttttccataggctccgcccccctgacgagcatcacaaaaatcgacgctcaagtcagaggtggcgaaacccgacaggactataaagataccaggcgtttccccctggaagctccctcgtgcgctctcctgttccgaccctgccgcttaccggatacctgtccgcctttctcccttcgggaagcgtggcgctttctcatagctcacgctgtaggtatctcagttcggtgtaggtcgttcgctccaagctgggctgtgtgcacgaaccccccgttcagcccgaccgctgcgccttatccggtaactatcgtcttgagtccaacccggtaagacacgacttatcgccactggcagcagccactggtaacaggattagcagagcgaggtatgtaggcggtgctacagagttcttgaagtggtggcctaactacggctacactagaaggacagtatttggtatctgcgctctgctgaagccagttaccttcggaaaaagagttggtagctcttgatccggcaaacaaaccaccgctggtagcggtggtttttttgtttgcaagcagcagattacgcgcagaaaaaaaggatctcaagaagatcctttgatcttttctacggggtctgacgctcagtggaacgaaaactcacgttaagggattttggtcatgagattatcaaaaaggatcttcacctagatccttttaaattaaaaatgaagttttaaatcaatctaaagtatatatgagtaaacttggtctgacagttaccaatgcttaatcagtgaggcacctatctcagcgatctgtctatttcgttcatccatagttgcctgactccccgtcgtgtagataactacgatacgggagggcttaccatctggccccagtgctgcaatgataccgcgagacccacgctcaccggctccagatttatcagcaataaaccagccagccggaagggccgagcgcagaagtggtcctgcaactttatccgcctccatccagtctattaattgttgccgggaagctagagtaagtagttcgccagttaatagtttgcgcaacgttgttgccattgctacaggcatcgtggtgtcacgctcgtcgtttggtatggcttcattcagctccggttcccaacgatcaaggcgagttacatgatcccccatgttgtgcaaaaaagcggttagctccttcggtcctccgatcgttgtcagaagtaagttggccgcagtgttatcactcatggttatggcagcactgcataattctcttactgtcatgccatccgtaagatgcttttctgtgactggtgagtactcaaccaagtcattctgagaatagtgtatgcggcgaccgagttgctcttgcccggcgtcaatacgggataataccgcgccacatagcagaactttaaaagtgctcatcattggaaaacgttcttcggggcgaaaactctcaaggatcttaccgctgttgagatccagttcgatgtaacccactcgtgcacccaactgatcttcagcatcttttactttcaccagcgtttctgggtgagcaaaaacaggaaggcaaaatgccgcaaaaaagggaataagggcgacacggaaatgttgaatactcatactcttcctttttcaatattattgaagcatttatcagggttattgtctcatgagcggatacatatttgaatgtatttagaaaaataaacaaataggggttccgcgcacatttccccgaaaagtgccacctgacgtctaagaaaccattattatcatgacattaacctataaaaataggcgtatcacgaggccctttcgtctcgcgcgtttcggtgatgacggtgaaaacctctgacacatgcagctcccggagacggtcacagcttgtctgtaagcggatgccgggagcagacaagcccgtcagggcgcgtcagcgggtgttggcgggtgtcggggctggcttaactatgcggcatcagagcagattgtactgagagtgcaccatatatgcggtgtgaaataccgcacagatgcgtaaggagaaaataccgcatcaggcgccattcgccattcaggctgcgcaactgttgggaagggcgatcggtgcgggcctcttcgctattacgccagctggcgaaagggggatgtgctgcaaggcgattaagttgggtaacgccagggttttcccagtcacgacgttgtaaaacgacggccagtgccaagctg

SEQ ID NO: 52 - DNA, 11295 bp, Artificial Sequence
  Vector
acgcgtgtagtcttatgcaatactcttgtagtcttgcaacatggtaacgatgagttagcaacatgccttacaaggagagaaaaagcaccgtgcatgccgattggtggaagtaaggtggtacgatcgtgccttattaggaaggcaacagacgggtctgacatggattggacgaaccactgaattgccgcattgcagagatattgtatttaagtgcctagctcgatacaataaacgggtctctctggttagaccagatctgagcctgggagctctctggctaactagggaacccactgcttaagcctcaataaagcttgccttgagtgcttcaagtagtgtgtgcccgtctgttgtgtgactctggtaactagagatccctcagacccttttagtcagtgtggaaaatctctagcagtggcgcccgaacagggacctgaaagcgaaagggaaaccagagctctctcgacgcaggactcggcttgctgaagcgcgcacggcaagaggcgaggggcggcgactggtgagtacgccaaaaattttgactagcggaggctagaaggagagagatgggtgcgagagcgtcagtattaagcgggggagaattagatcgcgatgggaaaaaattcggttaaggccagggggaaagaaaaaatataaattaaaacatatagtatgggcaagcagggagctagaacgattcgcagttaatcctggcctgttagaaacatcagaaggctgtagacaaatactgggacagctacaaccatcccttcagacaggatcagaagaacttagatcattatataatacagtagcaaccctctattgtgtgcatcaaaggatagagataaaagacaccaaggaagctttagacaagatagaggaagagcaaaacaaaagtaagaccaccgcacagcaagcggccactgatcttcagacctggaggaggagatatgagggacaattggagaagtgaattatataaatataaagtagtaaaaattgaaccattaggagtagcacccaccaaggcaaagagaagagtggtgcagagagaaaaaagagcagtgggaataggagctttgttccttgggttcttgggagcagcaggaagcactatgggcgcagcctcaatgacgctgacggtacaggccagacaattattgtctggtatagtgcagcagcagaacaatttgctgagggctattgaggcgcaacagcatctgttgcaactcacagtctggggcatcaagcagctccaggcaagaatcctggctgtggaaagatacctaaaggatcaacagctcctggggatttggggttgctctggaaaactcatttgcaccactgctgtgccttggaatgctagttggagtaataaatctctggaacagattggaatcacacgacctggatggagtgggacagagaaattaacaattacacaagcttaatacactccttaattgaagaatcgcaaaaccagcaagaaaagaatgaacaagaattattggaattagataaatgggcaagtttgtggaattggtttaacataacaaattggctgtggtatataaaattattcataatgatagtaggaggcttggtaggtttaagaatagtttttgctgtactttctatagtgaatagagttaggcagggatattcaccattatcgtttcagacccacctcccaaccccgaggggacccgacaggcccgaaggaatagaagaagaaggtggagagagagacagagacagatccattcgattagtgaacggatctcgacggttaacttttaaaagaaaaggggggattggggggtacagtgcaggggaaagaatagtagacataatagcaacagacatacaaactaaagaattacaaaaacaaattacaaaaattcaaaattttatcgatagcgcggccgcttcgaacgcgcgcgatgcatcatatggagactttttttgaaaaacggaacatctgcctatcgcaaggactactattattctgaaaatcaccttcttcattagaaagtaatatttatcattttattatagaactttgatcttacttcttgtgacttcattctgcgtagagcacactcccatccttgaattaaatgacaaagcattttatattaactgacaatgactgatgccatgggcaaatcctatttctgtaaataactgaattttcttctggactgcgcatgaggggagaaagatgtctgcagtttcggtttcctggaaaatgaaacctatctcatttgttgcctgtgtcaaggggcagtgcttcagtcggggtggagctgcttaaaaggcctgggatcacaccctttgggaacacatccaagcttaagacggtgaggtcagcttcacattctcaggaactctccttctttgggtaagactgggagggtgggcaggagctacccttcccgtggccccggaccttgggtgggctgtgggctcagggagcggaggggaggccttaagcatccactctctgcccggtgtttttgttccgtacgcggtctagaattcctgcagggcccactagtctcccaggcatgactccaacaatgcatcccatgggatttggggttccccagatctggggcttgtaggcctgactctcccctgtgcacacgtctcatacacgcatgcgtgcacccattgcctgccccgccccttgcacagggagtcagcagggaggactgggttatgccctgcttatcagcagcttcccagcttcctctgcctggattcttagaggcctggggtcctagaacgagctggtgcacgtggcttcccaaagatctctcagataatgagaggaaatgcagtcatcagtttgcagaaggctagggattctgggccatagctcagacctgcgcccaccatctccctccaggcagcccttggctggtccctgcgagcccgtggagactgccagtcagcgctgctggatctcgggctcgaggccaccatgcagatcgagctgtccacctgcttttttctgtgcctgctgcggttctgcttcagcgccacccggcggtactacctgggcgccgtggagctgtcctgggactacatgcagagcgacctgggcgagctgcccgtggacgcccggttcccccccagagtgcccaagagcttccccttcaacaccagcgtggtgtacaagaaaaccctgttcgtggagttcaccgaccacctgttcaatatcgccaagcccaggcccccctggatgggcctgctgggccccaccatccaggccgaggtgtacgacaccgtggtgatcaccctgaagaacatggccagccaccccgtgagcctgcacgccgtgggcgtgagctactggaaggccagcgagggcgccgagtacgacgaccagaccagccagcgggagaaagaagatgacaaggtgttccctggcggcagccacacctacgtgtggcaggtgctgaaagaaaacggccccatggcctccgaccccctgtgcctgacctacagctacctgagccacgtggacctggtgaaggacctgaacagcggcctgatcggcgctctgctcgtctgccgggagggcagcctggccaaagagaaaacccagaccctgcacaagttcatcctgctgttcgccgtgttcgacgagggcaagagctggcacagcgagacaaagaacagcctgatgcaggaccgggacgccgcctctgccagagcctggcccaagatgcacaccgtgaacggctacgtgaacagaagcctgcccggcctgattggctgccaccggaagagcgtgtactggcacgtgatcggcatgggcaccacacccgaggtgcacagcatctttctggaagggcacacctttctggtccggaaccaccggcaggccagcctggaaatcagccctatcaccttcctgaccgcccagacactgctgatggacctgggccagttcctgctgttttgccacatcagctctcaccagcacgacggcatggaagcctacgtgaaggtggactcttgccccgaggaaccccagctgcggatgaagaacaacgaggaagccgaggactacgacgacgacctgaccgacagcgagatggacgtggtgcggttcgacgacgacaacagccccagcttcatccagatcagaagcgtggccaagaagcaccccaagacctgggtgcactatatcgccgccgaggaagaggactgggactacgcccccctggtgctggcccccgacgacagaagctacaagagccagtacctgaacaatggcccccagcggatcggccggaagtacaagaaagtgcggttcatggcctacaccgacgagacattcaagacccgggaggccatccagcacgagagcggcatcctgggccccctgctgtacggcgaagtgggcgacacactgctgatcatcttcaagaaccaggctagccggccctacaacatctacccccacggcatcaccgacgtgcggcccctgtacagcaggcggctgcccaagggcgtgaagcacctgaaggacttccccatcctgcccggcgagatcttcaagtacaagtggaccgtgaccgtggaggacggccccaccaagagcgaccccagatgcctgacccggtactacagcagcttcgtgaacatggaacgggacctggcctccgggctgatcggacctctgctgatctgctacaaagaaagcgtggaccagcggggcaaccagatcatgagcgacaagcggaacgtgatcctgttcagcgtgttcgatgagaaccggtcctggtatctgaccgagaacatccagcggtttctgcccaaccctgccggcgtgcagctggaagatcccgagttccaggccagcaacatcatgcactccatcaatggctacgtgttcgactctctgcagctctccgtgtgtctgcacgaggtggcctactggtacatcctgagcatcggcgcccagaccgacttcctgagcgtgttcttcagcggctacaccttcaagcacaagatggtgtacgaggacaccctgaccctgttccctttcagcggcgagacagtgttcatgagcatggaaaaccccggcctgtggattctgggctgccacaacagcgacttccggaaccggggcatgaccgccctgctgaaggtgtccagctgcgacaagaacaccggcgactactacgaggacagctacgaggatatcagcgcctacctgctgtccaagaacaacgccatcgaaccccggagcttcagccagaacccccccgtgctgacgcgtcaccagcgggagatcacccggacaaccctgcagtccgaccaggaagagatcgattacgacgacaccatcagcgtggagatgaagaaagaggatttcgatatctacgacgaggacgagaaccagagccccagaagcttccagaagaaaacccggcactacttcattgccgccgtggagaggctgtgggactacggcatgagttctagcccccacgtgctgcggaaccgggcccagagcggcagcgtgccccagttcaagaaagtggtgttccaggaattcacagacggcagcttcacccagcctctgtatagaggcgagctgaacgagcacctggggctgctggggccctacatcagggccgaagtggaggacaacatcatggtgaccttccggaatcaggccagcagaccctactccttctacagcagcctgatcagctacgaagaggaccagcggcagggcgccgaaccccggaagaacttcgtgaagcccaacgaaaccaagacctacttctggaaagtgcagcaccacatggcccccaccaaggacgagttcgactgcaaggcctgggcctacttcagcgacgtggatctggaaaaggacgtgcactctggactgattggcccactcctggtctgccacactaacaccctcaaccccgcccacggccgccaggtgaccgtgcaggaattcgccctgttcttcaccatcttcgacgagacaaagtcctggtacttcaccgagaatatggaacggaactgcagagccccctgcaacatccagatggaagatcctaccttcaaagagaactaccggttccacgccatcaacggctacatcatggacaccctgcctggcctggtgatggcccaggaccagagaatccggtggtatctgctgtccatgggcagcaacgagaatatccacagcatccacttcagcggccacgtgttcaccgtgcggaagaaagaagagtacaagatggccctgtacaacctgtaccccggcgtgttcgagacagtggagatgctgcccagcaaggccggcatctggcgggtggagtgtctgatcggcgagcacctgcacgctggcatgagcaccctgtttctggtgtacagcaacaagtgccagaccccactgggcatggcctctggccacatccgggacttccagatcaccgcctccggccagtacggccagtgggcccccaagctggccagactgcactacagcggcagcatcaacgcctggtccaccaaagagcccttcagctggatcaaggtggacctgctggcccctatgatcatccacggcattaagacccagggcgccaggcagaagttcagcagcctgtacatcagccagttcatcatcatgtacagcctggacggcaagaagtggcagacctaccggggcaacagcaccggcaccctgatggtgttcttcggcaatgtggacagcagcggcatcaagcacaacatcttcaacccccccatcattgcccggtacatccggctgcaccccacccactacagcattagatccacactgagaatggaactgatgggctgcgacctgaactcctgcagcatgcctctgggcatggaaagcaaggccatcagcgacgcccagatcacagccagcagctacttcaccaacatgttcgccacctggtccccctccaaggccaggctgcacctgcagggccggtccaacgcctggcggcctcaggtcaacaaccccaaagaatggctgcaggtggactttcagaaaaccatgaaggtgaccggcgtgaccacccagggcgtgaaaagcctgctgaccagcatgtacgtgaaagagtttctgatcagcagctctcaggatggccaccagtggaccctgttctttcagaacggcaaggtgaaagtgttccagggcaaccaggactccttcacccccgtggtgaactccctggacccccccctgctgacccgctacctgagaatccacccccagtcttgggtgcaccagatcgccctcaggatggaagtcctgggatgtgaggcccaggatctgtactgatgacgtctggaacgcgtcgacaatcaacctctggattacaaaatttgtgaaagattgactggtattcttaactatgttgctccttttacgctatgtggatacgctgctttaatgcctttgtatcatgctattgcttcccgtatggctttcattttctcctccttgtataaatcctggttgctgtctctttatgaggagttgtggcccgttgtcaggcaacgtggcgtggtgtgcactgtgtttgctgacgcaacccccactggttggggcattgccaccacctgtcagctcctttccgggactttcgctttccccctccctattgccacggcggaactcatcgccgcctgccttgcccgctgctggacaggggctcggctgttgggcactgacaattccgtggtgttgtcggggaaatcatcgtcctttccttggctgctcgcctgtgttgccacctggattctgcgcgggacgtccttctgctacgtcccttcggccctcaatccagcggaccttccttcccgcggcctgctgccggctctgcggcctcttccgcgtcttcgccttcgccctcagacgagtcggatctccctttgggccgcctccccgcctggtacctttaagaccaatgacttacaaggcagctgtagatcttagccactttttaaaagaaaaggggggactggaagggctaattcactcccaacgaaaataagatctgctttttgcttgtactgggtctctctggttagaccagatctgagcctgggagctctctggctaactagggaacccactgcttaagcctcaataaagcttgccttgagtgcttcaagtagtgtgtgcccgtctgttgtgtgactctggtaactagagatccctcagacccttttagtcagtgtggaaaatctctagcagtagtagttcatgtcatcttattattcagtatttataacttgcaaagaaatgaatatcagagagtgagaggaacttgtttattgcagcttataatggttacaaataaagcaatagcatcacaaatttcacaaataaagcatttttttcactgcattctagttgtggtttgtccaaactcatcaatgtatcttatcatgtctggctctagctatcccgcccctaactccgcccagttccgcccattctccgccccatggctgactaattttttttatttatgcagaggccgaggccgcctcggcctctgagctattccagaagtagtgaggaggcttttttggaggcctagacttttgcagagacggcccaaattcgtaatcatggtcatagctgtttcctgtgtgaaattgttatccgctcacaattccacacaacatacgagccggaagcataaagtgtaaagcctggggtgcctaatgagtgagctaactcacattaattgcgttgcgctcactgcccgctttccagtcgggaaacctgtcgtgccagctgcattaatgaatcggccaacgcgcggggagaggcggtttgcgtattgggcgctcttccgcttcctcgctcactgactcgctgcgctcggtcgttcggctgcggcgagcggtatcagctcactcaaaggcggtaatacggttatccacagaatcaggggataacgcaggaaagaacatgtgagcaaaaggccagcaaaaggccaggaaccgtaaaaaggccgcgttgctggcgtttttccataggctccgcccccctgacgagcatcacaaaaatcgacgctcaagtcagaggtggcgaaacccgacaggactataaagataccaggcgtttccccctggaagctccctcgtgcgctctcctgttccgaccctgccgcttaccggatacctgtccgcctttctcccttcgggaagcgtggcgctttctcatagctcacgctgtaggtatctcagttcggtgtaggtcgttcgctccaagctgggctgtgtgcacgaaccccccgttcagcccgaccgctgcgccttatccggtaactatcgtcttgagtccaacccggtaagacacgacttatcgccactggcagcagccactggtaacaggattagcagagcgaggtatgtaggcggtgctacagagttcttgaagtggtggcctaactacggctacactagaaggacagtatttggtatctgcgctctgctgaagccagttaccttcggaaaaagagttggtagctcttgatccggcaaacaaaccaccgctggtagcggtggtttttttgtttgcaagcagcagattacgcgcagaaaaaaaggatctcaagaagatcctttgatcttttctacggggtctgacgctcagtggaacgaaaactcacgttaagggattttggtcatgagattatcaaaaaggatcttcacctagatccttttaaattaaaaatgaagttttaaatcaatctaaagtatatatgagtaaacttggtctgacagttaccaatgcttaatcagtgaggcacctatctcagcgatctgtctatttcgttcatccatagttgcctgactccccgtcgtgtagataactacgatacgggagggcttaccatctggccccagtgctgcaatgataccgcgagacccacgctcaccggctccagatttatcagcaataaaccagccagccggaagggccgagcgcagaagtggtcctgcaactttatccgcctccatccagtctattaattgttgccgggaagctagagtaagtagttcgccagttaatagtttgcgcaacgttgttgccattgctacaggcatcgtggtgtcacgctcgtcgtttggtatggcttcattcagctccggttcccaacgatcaaggcgagttacatgatcccccatgttgtgcaaaaaagcggttagctccttcggtcctccgatcgttgtcagaagtaagttggccgcagtgttatcactcatggttatggcagcactgcataattctcttactgtcatgccatccgtaagatgcttttctgtgactggtgagtactcaaccaagtcattctgagaatagtgtatgcggcgaccgagttgctcttgcccggcgtcaatacgggataataccgcgccacatagcagaactttaaaagtgctcatcattggaaaacgttcttcggggcgaaaactctcaaggatcttaccgctgttgagatccagttcgatgtaacccactcgtgcacccaactgatcttcagcatcttttactttcaccagcgtttctgggtgagcaaaaacaggaaggcaaaatgccgcaaaaaagggaataagggcgacacggaaatgttgaatactcatactcttcctttttcaatattattgaagcatttatcagggttattgtctcatgagcggatacatatttgaatgtatttagaaaaataaacaaataggggttccgcgcacatttccccgaaaagtgccacctgacgtctaagaaaccattattatcatgacattaacctataaaaataggcgtatcacgaggccctttcgtctcgcgcgtttcggtgatgacggtgaaaacctctgacacatgcagctcccggagacggtcacagcttgtctgtaagcggatgccgggagcagacaagcccgtcagggcgcgtcagcgggtgttggcgggtgtcggggctggcttaactatgcggcatcagagcagattgtactgagagtgcaccatatatgcggtgtgaaataccgcacagatgcgtaaggagaaaataccgcatcaggcgccattcgccattcaggctgcgcaactgttgggaagggcgatcggtgcgggcctcttcgctattacgccagctggcgaaagggggatgtgctgcaaggcgattaagttgggtaacgccagggttttcccagtcacgacgttgtaaaacgacggccagtgccaagctg

SEQ ID NO: 53 - DNA, 20 bp, Artificial Sequence
  Primer
aacggctacgtgaacagaag

SEQ ID NO: 54 - DNA, 20 bp, Artificial Sequence
  Primer
gatagggctgatttccaggc

SEQ ID NO: 55 - DNA, 19 bp, Artificial Sequence
  Primer
gaaggtgaaggtcggagtc

SEQ ID NO: 56 - DNA, 20 bp, Artificial Sequence
  Primer
gaagatggtgatgggatttc